European Patent Specification EP 3 607 055 B1, published May 14, 2025. Title: COMPOSITIONS FOR REPROGRAMMING CELLS INTO DENDRITIC CELLS OR ANTIGEN PRESENTING CELLS, METHODS AND USES THEREOF. Applicant: CENTRO DE NEUROCIÊNCIAS E BIOLOGIA CELULAR. The sequence listing filed with the application follows.

SEQUENCE LISTING (66 sequences)

SEQ ID NO: 1 - DNA, 992 bp, Homo sapiens
  Human BATF3 (NM_018664.2)
ggggcagacgtgggacgggaaggacggctgccgggactggcgcgcggggacactgggccgacgcgtggagtagcggggagagcgggaagcctgagggggcggggccggcgcgaggccgtgggtgcggcacgaggatgccggcggcgggacagcgcccgtaggcagccccacgggcagggcgcgcgggcggggcggggcgggccgggccagaggagcgcccggcatgtcgcaagggctcccggccgccggcagcgtcctgcagaggagcgtcgcggcgcccgggaaccagccgcagccgcagccgcagcagcagagccctgaggatgatgacaggaaggtccgaaggagagaaaaaaaccgagttgctgctcagagaagtcggaagaagcagacccagaaggctgacaagctccatgaggaatatgagagcctggagcaagaaaacaccatgctgcggagagagatcgggaagctgacagaggagctgaagcacctgacagaggcactgaaggagcacgagaagatgtgcccgctgctgctctgccctatgaactttgtgccagtgcctccccggccggaccctgtggccggctgcttgccccgatgaagccggggacactcctctgcccagcaaggagccttggtcattttcatacctgggaggaaggcttttccttcacaattgtatacagggggcacctgtggccaggcctcctcctgggagctccaggaccagccagctgtgttccctgcagactgggctcagcccgacatccaacaggcgccaaactcacagagcccttgtgcagatccagcatggaggccaccctcaggagtgacttctcatccaccctggcagctagtaggttctgctgttatgcagagccatttcctctagaatttggataataaagatgcttattgtctctcccttctccagttctgggaatttacaggcacaatacacttccttttcctggaaaaaaaaaaaa

SEQ ID NO: 2 - DNA, 712 bp, Mus <mouse, genus>
  Mouse Batf3 (NM_030060.2)
agcagagccccacgttcagggcgccccgtgtggcgagcgcgcggcatgtcgcaagggccccccgcggtcagcgtgctgcagagaagcgtggatgcgcccgggaaccagccgcagagccccaaggacgatgacaggaaagttcgaaggagagagaaaaaccgggttgcagctcagaggagccggaagaagcagacccagaaggctgacaagctccacgaggagcacgagagcctggagcaggagaactctgtgctgcgcagggagatttcgaagctgaaggaggagctgcgtcacctgagcgaggtgctgaaggagcacgagaagatgtgcccgctgctgctgtgtcctatgaactttgtgcagcttcggtcagaccccgtggccagctgtctaccacgatgacaccccagctcactcctcctttgtccggctcggaaccttggtttgcacactcaggagtttccctacacacctgtgtccaggggtacatgtggctgtgcccttccagggagctctggggccagcctgggctcagcatcgtgctctggggcatctgacttccggcccctgccttccggccccaggacagaggatccagaggccccagcaagaaggccctttgagtcgttcctctctcactttggcagctagccggtgctgtcctttggcaggatcttttcgtctagaacttggaaaataaagatagttacct

SEQ ID NO: 3 - DNA, 3537 bp, Homo sapiens
  Human SPIB (NM_003121.4)
ggcaaacagcccgcccggcaccaccatgctcgccctggaggctgcacagctcgacgggccacacttcagctgtctgtacccagatggcgtcttctatgacctggacagctgcaagcattccagctaccctgattcagagggggctcctgactccctgtgggactggactgtggccccacctgtcccagccaccccctatgaagccttcgacccggcagcagccgcttttagccacccccaggctgcccagctctgctacgaaccccccacctacagccctgcagggaacctcgaactggcccccagcctggaggccccggggcctggcctccccgcataccccacggagaacttcgctagccagaccctggttcccccggcatatgccccgtaccccagccctgtgctatcagaggaggaagacttaccgttggacagccctgccctggaggtctcggacagcgagtcggatgaggccctcgtggctggccccgaggggaagggatccgaggcagggactcgcaagaagctgcgcctgtaccagttcctgctggggctactgacgcgcggggacatgcgtgagtgcgtgtggtgggtggagccaggcgccggcgtcttccagttctcctccaagcacaaggaactcctggcgcgccgctggggccagcagaaggggaaccgcaagcgcatgacctaccagaagctggcgcgcgccctccgaaactacgccaagaccggcgagatccgcaaggtcaagcgcaagctcacctaccagttcgacagcgcgctgctgcctgcagtccgccgggcctgagcacacccgaggctcccacctgcggagccgctgggggacctcacgtcccagccaggatccccctggaagaaaaagggcgtccccacactctaggtgataggacttacgcatccccaccttttggggtaaggggagtgctgccctgccataatccccaagcccagcccgggcctgtctgggattccccacttgtgcctggggtccctctgggatttctttgtcatgtacagactccctgggatcctcatgttttgggtgacaggacctatggaccactatactcggggaggcagggtagcagttcttccagaatcccaagagcttctctgggattttcttgtgatatctgattccccagtgaggcctgggacgtttttaagatcgctgtgtgtctgtaaaccctgaatctcatctggggtgggggccctgctggcaaccctgagccctgtccaaggttccctcttgtcagatctgagatttcctagttatgtctggggccctctgggagctgttatcatctcagatctcttcgcccatctatggctgtgttgtcacatctgtcccctcatttttgagatcccccaattctctggaactattctgctgcccctttttatgtgtctggagttccccaatcacatctagggctcctccaagatccttttgtcatgtctgaaatcactcttgagaggtctggggtggaggatggggagtcagtgaaatgtgtcatgtctgggccctgtcagggacacccttgttatatctgggatcctccaatcacatctgagacctcctaggctctccatctgatatgccctttcagggaccccacaaagactgagttctcatggggatcctacccttcctagtgccactccctatggccatgctgaagaccactctggccacgcgactgattttgggtgatcatggcagctccccacccatgtcatttctaaccagaagtctcaaggtcgtcacccccctgccccccaaccgaggccccggtcgctggtggtggtctctttagtgcactgtagcacttggtggtggaggtgtgagggatccacattaacagcaggccatcagctgggcaatggctcacacctgtaatcccagcactttgggaggcgaggcagggggaatggcttgaacccaggcattcaagaccagcctgggcaacataatgagacctcgtctctacaaaacataacaaaaacaattagccgagcgtgggggtgaacacctgtggtcccagctgctcaggaggctgaggtgggaggatctcttgagcccaggaagtaggaggctgtagtgagctgtaatcgtgccactgcactccagcctgggcgacagagtgagacaccgtcttaaaaacaaaaacaaggccgggcacggtggctcatgcctgttgtcccagcactttgggaggccgaggcaggcggatcacgaggtcgagagatcgagaccatcctggccaacatggtgaaaccctgtctctactaaaaatacagaaattagctgggcgtggtggcacgtgcctgtagtcccagctactcgggaggctgaggcaagagaatcgcttgaacgtgggaggcagaggttgcagtgagcctagattgtgccactgcactccagcctgggggacagagcgagactccgtctgaaaataaaaacaacaaaaacagcagaccattcaaaatagggagactttgcataatccagatttctgccttcacttaaaactttggacggtctggagagagtcggccagttttcggtggggggtggggagctggaacaggacagtagcctttcctaatgaggcatttgttctccaatctgccccagtcgctgccatccctggctatctcaccctagcagcttctcaagcctgttggctttagaccactgtataaacccagctggaactgaagcctgggtggactatggagccctggttgggacccccagggagtcaaaggctgcgggccaagaggccagaggtccttgagcctgggtgggcaggtggatctagggtgcatgacttgctgcttcccaaccttagtttgtcccttctgtgaaaaagggagagaaggaggaggaagatctcaaaaagactttccagcccagtgcggtggctcacgcctgtaatcccagcactttgggaggccgatgcaggtggatcacctgaggtaggagttcaagaccagcctgaccaacatagtgaagccccttctctactaaaaatacaaaattagctgggcgtggtggcatgtgcctgtactcccagctacttgggaggctgaggcaggagaatcgcttgaacctgggaggcggaggttgtagtgagctgagatcacaccactgcacaccagcctgggcgacaagagcgaaactccgtctcaaaaaaaaaaaactgttgcagccccgttgagcctttgacaccgcctgaaatccaccccactcccaggaggaggaggaggaaggaatgccaatgacctagagacacgagaagtccatgtggaggcacacagcagctgatggcagagcccaggctgggacctgcccttaagagaatgagtgggaagggggagggaggaagggcaggtaaaacgtcctccccagggccccctgcaacggggaaggtactttttacaaaagctatcattgtcaccctaaatgtggaataaaataagatgcatcgacgtagacaaaaaaaa

SEQ ID NO: 4 - DNA, 2786 bp, Mus <mouse, genus>
  Mouse SpiB (NM_019866.1)
agcctgctctgaaccaccatgcttgctctggaggctgcacagctggatggcccacacttaagctgtttgtacccagaaggagtcttctacgacctggacagctgcaagcccttcagttacccagattcagatgggggccttgactctacatggggctggacagaggccccgcctgctcctgccatcgctccctatgaagccttcgatcctgctactgctgcctttagccactcccaaactgttcagctctgttatagccatggtcctaacccctccacctatagccccatggggaccctcgacccagcccccagcttggaggccccagggcctggcctccaggtgtaccccccagaggacttcaccagccagaccctgggctccttggcttatgctccgtaccccagccctgtgctatcagaggaagaagacattatgctggacagccccgccctggaggtctcggacagtgagtcagacgaggccctcttggctggctccgaggggaggggatctgaggcaggtgcacgcaagaagctgcgcctgtaccagttcttgctggggttgctcctacgcggggacatgcgcgagtgcgtgtggtgggtggagccaggtgccggcgtcttccagttctcctccaagcacaaggagttgttggctcgccgctggggccagcagaagggcaaccgcaagcgcatgacgtatcagaagctggcccgagcgctgcgcaactatgccaagacaggcgaaatccgcaaggtcaaacgcaaactcacctaccagtttgacagcgcgctgctgccagcctcccggcatgtctgagcactccgctaaggacccctttctggcccctaagtcccatggagccccatatgagggcagtcagggttctcagctctccctagagcctccccagagtttcctgtgccgtgtataggattccaatctaggatggtcgtgtttgagggagcactggccattctacacggtttcagaatggcaggtttctcgggggggggggggatgggggagccctgatgtcgtctacggttccagaaaccgcagttcttgcgagtcctgtgagctcacatgacatctcaccagcaggtggcgctgtctacagccccccccaaacccttgttttgttggccagataggtcggtccctctgtactccccctgaagcccttgttagatctgaggtctagttatgtttggagctctctgagaaccctgtgccacctgtgtgtgacttttctctgcgtccgtttatgacttttgtttgtttgagacagggtctcattatgtagctcaggctggccccccaacttttaacaatcgtcctgcctcggcctcctgagtgctgggatgacaagggtgcaccatcacaccaggttttttccttttttgagagattttactatgtaacccgggctgggctattctcaagctagtggcagtcctcttgcctcaggctcctcttgcctcaggcaccccttgggaccctctgggacctatgtccgagatgaatggctgggtaaggtagggtgggaggttcagtgaaccttataggttgggcccttccttctgggatcccttgatcatatgggaagttctctaggctctcagcagccctgcattcacacactgactgaggcgcgacctgtatgttgtgtttgagggggatgtgtggcagaggtatggctgtggcaaggccggtgccttttattcttgagattgagtcttatgtagctcaggctggtcttgaactcactctcactgtgtagctagggaagaccttgagcccttgcctcagccagaatgctcagatgtcaggcagcgcaccacgtgactgtttctttccattgtcttgtctttttgttgttgttgttttcgagacagggtttctctgtgtagccctggccgttctggaactcactctgtagaccaggctggccttaaactcagaaatccacctgcctctgcctctcaaatgctgggattaaaggcgtgcaccaccacgccctttttcctttttcttaagtcaaggtctatttgtgtagcccaggctggcttcaagctcatgacactcttcctgcctctgcgtctggaactatgaacataccttactactctgtgcttacccacgccatgggtagacagacttctagacttggtcaacccccacccacaaggcaggcaaattaagtccctgcaggtgctttctttggaggaaagcccgctttcatagtgatctgtcaagctagaaagcactcccgccacccagatatctaagtgtgaatctttggacaactggtgacttctggccagcttttctggggccggcctctgtccaggtgtctgcccaggaccctgctcagtgcctgtctgtctcacaccagtgacttcctcacacccgcctgttcaggcccagtcttttccgttcaagtgctacaggccaagtaggctcaaactgtgggtttgtcttgggcatccacagcagaatcagaacccagagctttgaagcctgagtgaggggaggggggcactcaggcttccgtctctctgagaaacagacgatgaagaggcccttaaaactctttgcaaccccatgagcctccccaatgagcctgtgacacaccggaactcacctctgtgggtggccgggagggggaacagggtcatggaagatccagatgtccatgtggtcaaggctaaactgtactaaataaaattatttctcatcaccactatacatgcataataaataaagtgtacatcaaaatt

SEQ ID NO: 5 - DNA, 2678 bp, Homo sapiens
  Human IRF8 (NM_002163.2)
agcgcggcagcaagcgtgggaacgcgggcggcgagacggcggcaggacggcggcaggatgtgtgaccggaatggtggtcggcggcttcgacagtggctgatcgagcagattgacagtagcatgtatccaggactgatttgggagaatgaggagaagagcatgttccggatcccttggaaacacgctggcaagcaagattataatcaggaagtggatgcctccatttttaaggcctgggcagtttttaaagggaagtttaaagaaggggacaaagctgaaccagccacttggaagacgaggttacgctgtgctttgaataagagcccagattttgaggaagtgacggaccggtcccaactggacatttccgagccatacaaagtttaccgaattgttcctgaggaagagcaaaaatgcaaactaggcgtggcaactgctggctgcgtgaatgaagttacagagatggagtgcggtcgctctgaaatcgacgagctgatcaaggagccttctgtggacgattacatggggatgatcaaaaggagcccttccccgccggaggcctgtcggagtcagctccttccagactggtgggcgcagcagcccagcacaggcgtgccgctggtgacggggtacaccacctacgacgcgcaccattcagcattctcccagatggtgatcagcttctactatgggggcaagctggtgggccaggccaccaccacctgccccgagggctgccgcctgtccctgagccagcctgggctgcccggcaccaagctgtatgggcccgagggcctggagctggtgcgcttcccgccggccgacgccatccccagcgagcgacagaggcaggtgacgcggaagctgttcgggcacctggagcgcggggtgctgctgcacagcagccggcagggcgtgttcgtcaagcggctgtgccagggccgcgtgttctgcagcggcaacgccgtggtgtgcaaaggcaggcccaacaagctggagcgtgatgaggtggtccaggtcttcgacaccagccagttcttccgagagctgcagcagttctataacagccagggccggcttcctgacggcagggtggtgctgtgctttggggaagagtttccggatatggcccccttgcgctccaaactcattctcgtgcagattgagcagctgtatgtccggcaactggcagaagaggctgggaagagctgtggagccggctctgtgatgcaggcccccgaggagccgccgccagaccaggtcttccggatgtttccagatatttgtgcctcacaccagagatcatttttcagagaaaaccaacagatcaccgtctaagtgcgtcgcttgggcgccccaccccgtctgcgtcctgcatccatctccctgttacagtggcccgcatcatgattaaagaatgtggatccctctgtctggggtgggatgccttactttgcacttaatttaataagggcattctcggaggagtagacgtttaatacgaagtggcggcatagccctgccgagatgtcggtgatggcctggatgctgtaaccacaacctgtggctaaaaattttattttctatcctttacccgtcattatcattagttgctatgattctttctgcattttcggttaactatcatttccaaagacttgtcattcagtaatattagcagatagctgcttcgataaaggaatttggagtttaaaaatcaacttgtgaaaacaaggttgtttttgtctttatcgtttgttagagttatagatttatgatttcataggcttgattctatgtgaaatatctttttacttttatgcattttaataagatttaaaaatatttagattaaagccccctttaatgagtacaagaaaaactcttggcttgttagaagaaagtatattctttctagaatttggtgcaggaatatgtgttcatatccaggcaaacgggtgtgtttttatcttcagacaatgaaaccttctcctctggggctttgttgccaggaagattagaactaaatttatttttttcatttctgtcatgaaatcattccagatacctcttttcttctttccaaatggttttcacatgtgtttgaaatatttgtacttcgaattgtcggattttccatgtcctcctttctcctttgtgcccagcctgagtcagcaccaatcccgcattcagaacctcccagtgaaagggcagccttcattttgagaaggtggaaggtgttagggtttgggagacagctcatccaatctcccaagtctcatggtggatttgtgactgtgagagtttccggtttaaaatctgaaaagccagatatgcctgtttccttttcccagcaccatgcctgtggaggggacagtcagacccagaggtcctttacgtgtggatggagttcacaggcgaatagaggagaggaccaggggacgtggcttgtcccttttgtccaacaaagcattatatttttaagaatggcagacctgtttgctgaagtgttcataagataacaataggcttgaatctccaattcaaatgaatgtcaaagcacatatctttaatatgctgaatgaatatttatttttgtatccattaaaacagtatattgatctcttttattctttattaaaataaaatgctcttttttaaaaaaaaaaaaaaaaaaa

SEQ ID NO: 6 - DNA, 3391 bp, Mus <mouse, genus>
  Mouse Irf8 (NM_001301811.1)
ttccaagcccactggtggcagttagggctgctgtgtggctaaaaccagccctggagagacctcatctccctcctctcaggctgctgccgtctttcctggccccactaccacctgcaagcggcctggagtttctgaccctcaggcctctttccagcaatcctgactttgtgggacatgctggctctggatgtgactatgttcttggggatatcttgacttctcactgatgataacttcttttttttttttttttccctaccccaagaggtcattttagttggaagactagaagtgctgtgttctggttttcagggtgggcgtctgtccaactgctttggggatttccaggctgttctagtaaatgctggctgcaagtccctgtgcacaaatgccctctctccccacgctgtaggaaaagcagacccgagagtgtccaagtgtgccattaggtgtctggggatggcgggcctggatatggagtccctgagctggctttgtactgtccctttgttctcactgagggctgattgtaagagggactccctgtgttgttggaggagtcctctaggatacaggctctgattgcaggatgtgtgaccggaacggcgggcggcggctgcggcagtggctgatcgaacagatcgacagcagcatgtacccggggctgatctgggaaaatgatgagaagaccatgttccgtatcccctggaagcatgccggcaagcaggattacaatcaggaggtggatgcttccatcttcaaggcctgggcagtttttaaagggaagtttaaagagggagacaaagctgaaccagccacgtggaagacgaggttacgctgtgctctgaacaagagcccagattttgaagaagtgactgaccggtcccagctggacatttctgagccatataaagtttaccgaattgtccccgaggaagaacaaaaatgcaagctgggcgtggcacctgcaggctgcatgagcgaagttcctgagatggagtgtggccgctcagagattgaggagctgatcaaggaaccttctgtggatgagtacatgggtatgaccaagaggagcccatccccaccagaggcctgcaggagccagatcctccctgactggtgggtccagcagcccagtgcaggcctgccactggtgaccggatatgccgcctatgacacacaccattcagctttctcccagatggtcatcagcttctactacgggggcaagctggtgggccaggccaccaccacctgccttgaaggctgccgtctctccctgagccagccggggctgcctaagttgtatgggccggatggcctggaacccgtgtgctttccgacggccgacaccatccccagtgagcggcagaggcaggtgacccggaagctgtttgggcacctggaacgtggcgtgctactgcacagcaaccgcaagggcgtgttcgtgaagcggctgtgccagggccgcgtgttctgcagcggcaacgcggtggtgtgcaagggcaggcccaacaagctggagcgggacgaggtggtgcaggtctttgacaccaaccagttcatccgagagctgcagcaattctacgccacccagagccgcctacctgacagcagggtggtcctgtgcttcggggaggagtttccggacactgtgcccttgcgctccaaactcattctggtgcaggtagagcagctgtatgccaggcagctggtggaggaagcgggcaagagctgcggtgctggctccctgatgccagccctggaggagccccagccggaccaggctttccgcatgtttccggatatctgtacctcacaccagagacccttttttagagaaaatcaacagatcaccgtctaagcctcagtccgggcaccccacctcgcctgagctcaagcttcaagagtctgtgactaagagaattccgaaaggatgtggagccctctgactggggtgggcgggtgtcctccaaggggcctccggaagcccacagagggatgcgctcctgctcaggcaggtgtcagaagcttgcaggggctgtggccgcaacctgtgattaaagcattcctttcctgcgtttcccccttcaccactaatggctggcctttctgtgtgctgaggtctttcgacagttcaaatcatctggtggcagcagactcgcctttgcccttctgcggccgagggcggagatttatgactttctctgcttggttggagaagaagaatctttactattcagcttcttttctttttggccagaactctgaaaaaaaaaaaaactctttttaagacaatatttgtattctcacaggctcagctgtcaatcacttgagaccttccctgtaaagtggggcagattttaaatatgggtgtagatactgcttgcagccttcgcaggaattttggttgtggttcattgattcacacagactctgtgtcagctgacagggctgtgtggggcatcaaaggaggaccaggcactgtggagaagacccattcactggcatctcacccttccttgtccagctccatacccagtcctaagacccagtgaaaagccacgtccaaactgtgctctgggctcatcagtgcccacccacgtaccagggaaaggcacacaccctacccagtgggcacagagcggaatgtccccctaccgcaccatttgcgcccccaatctggctgtccaacctagtttgtaagtaatctaaatcagtgactatagccccgcctaagggacacttcccggaggagggagccgctgaaaaggagttagtttgagggtcagtacacaacaggggcagaaagccaagcagatgtgggggcagggagagtcatcatctgcttttgtctgagagaaggagagcttctccgtttgttcaactttgtaacaagctgggttacatgctccacgcagctagagaagcctaggtgctctgcattccctggggaactgcaggaaagccttacctgctgactgttgctctggggaaaagcctgagggtccagagcagctacaagctacaggccataccttacaacctgaaaagctaaggaccacggtgaccttcccggctactgtgtgaaggtgctgggtggggcctgctcaacagacagggtcgacagagtgtgtgatacatgcaaacagaatccttggagtgtgtgatacatgcaaacagaatcctgggcccctgcttctccccctcagtcaaagcaggagtgtcccttccgaagccaggacaacctgttcacaaggccccttgtcacatgtcaccttccacctgcctcaaggagtgctagtgtccaaatatttatttttgtattctcttaagaagtattgatttcatcctttattaaaaaaagttgctctttcacaaaaaaaaaaaa

SEQ ID NO: 7 - DNA, 1426 bp, Homo sapiens
  Human PU.1 (NM_001080547.1)
gactatctcccagcggcaggcccttcgataaaatcaggaacttgtgctggccctgcaatgtcaagggagggggctcacccagggctcctgtagctcagggggcaggcctgagccctgcacccgccccacgaccgtccagcccctgacggggcaccccatcctgaggggctctgcattggcccccaccgaggcaggggatctgaccgactcggagcccggctggatgttacaggcgtgcaaaatggaagggtttcccctcgtcccccctcagccatcagaagacctggtgccctatgacacggatctataccaacgccaaacgcacgagtattacccctatctcagcagtgatggggagagccatagcgaccattactgggacttccacccccaccacgtgcacagcgagttcgagagcttcgccgagaacaacttcacggagctccagagcgtgcagcccccgcagctgcagcagctctaccgccacatggagctggagcagatgcacgtcctcgatacccccatggtgccaccccatcccagtcttggccaccaggtctcctacctgccccggatgtgcctccagtacccatccctgtccccagcccagcccagctcagatgaggaggagggcgagcggcagagccccccactggaggtgtctgacggcgaggcggatggcctggagcccgggcctgggctcctgcctggggagacaggcagcaagaagaagatccgcctgtaccagttcctgttggacctgctccgcagcggcgacatgaaggacagcatctggtgggtggacaaggacaagggcaccttccagttctcgtccaagcacaaggaggcgctggcgcaccgctggggcatccagaagggcaaccgcaagaagatgacctaccagaagatggcgcgcgcgctgcgcaactacggcaagacgggcgaggtcaagaaggtgaagaagaagctcacctaccagttcagcggcgaagtgctgggccgcgggggcctggccgagcggcgccacccgccccactgagcccgcagcccccgccgggccccgccaggcctccccgctggccatagcattaagccctcgcccggcccggacacagggaggacgctcccggggcccagaggcaggactgtggcgggccgggcctcgcctcacccgccccctccccccactccaggccccctccacatcccgcttcgcctccctccaggactccaccccggctcccggacgccagctgggcgtcagaccccaccggggcaaccttgcagaggacgacccggggtactgccttgggagtctcaagtccgtatgtaaatcagatctcccctctcacccctcccacccattaacctcctcccaaaaaacaagtaaagttattctcaatccatcaaaaaaaaaaaaaaaaaa

SEQ ID NO: 8 - DNA, 1473 bp, Mus <mouse, genus>
  Mouse Pu.1 (NM_011355.2)
aagagatttatgcaaacgggctggggcggtgatgtcaccccaaggggactatctcccagtggcaggcccttcgataaaatcaggaacttgtgctggccctgcaatgtcaagggagggggctcacccagggctcctgtagctcagggggcaggcctgagccctgcgtctgacccacgaccgtccagtcccccgacggggcacctggtcctgagggggatccgccttgatccccaccgaagcaggggatctgaccaacctggagctcagctggatgttacaggcgtgcaaaatggaagggttttccctcaccgcccctccatcggatgacttggttacttacgattcagagctataccaacgtccaatgcatgactactactccttcgtgggcagcgatggagaaagccatagcgatcactactgggatttctccgcacaccatgtccacaacaacgagtttgagaacttccctgagaaccacttcacagagctgcagagtgtgcagcccccgcagctacagcagctctatcgccacatggagctggaacagatgcacgtcctcgatactcccatggtgccaccccacaccggcctcagtcaccaggtttcctacatgccccggatgtgcttcccttatcaaaccttgtccccagcccaccagcagagctcagatgaggaggagggtgagaggcagagccctcccctggaggtgtctgatggagaagctgatggcttggagcctgggccaggtcttctgcacggggagacaggcagcaagaaaaagattcgcctgtaccagttcctgctggacctgctgcgcagcggcgacatgaaggacagcatctggtgggtggacaaggacaaaggtaccttccagttctcgtccaagcacaaggaggcgctggcgcaccgctggggcatccagaagggcaaccgcaagaagatgacctaccagaagatggcgcgcgcgctgcgcaactacggcaagacaggcgaggtgaagaaagtcaagaagaagctcacctaccagttcagcggcgaggtgctgggccgtgggggcctggccgagcggcgcctcccgccccactgatcgcccgcagagaccgccaggctcctggaccccgccggccatagcattaacccgtcgcccggcccggacacagggaggacattcccagggccgaggcaggactgggggcccggcctcgccctcccatgcccggcctggcccgccccacccgctttgcctcccaccaggactctagcccgctccaagggccgcctgggcctcggacctcaaccgagggtcagcctggcttagtggccacggtgcttccttgggagtctggcgctggcacctttttgtatattgaatgctttttaaaaagctcttcctccccaccccctcattagtcactaaagacaagtaaaattattgacagctattctcccagaaaaaaaaaaaaaaaaaaa

SEQ ID NO: 9 - DNA, 5332 bp, Homo sapiens
  Human IRF4 (NM_002460.3)
acctcgcactctcagtttcaccgctcgatcttgggacccaccgctgccctcagctccgagtccagggcgagtgcagagcagagcgggcggaggaccccgggcgcgggcgcggacggcacgcggggcatgaacctggagggcggcggccgaggcggagagttcggcatgagcgcggtgagctgcggcaacgggaagctccgccagtggctgatcgaccagatcgacagcggcaagtaccccgggctggtgtgggagaacgaggagaagagcatcttccgcatcccctggaagcacgcgggcaagcaggactacaaccgcgaggaggacgccgcgctcttcaaggcttgggcactgtttaaaggaaagttccgagaaggcatcgacaagccggaccctcccacctggaagacgcgcctgcggtgcgctttgaacaagagcaatgactttgaggaactggttgagcggagccagctggacatctcagacccgtacaaagtgtacaggattgttcctgagggagccaaaaaaggagccaagcagctcaccctggaggacccgcagatgtccatgagccacccctacaccatgacaacgccttacccttcgctcccagcccagcaggttcacaactacatgatgccacccctcgaccgaagctggagggactacgtcccggatcagccacacccggaaatcccgtaccaatgtcccatgacgtttggaccccgcggccaccactggcaaggcccagcttgtgaaaatggttgccaggtgacaggaaccttttatgcttgtgccccacctgagtcccaggctcccggagtccccacagagccaagcataaggtctgccgaagccttggcgttctcagactgccggctgcacatctgcctgtactaccgggaaatcctcgtgaaggagctgaccacgtccagccccgagggctgccggatctcccatggacatacgtatgacgccagcaacctggaccaggtcctgttcccctacccagaggacaatggccagaggaaaaacattgagaagctgctgagccacctggagaggggcgtggtcctctggatggcccccgacgggctctatgcgaaaagactgtgccagagcaggatctactgggacgggcccctggcgctgtgcaacgaccggcccaacaaactggagagagaccagacctgcaagctctttgacacacagcagttcttgtcagagctgcaagcgtttgctcaccacggccgctccctgccaagattccaggtgactctatgctttggagaggagtttccagaccctcagaggcaaagaaagctcatcacagctcacgtagaacctctgctagccagacaactatattattttgctcaacaaaacagtggacatttcctgaggggctacgatttaccagaacacatcagcaatccagaagattaccacagatctatccgccattcctctattcaagaatgaaaaatgtcaagatgagtggttttctttttcctttttttttttttttttttgatacggggatacggggtcttgctctgtctcccaggctggagtgcagtgacacaatctcagctcactgtgacctccgcctcctgggttcaagagactctcctgcctcagcctccctggtagctgggattacaggtgtgagccactgcacccacccaagacaagtgattttcattgtaaatatttgactttagtgaaagcgtccaattgactgccctcttactgttttgaggaattcagaagtggagatttcagttcagcggttgaggagaattgcggcgagacaagcatggaaaatcagtgacatctgattggcagatgagcttatttcaaaaggaagggtggctttgcatttcttgtgttctgtagactgccatcattgatgatcactgtgaaaattgaccaagtgatgtgtttacatttactgaaatgcgctctttaatttgttgtagattaggtcttgctggaagacagagaaaacttgcctttcagtattgacactgactagagtgatgactgcttgtaggtatgtctgtgccatttctcagggaagtaagatgtaaattgaagaagcctcacacgtaaaagaaatgtattaatgtatgtaggagctgcagttcttgtggaagacacttgctgagtgaaggaaatgaatctttgactgaagccgtgcctgtagccttggggaggcccatcccccacctgccagcggtttcctggtgtgggtccctctgccccgccctccttcccattggctttctctccttggcctttcctggaagccagttagtaaacttcctattttcttgagtcaaaaaacatgagcgctactcttggatgggacatttttgtctgtcctacaatctagtaatgtctaagtaatggttaagttttcttgtttctgcatctttttgaccctcattctttagagatgctaaaattcttcgcataaagaagaagaaattaaggaacataaatcttaatacttgaactgttgcccttctgtccaagtacttaactatctgttcccttcctctgtgccacgctcctctgtttgtttggctgtccagcgatcagccatggcgacactaaaggaggaggagccggggactcccaggctggagagcactgccaggacccaccactggaagcaggatggagctgactacggaactgcacactcagtgggctgtttctgcttatttcatctgttctatgcttcctcgtgccaattatagtttgacagggccttaaaattacttggctttttccaaatgcttctatttatagaatcccaaagacctccacttgcttaagtatacctatcacttacatttttgtggttttgagaaagtacagcagtagactggggcgtcacctccaggccgtttctcatactacaggatatttactattactcccaggatcagcagaagattgcgtagctctcaaatgtgtgttcctgcttttctaatggatattttaaattcattcaacaagcacctagtaagtgcctgctgtatccctacattacacagttcagcctttatcaagcttagtgagcagtgagcactgaaacattattttttaatgtttaaaaagtttctaatattaaagtcagaatattaatacaattaatattaatattaactacagaaaagacaaacagtagagaacagcaaaaaaataaaaaggatctccttttttcccagcccaaattctcctctctaaaagtgtccacaagaaggggtgtttattcttccaacacatttcacttttctgtaaatatacataaacttaaaaagaaaacctcatggagtcatcttgcacacactttcatgcagtgctctttgtagctaacagtgaagatttacctcgttctgctcagaggccttgctgtggagctccactgccatgtacccagtagggtttgacatttcattagccatgcaacatggatatgtattgggcagcagactgtgtttcgtgaactgcagtgatgtatacatcttatagatgcaaagtattttggggtatattatcctaagggaagataaagatgatattaagaactgctgtttcacggggcccttacctgtgaccctctttgctgaagaatatttaaccccacacagcacttcaaagaagctgtcttggaagtctgtctcaggagcaccctgtcttcttaattctccaagcggatgctccatttcaattgctttgtgacttcttcttctttgtttttttaaatattatgctgctttaacagtggagctgaattttctggaaaatgcttcttggctggggccactacctcctttcctatctttacatctatgtgtatgttgactttttaaaattctgagtgatccagggtatgacctagggaatgaactagctatgaaatactcagggttaggaatcctagcacttgtctcaggactctgaaaaggaacggcttcctcattccttgtcttgataaagtggaattggcaaactagaatttagtttgtactcagtggacagtgctgttgaagatttgaggacttgttaaagagcactgggtcatatggaaaaaatgtatgtgtctcccaggtgcatttcttggtttatgtcttgttcttgagattttgtatatttaggaaaacctcaagcagtaattaatatctcctggaacactatagagaaccaagtgaccgactcatttacaactgaaacctaggaagcccctgagtcctgagcgaaaacaggagagttagtcgccctacagaaaacccagctagactattgggtatgaactaaaaagagactgtgccatggtgagaaaaatgtaaaatcctacagtgaaatgagcagcccttacagtattgttaccaccaagggcaggtaggtattagtgtttgaaaaagctggtctttgagcgagggcataaatacagctagccccaggggtggaacaactctgggagtcttgggtactcgcacctcttggctttgttgatgctccgccaggaaggccacttgtgtgtgcgtgtcagttacttttttagtaacaattcagatccagtgtaaacttccgttcattgctctccagtcacatgcccccacttccccacaggtgaaagtttttctgaaagtgttgggattggttaaggtctttatttgtattacgtatctccccaagtcctctgtggccagctgcatctgtctgaatggtgcgtgaaggctctcagaccttacacaccattttgtaagttatgttttacatgccccgtttttgagactgatctcgatgcaggtggatctccttgagatcctgatagcctgttacaggaatgaagtaaaggtcagtttttttttgtattgattttcacagctttgaggaacatgcataagaaatgtagctgaagtagaggggacgtgagagaagggccaggccggcaggccaaccctcctccaatggaaattcccgtgttgcttcaaactgagacagatgggacttaacaggcaatggggtccacttccccctcttcagcatcccccgtaccccactttctgctgaaagaactgccagcaggtaggaccccagaggcccccaaatgaaagcttgaatttcccctactggctctgcgttttgctgagatctgtaggaaaggatgcttcacaaactgaggtagataatgctatgctgtcgttggtatacatcatgaatttttatgtaaattgctctgcaaagcaaattgatatgtttgataaatttatgtttttaggtaaataaaaacttttaaaaatttgttaaaaaa

SEQ ID NO: 10 - DNA, 4762 bp, Mus <mouse, genus>
  Mouse Irf4 (NM_013674.2)
tttcctagtttcaccacttgaacttgggaccctttgctgccctcagctaagagtgcgggtgagcgcacaagcccaggaggaggtccgcacgcgtcatgaacttggagacgggcagccggggctcagagttcggcatgagcgcagtgagctgcggcaatgggaaactccgacagtggttgatcgaccagatcgacagcggcaagtaccccgggctggtgtgggagaacgaggagaagagcgtcttccgcatcccgtggaaacacgcgggcaagcaggactacaatcgtgaggaggacgctgccctcttcaaggcttgggcattgtttaaaggcaagttccgagaagggatcgacaagccagatcctcctacttggaagacaagattacgatgtgctctgaacaagagcaatgactttgaggaattggtcgagaggagccagctggatatctctgacccatacaaggtgtacaggattgttccagagggagccaaaaaaggagcaaagcagctcactttggatgacacacagatggccatgggccacccctaccccatgacagcaccttatggctctctgccagcccagcaggttcataactacatgatgccaccccatgacaggagctggagggattatgcccctgaccagtcacacccagaaatcccatatcaatgtcctgtgacgtttggcccacgaggccaccactggcaaggcccatcttgtgaaaatggttgccaggtgacaggaaccttttatgcttgtgccccacctgagtcccaggctcctggaatccccattgagccaagcataaggtctgctgaagccttggcgctctcagactgccggctgcatatctgcctgtattaccgggacatcctcgtgaaagagctgaccacgacgagccctgaaggctgccggatctcccacggacacacctatgatgttagcaacctggaccaggtcctgtttccctacccggacgacaatggacagaggaagaacattgagaagttgctgagccacctggagaggggactggtcctctggatggctccagatgggctttatgccaaaagactctgccagagtaggatctactgggatgggcccctggcactgtgcagcgatcggcccaacaagctagaaagagaccagacttgcaagctctttgacacacagcagtttctatcagagctgcaagtgtttgctcaccatggccggccagcaccgagattccaggtgactctgtgctttggtgaggagtttccagaccctcagagacagaggaagctcatcacagctcatgtggaacctctgctagccagacaactgtattactttgctcaacaaaacactggacatttcctgaggggctacgagttacctgaacacgttaccactccagattaccaccgctccctccgtcattcttccatccaagagtgagaagaaatactctgacagggcagccggctgctgccctttctctttggaagagctaagaagtgagtgggtttccacttgaagacaacaacagggctttgtgaggaaaaacagctgtatctgctcaacagaggagcttcccccagaagagtgcctgtcatccaggtcttgacaagtgccaggacttgggtgactgtgccctggcttataactgtgaaacttgatcagtgttgtgtttacatgtacttgaatgctggctttagcctggtatagatggacttttgcttgaagactgaaaacctgtgccagcatgaatccctgacaagagaagacatacgtattattggtccatttctcagggaagtaaagtctagactagagactacgctgtccactcacagagaaacgcattcctggatagaggagctgtaggttgcccagatcatgtccactgagtgaagggacttggttcttaggtccagtctaggctatcatgtcctgatcctgcactctctctgagtagaccctacatcctgtttgctccctcttcttgcccttccctaaaagccagctggtggactcttgttgccacatacttgagccaaaaaaccatcagggacatataagatgagacatgtttgcatctcctctgatctaacaacggctacaaagttttttgttgttgttgtctcccctttctgttttgcctctcattctttagaattgttgcttttttgtaaagaaaggaagagagagagaccgaatatactagagatagatttttaaaattctgtgccatttccccttctatttgttttgttggccatcagtggtccccatggcaacactggaagggcggagcctttgagcaggttgggaactgtcccggacaccagtggttcagtgtacagctgtagactcagtgagctgtttctgcttattttgtatattagatgcttccttgtgccaataatagtttgacagagtctcaaagctaccgggcttcttttccaacaacacattctttcacagaatcccaaagagtctcacttgccttcacaaccgtctgatcctttattgttactgttttgtttaggtggctttgccatgctctgggatttttctcctaccacaacatcattcctgactctttcgggctcagaaagagttaagcgctcttgcacacttggcacttacttctttttaattttttttttaacatgccactcttaatatttcttcttaagtctttcagcagcatacattcaataagcaatggaccattgggtgtctcatttcattgttttatttttaaaaaggaacctttgacaaataatacacattacagaaaatggaagcatttttcatagagaaggtaagaactgaaatgcattttatgttcgaatcctccttgctagtattagccccaagagttcagtctgtcctttaagcatgttttagttttcaatacatatatatgaagttgccctttcttagagagagagagagagatatgtgatgacactcttatgtacccaactatacagatttacctcatcttttgagtggcatgtggacttccactgctatgtgcctaggtgcagtttagacatcttcttagctacccatcccagcagcccactgagtctcgtgaactaaagtcacttatacatcttatagatgcaaaacattctggggtatattatcccaagggaagatgaaggcaaaatcgggaagcactcttcctgaggccccaagccacagctgtcctcctggagtatcttaaccatatctggcacttcaccaaggtcccttgcctggtcctgtatgaccatgactcttcagtccataagcagatgctttgtctcaattgccatgtgaagtcttttggtttttggtttttttccttaatgttaagctgttttaacagtgaagctgaattttctggaaaatgctgtatggttcgagcccccagttcatgtttcactttacagccatgcatgctgatgccttccatcttgacaaatggaatgatgggtaaacactcctgacacaaagaggaacaccttcctcgtcccttgctgaaacaaagtgcaatgcacacagtagaatttagtttgcttgcactggaagatgccgttgaagaggtaggctgaggaacactgtatcctagggagaaaatatgcaagtctcacgggtgctttctgttggcttgtttctggtccttgagcaggcttaagtatctagtttcaaactagaagccccaaagccctcagtcgttgtcctggacagagttggtagaccccacctgtagaaatccagatgcactctgggattggagcacagagaggcttgctctatcgtgagaatgcccagcctgcagaggcccaggtgcggtgcctgagtggctgtatgccagacacaggaacgccagcaggctgagtgtggtgactgatatgtgaggtgcccttgccctgcagacaggctgaatgtgagccccagcagcagaggattctgagagtcagggtggtgtcatgtcctacacaggaagagccttcaatattactttttaaacgaactttcccattgctgatattttgataaaaacccacacaaggtttaattacatgccccctcatccctctccacacagtcttgcccatcccactggtgaattgttgttgttcttgttgttgttttttgttattggtgaaaattgtgaaattgttaaggtctctgtttttgttatttatctccctaaatcacatggctgctgcatacattgcaatgttgccctaccacatgtatgtttttgcaagttgcttcttcactcattgaagaagcctgcaccgtaagtgaaactcacttagtccttgctaattgctgctcactgtcacgtgaacgcagagaaggctgattttcctggacccattttcagtgctttgaggaacatgagtccagagtatattgaagtagaagacagtgtttggcaagccagttcttattagacactgctacaggcttcacaatcttcaaggtggacccacctcatgtggaagggcatcattgcccctctgctcccatgcgctgtgcacccccttcacagtgaaagacctgctggggaccaggactcagagatctctggcttcgagctcatatcttggcttcctgtcatgtctaagcccgacaggaaagtgtggcaccatcctgcctgcggcgttggatggataggccatggattttgctgtaaacttgcttcacaaggaaagctgtgtgttttaaaatatttgataaataaaggatttctagaaagattg

SEQ ID NO: 11 - DNA, 4978 bp, Homo sapiens
  Human STAT3 (NM_139276.2)
ggtttccggagctgcggcggcgcagactgggagggggagccgggggttccgacgtcgcagccgagggaacaagccccaaccggatcctggacaggcaccccggcttggcgctgtctctccccctcggctcggagaggcccttcggcctgagggagcctcgccgcccgtccccggcacacgcgcagccccggcctctcggcctctgccggagaaacagttgggacccctgattttagcaggatggcccaatggaatcagctacagcagcttgacacacggtacctggagcagctccatcagctctacagtgacagcttcccaatggagctgcggcagtttctggccccttggattgagagtcaagattgggcatatgcggccagcaaagaatcacatgccactttggtgtttcataatctcctgggagagattgaccagcagtatagccgcttcctgcaagagtcgaatgttctctatcagcacaatctacgaagaatcaagcagtttcttcagagcaggtatcttgagaagccaatggagattgcccggattgtggcccggtgcctgtgggaagaatcacgccttctacagactgcagccactgcggcccagcaagggggccaggccaaccaccccacagcagccgtggtgacggagaagcagcagatgctggagcagcaccttcaggatgtccggaagagagtgcaggatctagaacagaaaatgaaagtggtagagaatctccaggatgactttgatttcaactataaaaccctcaagagtcaaggagacatgcaagatctgaatggaaacaaccagtcagtgaccaggcagaagatgcagcagctggaacagatgctcactgcgctggaccagatgcggagaagcatcgtgagtgagctggcggggcttttgtcagcgatggagtacgtgcagaaaactctcacggacgaggagctggctgactggaagaggcggcaacagattgcctgcattggaggcccgcccaacatctgcctagatcggctagaaaactggataacgtcattagcagaatctcaacttcagacccgtcaacaaattaagaaactggaggagttgcagcaaaaagtttcctacaaaggggaccccattgtacagcaccggccgatgctggaggagagaatcgtggagctgtttagaaacttaatgaaaagtgcctttgtggtggagcggcagccctgcatgcccatgcatcctgaccggcccctcgtcatcaagaccggcgtccagttcactactaaagtcaggttgctggtcaaattccctgagttgaattatcagcttaaaattaaagtgtgcattgacaaagactctggggacgttgcagctctcagaggatcccggaaatttaacattctgggcacaaacacaaaagtgatgaacatggaagaatccaacaacggcagcctctctgcagaattcaaacacttgaccctgagggagcagagatgtgggaatgggggccgagccaattgtgatgcttccctgattgtgactgaggagctgcacctgatcacctttgagaccgaggtgtatcaccaaggcctcaagattgacctagagacccactccttgccagttgtggtgatctccaacatctgtcagatgccaaatgcctgggcgtccatcctgtggtacaacatgctgaccaacaatcccaagaatgtaaacttttttaccaagcccccaattggaacctgggatcaagtggccgaggtcctgagctggcagttctcctccaccaccaagcgaggactgagcatcgagcagctgactacactggcagagaaactcttgggacctggtgtgaattattcagggtgtcagatcacatgggctaaattttgcaaagaaaacatggctggcaagggcttctccttctgggtctggctggacaatatcattgaccttgtgaaaaagtacatcctggccctttggaacgaagggtacatcatgggctttatcagtaaggagcgggagcgggccatcttgagcactaagcctccaggcaccttcctgctaagattcagtgaaagcagcaaagaaggaggcgtcactttcacttgggtggagaaggacatcagcggtaagacccagatccagtccgtggaaccatacacaaagcagcagctgaacaacatgtcatttgctgaaatcatcatgggctataagatcatggatgctaccaatatcctggtgtctccactggtctatctctatcctgacattcccaaggaggaggcattcggaaagtattgtcggccagagagccaggagcatcctgaagctgacccaggtagcgctgccccatacctgaagaccaagtttatctgtgtgacaccaacgacctgcagcaataccattgacctgccgatgtccccccgcactttagattcattgatgcagtttggaaataatggtgaaggtgctgaaccctcagcaggagggcagtttgagtccctcacctttgacatggagttgacctcggagtgcgctacctcccccatgtgaggagctgagaacggaagctgcagaaagatacgactgaggcgcctacctgcattctgccacccctcacacagccaaaccccagatcatctgaaactactaactttgtggttccagattttttttaatctcctacttctgctatctttgagcaatctgggcacttttaaaaatagagaaatgagtgaatgtgggtgatctgcttttatctaaatgcaaataaggatgtgttctctgagacccatgatcaggggatgtggcggggggtggctagagggagaaaaaggaaatgtcttgtgttgttttgttcccctgccctcctttctcagcagctttttgttattgttgttgttgttcttagacaagtgcctcctggtgcctgcggcatccttctgcctgtttctgtaagcaaatgccacaggccacctatagctacatactcctggcattgcactttttaaccttgctgacatccaaatagaagataggactatctaagccctaggtttctttttaaattaagaaataataacaattaaagggcaaaaaacactgtatcagcatagcctttctgtatttaagaaacttaagcagccgggcatggtggctcacgcctgtaatcccagcactttgggaggccgaggcggatcataaggtcaggagatcaagaccatcctggctaacacggtgaaaccccgtctctactaaaagtacaaaaaattagctgggtgtggtggtgggcgcctgtagtcccagctactcgggaggctgaggcaggagaatcgcttgaacctgagaggcggaggttgcagtgagccaaaattgcaccactgcacactgcactccatcctgggcgacagtctgagactctgtctcaaaaaaaaaaaaaaaaaaaagaaacttcagttaacagcctccttggtgctttaagcattcagcttccttcaggctggtaatttatataatccctgaaacgggcttcaggtcaaacccttaagacatctgaagctgcaacctggcctttggtgttgaaataggaaggtttaaggagaatctaagcattttagacttttttttataaatagacttattttcctttgtaatgtattggccttttagtgagtaaggctgggcagagggtgcttacaaccttgactccctttctccctggacttgatctgctgtttcagaggctaggttgtttctgtgggtgccttatcagggctgggatacttctgattctggcttccttcctgccccaccctcccgaccccagtccccctgatcctgctagaggcatgtctccttgcgtgtctaaaggtccctcatcctgtttgttttaggaatcctggtctcaggacctcatggaagaagagggggagagagttacaggttggacatgatgcacactatggggccccagcgacgtgtctggttgagctcagggaatatggttcttagccagtttcttggtgatatccagtggcacttgtaatggcgtcttcattcagttcatgcagggcaaaggcttactgataaacttgagtctgccctcgtatgagggtgtatacctggcctccctctgaggctggtgactcctccctgctggggccccacaggtgaggcagaacagctagagggcctccccgcctgcccgccttggctggctagctcgcctctcctgtgcgtatgggaacacctagcacgtgctggatgggctgcctctgactcagaggcatggccggatttggcaactcaaaaccaccttgcctcagctgatcagagtttctgtggaattctgtttgttaaatcaaattagctggtctctgaattaagggggagacgaccttctctaagatgaacagggttcgccccagtcctcctgcctggagacagttgatgtgtcatgcagagctcttacttctccagcaacactcttcagtacataataagcttaactgataaacagaatatttagaaaggtgagacttgggcttaccattgggtttaaatcatagggacctagggcgagggttcagggcttctctggagcagatattgtcaagttcatggccttaggtagcatgtatctggtcttaactctgattgtagcaaaagttctgagaggagctgagccctgttgtggcccattaaagaacagggtcctcaggccctgcccgcttcctgtccactgccccctccccatccccagcccagccgagggaatcccgtgggttgcttacctacctataaggtggtttataagctgctgtcctggccactgcattcaaattccaatgtgtacttcatagtgtaaaaatttatattattgtgaggttttttgtcttttttttttttttttttttttggtatattgctgtatctactttaacttccagaaataaacgttatataggaaccgtaaaaa

SEQ ID NO: 12 - DNA, 4520 bp, Mus <mouse, genus>
  Mouse Stat3 (NM_213659.3)
aattatgcatggaggcgtgtcttggccagtggcggctgggtggggattggctggaggggctgtaattcagcggtttccggagctgcagtgtagacagggagggggaacctggggttccgacgtcgcggcggagggaacgagccctaaccggatcgctgaggtacaaccccgctcggtgtcgcctgaccgcgtcggctaggagaggccaggcggccctcgggagcccagcagctcgcgcctggagtcagcgcaggccggccagtcgggcctcagccccggagacagtcgagacccctgactgcagcaggatggctcagtggaaccagctgcagcagctggacacacgctacctggagcagctgcaccagctgtacagcgacagcttccccatggagctgcggcagttcctggcaccttggattgagagtcaagactgggcatatgcagccagcaaagagtcacatgccacgttggtgtttcataatctcttgggtgaaattgaccagcaatatagccgattcctgcaagagtccaatgtcctctatcagcacaaccttcgaagaatcaagcagtttctgcagagcaggtatcttgagaagccaatggaaattgcccggatcgtggcccgatgcctgtgggaagagtctcgcctcctccagacggcagccacggcagcccagcaagggggccaggccaaccacccaacagccgccgtagtgacagagaagcagcagatgttggagcagcatcttcaggatgtccggaagcgagtgcaggatctagaacagaaaatgaaggtggtggagaacctccaggacgactttgatttcaactacaaaaccctcaagagccaaggagacatgcaggatctgaatggaaacaaccagtctgtgaccagacagaagatgcagcagctggaacagatgctcacagccctggaccagatgcggagaagcattgtgagtgagctggcggggctcttgtcagcaatggagtacgtgcagaagacactgactgatgaagagctggctgactggaagaggcggcagcagatcgcgtgcatcggaggccctcccaacatctgcctggaccgtctggaaaactggataacttcattagcagaatctcaacttcagacccgccaacaaattaagaaactggaggagctgcagcagaaagtgtcctacaagggcgaccctatcgtgcagcaccggcccatgctggaggagaggatcgtggagctgttcagaaacttaatgaagagtgccttcgtggtggagcggcagccctgcatgcccatgcacccggaccggcccttagtcatcaagactggtgtccagtttaccacgaaagtcaggttgctggtcaaatttcctgagttgaattatcagcttaaaattaaagtgtgcattgataaagactctggggatgttgctgccctcagagggtctcggaaatttaacattctgggcacgaacacaaaagtgatgaacatggaggagtctaacaacggcagcctgtctgcagagttcaagcacctgacccttagggagcagagatgtgggaatggaggccgtgccaattgtgatgcctccttgatcgtgactgaggagctgcacctgatcaccttcgagactgaggtgtaccaccaaggcctcaagattgacctagagacccactccttgccagttgtggtgatctccaacatctgtcagatgccaaatgcttgggcatcaatcctgtggtataacatgctgaccaataaccccaagaacgtgaacttcttcactaagccgccaattggaacctgggaccaagtggccgaggtgctcagctggcagttctcgtccaccaccaagcgggggctgagcatcgagcagctgacaacgctggctgagaagctcctagggcctggtgtgaactactcagggtgtcagatcacatgggctaaattctgcaaagaaaacatggctggcaagggcttctccttctgggtctggctagacaatatcatcgaccttgtgaaaaagtatatcttggccctttggaatgaagggtacatcatgggtttcatcagcaaggagcgggagcgggccatcctaagcacaaagcccccgggcaccttcctactgcgcttcagcgagagcagcaaagaaggaggggtcactttcacttgggtggaaaaggacatcagtggcaagacccagatccagtctgtagagccatacaccaagcagcagctgaacaacatgtcatttgctgaaatcatcatgggctataagatcatggatgcgaccaacatcctggtgtctccacttgtctacctctaccccgacattcccaaggaggaggcatttggaaagtactgtaggcccgagagccaggagcaccccgaagccgacccaggtagtgctgccccgtacctgaagaccaagttcatctgtgtgacaccaacgacctgcagcaataccattgacctgccgatgtccccccgcactttagattcattgatgcagtttggaaataacggtgaaggtgctgagccctcagcaggagggcagtttgagtcgctcacgtttgacatggatctgacctcggagtgtgctacctcccccatgtgaggagctgaaaccagaagctgcagagacgtgacttgagacacctgccccgtgctccacccctaagcagccgaaccccatatcgtctgaaactcctaactttgtggttccagatttttttttttaatttcctacttctgctatctttgggcaatctgggcactttttaaaatagagaaatgagtgagtgtgggtgataaactgttatgtaaagaggagagcacctctgagtctggggatggggctgagagcagaagggagcaaggggaacacctcctgtcctgcccgcctgccctcctttttcagcagctcggggttggttgttagacaagtgcctcctggtgcccatggcatcctgttgccccactctgtgagctgataccccaggctgggaactcctggctctgcactttcaaccttgctaatatccacatagaagctaggactaagcccagaggttcctctttaaattaaaaaaaaaaaaaataagaattaaagggcaaaacacactgacacagcatagcctttccatatcaaggaatactcagttaacagcctctccagcgctgtcttcaggctgatcatctatataaaccctggaatggttgcagatcaaatctgtaaaagagatccgagagctgtggcttggcctctggttcaaacacaaaggctagagagaacctagatatccctgggttttgtttacccagtatgcttgtcggttggaggtgtgaggtaggccaagggcactggaaagcctttgtcatcaccctactccctccccaacccagactccagaccctgtttcagggtcagcctgccctgtgggtgccttactgggcctagggtcaacctgccttcctttcccacttgaccttgctggtagtatgtccccttcccatgtccaaaggccctctgtcctgcttctattgggaatccctgcctcaggaccttgtgtcgagagggattgccttacaggtttgaacctgcctcagactacaggccctcagcaaagctcagggagtatggtccttattctatgcgcttggttcccagggatatctgtaaccacagggcaaaagctgacatatactccaggtctgccctcatatgagtggtgtattcttggcctcccctgagactggcaactgtctgctccccattgggtctcccaggtgaggtggaacacagttcctgcacctactgtggcctccatgtcgcttgcttgcttcgctcactcagcttactggaacactgagtgttcaaggcaagcctttcctgacagaggcatggctagattcagtgactcaaagccacctcattcagctgatcagtgtctgtggaattgtttccttccagttaaccagtgtctgaattaagggcagtgaggacattgtctccaagacgaactgcttgccttgaccaccccagccttctgcttcgagacagttactgctctcccaccccatcaatgttctttagttatacaataagctgaacttataaactgaaagggtatttaggaaggcaaggcttgggcatttttatggctttcaatcctggggacccaggaacaaggtgagggcttctctggggctggtgttgtacctcaggggctctgggaagtctgtgtgcctgggttaaccacccatagtgagcccctggaactgcccactttccctctccttggccccacttggccccagcctcacccagcctgcagactgcttagcctttcagtgcagtggcttgtgttctggccactgcactcagattccaatgtaaactttctagtgtaaaaatttatattattgtgggttgttttttgttgttgtttgtttttgtatattgctgtaactactttaacttccagaaataaagattatataggaactgtctggc

SEQ ID NO: 13 - DNA, 8332 bp, Homo sapiens
  Human TCF4 (NM_001083962.1)
gtgtgtggatgtgtgagtgagagggaacgagagtaagagaaagaaagaagtgaggggatgtaaactcgaataaatttcaaagtgcctccgagggatgcaacgggcaaaaactgaactgttcaggcttcagattgtaactgacgatctgaggaaaaatgaggtgctcgatgaattttcgtttgtattttttggcgaggcgggggaggtgttgagattttttttttttcccctcggggtgggtgcgagggggatgcatcctagcctgcccgacccggagcaagtcgcgtctccccgccggagcccccccacccatttctttgctgaacttgcaattccgtgcgcctcggcgtgtttccccctccccccttccctccgtcccctcccctccccggagaagagagttggtgttaagagtcagggatcttggctgtgtgtctgcggatctgtagtggcggcggcggcggcggcggcggggaggcagcaggcgcgggagcgggcgcaggagcaggcggcggcggtggcggcggcggttagacatgaacgccgcctcggcgccggcggtgcacggagagccccttctcgcgcgcgggcggtttgtgtgattttgctaaaatgcatcaccaacagcgaatggctgccttagggacggacaaagagctgagtgatttactggatttcagtgcgatgttttcacctcctgtgagcagtgggaaaaatggaccaacttctttggcaagtggacattttactggctcaaatgtagaagacagaagtagctcagggtcctgggggaatggaggacatccaagcccgtccaggaactatggagatgggactccctatgaccacatgaccagcagggaccttgggtcacatgacaatctctctccaccttttgtcaattccagaatacaaagtaaaacagaaaggggctcatactcatcttatgggagagaatcaaacttacagggttgccaccagcagagtctccttggaggtgacatggatatgggcaacccaggaaccctttcgcccaccaaacctggttcccagtactatcagtattctagcaataatccccgaaggaggcctcttcacagtagtgccatggaggtacagacaaagaaagttcgaaaagttcctccaggtttgccatcttcagtctatgctccatcagcaagcactgccgactacaatagggactcgccaggctatccttcctccaaaccagcaaccagcactttccctagctccttcttcatgcaagatggccatcacagcagtgacccttggagctcctccagtgggatgaatcagcctggctatgcaggaatgttgggcaactcttctcatattccacagtccagcagctactgtagcctgcatccacatgaacgtttgagctatccatcacactcctcagcagacatcaattccagtcttcctccgatgtccactttccatcgtagtggtacaaaccattacagcacctcttcctgtacgcctcctgccaacgggacagacagtataatggcaaatagaggaagcggggcagccggcagctcccagactggagatgctctggggaaagcacttgcttcgatctattctccagatcacactaacaacagcttttcatcaaacccttcaactcctgttggctctcctccatctctctcagcaggcacagctgtttggtctagaaatggaggacaggcctcatcgtctcctaattatgaaggacccttacactctttgcaaagccgaattgaagatcgtttagaaagactggatgatgctattcatgttctccggaaccatgcagtgggcccatccacagctatgcctggtggtcatggggacatgcatggaatcattggaccttctcataatggagccatgggtggtctgggctcagggtatggaaccggccttctttcagccaacagacattcactcatggtggggacccatcgtgaagatggcgtggccctgagaggcagccattctcttctgccaaaccaggttccggttccacagcttcctgtccagtctgcgacttcccctgacctgaacccaccccaggacccttacagaggcatgccaccaggactacaggggcagagtgtctcctctggcagctctgagatcaaatccgatgacgagggtgatgagaacctgcaagacacgaaatcttcggaggacaagaaattagatgacgacaagaaggatatcaaatcaattactaggtcaagatctagcaataatgacgatgaggacctgacaccagagcagaaggcagagcgtgagaaggagcggaggatggccaacaatgcccgagagcgtctgcgggtccgtgacatcaacgaggctttcaaagagctcggccgcatggtgcagctccacctcaagagtgacaagccccagaccaagctcctgatcctccaccaggcggtggccgtcatcctcagtctggagcagcaagtccgagaaaggaatctgaatccgaaagctgcgtgtctgaaaagaagggaggaagagaaggtgtcctcagagcctccccctctctccttggccggcccacaccctggaatgggagacgcatcgaatcacatgggacagatgtaaaagggtccaagttgccacattgcttcattaaaacaagagaccacttccttaacagctgtattatcttaaacccacataaacacttctccttaacccccatttttgtaatataagacaagtctgagtagttatgaatcgcagacgcaagaggtttcagcattcccaattatcaaaaaacagaaaaacaaaaaaaagaaagaaaaaagtgcaacttgagggacgactttctttaacatatcattcagaatgtgcaaagcagtatgtacaggctgagacacagcccagagactgaacggcaatctttccacactgtggaacaatgcatttgtgcctaaacttcttttggaaaaaaaaaatataattaatttgtaagtctgaaaaaaaaatatttaatttaaaaaaaattgtaaacttgcaataatgaaaaagtgtacttctgaagaaaactacatgaacgtttttgttggtattcaagtcagctagtgtttataattactggatattgaattaggggaagctcggctgccctagtaacaaaaccagcaaacgtcctgatgacaacgaagtgatgacattagccattccttagggtaggaggaacagatggatcttatagacctatgacaaatatatatataaatatatatataaatatatattaaaaatttagtgactatggtaagcttttgttcatttgtttcagacttttttctcctgtaaaaaaatagtactgattaacttttttaaaagaaagattttactgtaaatatggatttttttttttttggtcttatttctgtccctttccctggtttgttatcgtaacctgtagtgccaactctgcttccagaggggtagtgcaggatgaaatgctgaccctgatgttgcttctcattcataaataagtagaaagttgtttctccagtcttttgggaacacaggacttaaaagtcacatcatgtgtagatattacaagcagcattaccaagacatggcaaaaagagtttgtctgaattgtaatgttgcgtttgtgaacctattctgggattttcagaggtacaaggttagaatgctacaatgttaccactgtgccttccaatgtttatatcatcggaaacataacataatcaaagtggctgtgatttaacaaaatgattaaagtgttacctacctgtgtagccgaagtagtgtgcagtgaggcgtttctgaatacatggtcagatttttggaaaaaaacaaaaacaaaaaaaacaagtaaagttcaaaaaccgtcaaatgagaaaattgcaagtagtgtgacagagctgattgattttgttgctttcttgattttttttttcaaaatgggtttactaaaatgtagatgacttaactgcctcctccttcgtctgaaaaatgccaatattcaatcatcatgcagcattataacaagccttataagtcctaaagcattaagttgcacttttttgaggaggggtagtgcagtatttctctggccagtatgaatgaagtttatacttaccatatttgatagaaacatagatcaagctatggcacagcgactcatcagatagctagctttgacgtctgggcacaattgaaccaacttccatcgtgaatctttataatgattgactttggtgtatagtgcagtaaacaaatagtgctcctagttaagtatttgtcagcatccttttgtctctaacttgtttctatttttacagccacacaattcttggcatgtattaagaaaaaaaaaaatccctgttcaagtagtttttccacctatcagcactgagtaaatgccataaatccattgaaatggtctaaatgttccatctgttctcctgttttgccagttatatagtaatgaaatacatttgtaaattttatgcaacaaatggcaaacgtatcattattttgaaattgtgtatgtaaaagttatatttttacatgtagactcttgttattatgtgttttaatacattgtatcagtttttgtttttttttaaaaactgtggtttaaaaagaagtctcatttaaatgaaatagctacaagaatcagaattttatgttcatttctgaaaatgtaagaacaaataagatagttaccacgtggtcatcttttacaaacccataaacattttgattagctgtgtgtgtgttgaaaaactgtaaatatgttcagtagcgataaaactaaaataactttgatttgttgataagttcctaaaatgtggaggtggattaaaaccttaggagaatagcagaaatcaaacttcatgaaaagttattttggggctttcctgtgaaatgtatgaacaaagaggctcagagaaggacatggaagacaataatgtatactctctcctcctccctgaataatgaaaaccatgtgtatttgttccctccgtatgttaaagatttccttttagtggtacattctgcactcattttgtatagtctaccaaggcgggtatccctaggaacaatattatataggaagcaggtatactctgatcacattcaggataagtgtacagaagaaaatacggtgtttactctttagggaactggaaacactccctgcattgatgtacattttaagaatggcacttttgatacatgttatcataaaggtgcttaatagagctgaattaaagtttttcaaatctgtaaacaaagcaaaaaagtaaattgtagtcatttgattattttttaaattggtgctttatattttgttctcactcagagtaaaagctgcaatttattgttcaccagctttgatgtattcattactcagtaatgcaatacctctattgttgaattccctttggaaataagtgaaaattctaacggccactgaaagctgctcgctaggttttgcttggtggagaaacataatctgcacctatccatattaattgggttgtatccccattaaaaaagaaaaaaagggaatgtggcctttttagtgtgttttttattgttgttgttttgtaattatcaaacccaggtaagatattggtatcctgcactggattttcaaatgaagttcagcagaagacagttaagattaaagtactatacaaaaatttcaaaagggtccatactacgctatctgtatgacgacacttaggctggggatctctttcagaaactcggactttaaaagcaacttggagcagttgatccacctccacattcaagtaatttatgaatatgcagaatagggatctgttcatctagaaatttttaccatttgtcttctgtgtagctgcaaggaacactaatgtttatacaactgtcagtccacccagtggtgcaactggttctgattcagtcttccgattcctttttatttttcactttttcctatttctgaatttttttttttatttgtgatcttgattttgatgaggggttggggagtggggagggagtcgaaccaagacttggagttaagaggattttcatcttttgcatccaacaggcagaatatgatctgtgtccaaaagtgaacttgagtcaggaatgaatcaatttcagcataaacaagcacaaaaatttagtctgctggctgactggaagcaaaaaagtcaagatggaatatgatgaattccaacacaatggggcaccaaggcctttaggcctctctttttattttgctttggttttgtttgtttttctttagagacatgctctttctcatgggacttgaagtggactcatctttgtgcagtgctggttttgccatactcatttcaagtattatagacatatgtaatggtgaaaatatatgaactgtggcctttttcattcttgttacttgtgatgcaattaagtgaagataagaaaaaaaaaaaaaaagcagagatttaccatgtatcagtgcctggctttttgttataaagctttgtttgtctagtgctcttttgctataaaatagactgtagtacaccctagtaggaaaaaaaaaaaactaaatttaaaaataaaaaatatatttggcttatttttcgcaggagcaatccttttataccatgaatattacaaaaaaattgtcagattctgaatatttcttctttgtagatttttggaatcattatgagtaaaagtttgttactttattttactatttaaaagatgttattttaccatgtgttaccaagatgaaactgtatgggtagcttttttgtttgttttttgttttgtttttgtttttgtttttgtttttagttgtaggtcgcagcggggaaattttttgcgactgtacacatagctgcagcattaaaaacttaaaaaaattgttaaaaaaaaaaaaagggaaaacatttcaaaaaaaaaaaaaaagataaacagttacaccttgttttcaatgtgtggctgagtgcctcgattttttcatgtttttggtgtatttctgatttgtagaagtgtccaaacaggttgtgtgctggagttccttcaagacaaaaacaaacccagcttggtcaaggccattacctgtttcccatctgtagttattcgatgaagtcatgtacatgaccgttctgtagcaataaatgtgccatttttataaactgtttctgacacttgtttcatttcattttgcattgtccatatagctatgattctcttctgtaagtaaaacgcatctatatttcattttccaagtgttggaggtattgacagcttaacaaacaaaacatacaaaaaaaatcacaaaaacaaattgaaaagcaaagcacatgattgatcaaggaagagatgcccttaatgaaaatggaacgggatgcatgcaaaacaaaaagaaaactgtctagaggattaactaattgaaggaatataattaatgtgtgtgtaacactgaagctatgcatttgaagagctctgaactgcaccagtgttttcggttgtgctgcaggttgctaagtcaagtcagccttaaccttttgcaccagttggtcggctgtttggcagaacattctcagatcttttcagtcaaaaatctaagatgatttattttgtatcactttgttaaaagctgaatattgttaactacagttaatattaacactgtatttatactttctcaaactacatccgccccaccacttctggttgcctctgttgactattaatccagatgtaaacaaccagatgtttttttctaacttgtacaaactgacgtgtgtcaactatcatggaaggaaaaaaatgtacagattaaaattattcagtgttatgtactgtaagttaatatttttgtagaatggacatcaatctactttgcaaaatttggaggctatttcaacattgcactgtagaaatgtaaagtaatgtatgcaatgtaaaggaaagcccgcggtagctgagcgcttcataacagaatgttctaatcaagtacgtggtatttggggatgtctccaatattgctcttgtattctttctaattgggtttagtgactagttgaaggaaaatgttataacgccatttggttcacatgtgaagtgccctccatagccaaatgttgggatttttttttttttcgtttttggttggactgtttgcagatatttaaattttatgaaatttccaaagattttggttgataacccccttttaccttctaaatgatttgagatgttcttatgttcttactgtgtgttttaaatatatataaaagagccacaagcattt

SEQ ID NO: 14 - DNA, 7462 bp, Mus <mouse, genus>
  Mouse Tcf4 (NM_013685.2)
ggagcagccgcggccgcagcgccttctctttataagccgcagtgcccggatgtgaatggattacaatgtatctttcagggaaacctattattatcaatgtgactcctcgggggagtcaatgatggtgttggggaggaggatgatgatgagacgcctctaaacttggaacaagtttaggactttgaaagagaagagaaaaaaaaatacaaccaacaagaccgaagaacaattataactatccagtgttgattatttttataaacaatacgaaaaagttgtcggatttttttttttaatgattactttttggggggagggaattttgttacagtttgatgatggaaaatgcaaaaaccgagccaggtgcataatcttgtaatctgtggctaaccctggaacaggactgacttctatttaaaatactcttttgggggaacactcatgtgagacactaagttcttgcagaagatttttgtctctctttttaaagtctctttccttggaatattgtgagcatatttgtggccattgaaggtttgtgtgattttgctaaaatgcatcaccaacagcgaatggctgccttagggacggacaaagagctgagtgatttactggatttcagtgcgatgttttcgcctcctgtaagcagtgggaaaaatggaccaacttctttggcgagtggacatttcactggctcaaatgtagaagacagaagtagctcagggtcctggggaactggaggccatccaagcccgtccaggaactatggagatgggactccctatgaccacatgactagcagggatcttgggtcacatgacaatctctctccaccttttgtcaattccagaatacaaagtaaaacagaaaggggctcatactcatcttatgggagagaaaacgttcagggttgccaccagcagagtctcctcggaggggacatggatatgggcaatccaggaaccctttcgcccaccaaacctggctcccagtactatcagtattcaagcaataatgcccgccggaggcctcttcacagtagtgccatggaggtacagacaaagaaagtccgaaaagttcctccgggtttgccgtcttcagtctacgctccttcagccagcactgccgactacaacagggactcgccaggctatccttcctccaagccagcagccagcactttccctagctccttcttcatgcaagatggccatcacagcagcgacccttggagctcctccagcgggatgaatcagcccggctacggagggatgctgggcaattcttctcatatcccacagtccagcagctactgtagcctgcatccacatgaacgtttgagctatccatcccactcctcggcagacatcaactccagtcttcctccgatgtccacgttccatcgtagtggcacaaaccattacagcacctcttcctgcacaccccctgccaacggaacagacagtataatggcaaacagaggaactggggcagcaggcagctcgcagactggagacgctctagggaaagccctagcttcgatctattctcctgaccacacgaacaacagcttttcctccaatccttcaactcctgtgggctcccctccttcactctcagcaggcacagctgtttggtctagaaatggaggacaggcctcgtcatctcccaattatgaaggacccttgcactcactgcaaagccgaatcgaagaccgtttggaaagactggacgatgcgattcatgttctccggaaccacgcagtgggcccgtccacagctgtgcctggtggccatggggacatgcatgggatcatgggaccctcccacaacggagcgatgggtagcctgggctcagggtacggaactagtcttctctcagccaacagacactcgctcatggttggggcccaccgtgaagatggcgtggctctgagaggcagccattctctcctgccaaaccaggttccggtcccacaacttccggtccagtctgcaacttcccctgacttgaacccaccccaagacccttacagagggatgccaccaggcctccagggccagagcgtgtcttctggtagctctgagatcaaatccgacgacgagggcgatgagaacctgcaagacacaaaatcttctgaggacaagaaattagatgacgacaagaaggatatcaaatcaattactaggtcaagatctagcaataacgatgatgaggacctgaccccagagcagaaggctgagcgcgagaaggaacggaggatggccaataatgcccgtgagcgcctgagggtccgagatatcaacgaggctttcaaggagcttggccgtatggtgcagctccacctgaagagcgacaagccccagaccaagctcctgattctccaccaggccgtggctgtcatcctcagcctggagcagcaagttcgagaaaggaatctgaacccgaaagctgcctgtctgaaaagaagggaggaagagaaggtgtcctcagagcctcccccactctccttggctggcccacaccctgggatgggagacgcagcgaatcacatgggacagatgtgaaaaggtccaagttgctaccttgcttcattaaacaagagaccacttccttaacagctgtattaccctaaacccacataaacactgctccttaaccccgtttttttttgtaatataagacaagtctgagtagttatgaatcgcagacgcaagaggtttcagcattcccaattatcaaaaaacagaaaaacaaacaaaaaaatgaatgaaagaaagaaagaaagaaaaaaatgcaacttgagggacgacttctttaacatatcactctgaatgtgcgaagcggtatgtacaggctgagacacagcccagagactgaatggcaatcctcccacactgtggagcaatgcatttgtgcctaaacttcttttggaaaaaaaaaatataattaatttgtaagtctgaaaaaaatatttaatttaaaaaaaaattgtaaacttgcaataatgaaaaagtgtacttctgaagaaaacgacatgaacgtttttgttggtattcacgtcagctagtgtttctaattaccggatattgaataggggaagcccggctgccctcgtaacaaaaccagcaaacgtcctgatggcaacgaagtgatgacattagccattccttagggtaggagggacagatggatgttatagacctatgacaaatatatatataaatatatatataaatatatattaaaaatttagtgactatggtaagcttttgttgatttgtttcagacttttttctcctgtaaaaaaatagtactgattaacttttttaaaagaaagattttactgtaaatatggatttttttttttgtctgatttttgtcccttcccccggtttgttatcgtaacctgtagtgccaactctgcttccggaggggcagtgcaggacgaaatgctgaccctgaagttgcttctcattcacaaatagtaaaaagttgtttctccagtcttttgggaacacaggacttaaaagtcacatcatgtgtaggaattacatgcagcattgcccgggcgaggcaaaaagcgtttgtctggcttgtggcgctgcccttgttaccctcccctgggattttcagaggtacacggttagaatgctacaatgttaccactgtgccttccaatgtttatatcatcggaaacataacataatcaaagtggctgtgatttaacaaaaaaaacgattcaagtgttacctacctgtgtagccgaagtagtgtgcagtgaccgagacgtttctgaatacatggtcagattttttttggaaaaaatacaaaaattaaaaaaaaaaaaaaaaaagaaaaaaagaaaaaaaaactaaaaaagaaagtcaagttcaaaaaccgtcaaatgagaaaattgcaaggagtgtgacagagctgattgatttttgttgctttcttgatttttttttcaaaatgggtttactaaaaagtagatgacttacctgcctcctccttcgtctgaaaaaaaaaaaaaatgccaaccaatcatgcagcattataacaagccttataagccctaaagcattaagttgcacttttgtgaggaggggtaacgcagtattctctctggccagtatgagtgaagtttatacttaacatttgatagaaacatagatcaaactacggcacagcaactcatcagatagctagcgttgactctgggcacaattgaaccaattcccatcgtaagtctttccaacaatggactttggtgtgtagtgcagtgaacacataggactcctacgtaagcatttgtcagcatccttttgtctctaactcggttctgttttgacagccacacaatcttggcatgtattaaggaaaaaaaaaatccctgttgaagtagtttttccacctatcagcactgagtaaatgccataactccgcggaaatggtctaaataccccatttgttgtcctgaactaccagttacatagtgacgaaacacatctgtaaattttatgcaaccaatggcaaacctatcattattttgaaactgtgtatgtaaaagttatatttttacatgtagactcttgttattatgtgttttaatacattgtatcagttttttgtttttttttaaactgtgtggttttaaaaagtcatttaaatgaaatagtgagctacaagaatctgaaatttatgttcatttctgaaaatgtaagaacaaataagatagttaccacgtggtcaccttttacaaacccatgaacattttgattagctgtgtgcatgtgtgtgcgtgtgtgctcttgcgcgtgtgtgtgtgtgtgtgtgtgtgtgtatgtgtgtgtgttgaaaattgtaaatatgttcagtagcgataaaactaaaatgctttgatttgttgagaagttcctaaaatgtggaggtggattgaaaatgtaggggaatagcaggaatcaaatctcataaaaagttcttcggggactttgctgtgatgcggtggcacaaaggtgctccaagaagggcaaagaagaaagacagtaacttcccctcctccctgaacgatggaaaacatgtgtacgtggtctctcaccatgttaaagattttctttccgtgatacattctgcactcattttgtatagtctgccaaggcgggtatccctaggaacaatattattatataggaaacaggtatcgtccgatcacattcaggagaagcgtatagaaaagaatatggtgtttactctttagggaactggaaatcctccccgcattgatggatatcttcagagtggcacttttgatacatgttatcataaaggtgcttactaaagcagaatcaaagtttttcaactctgtaaacaaagcaaaaaattaaatttttaaattaaatcatttgagattttttttttcaattggtgcttttatattttgttctcactcggacagagaaaaagctgcaatttcatgttctcaccagctttgatgtattcattacttggtaatgtaatatggctattgtcaaattccttttggaaataagcaaaagactccccaaaggccagcagcagctgctggctactttctgcttggtgcggaaacctgatctgaccctctttgtagtaatcaggtgtatctccagttttaaaaagaaggagaaaggaaatgtggccgttttaacgtgttggttttgttttgttttgttttgttttgttttccttgttgttattttgtaattatcaaacccaggtaagatattggtattcctgcactggatttttgaaagaaacttagcagaagtcaggattaaaatactacacaaacatttcataagtgttcatcctatactagacatacacgaaggcggtgaggcttaggtgcaggatcggtttaagagactttgaaagcaacttggaacagttgatccacctccacattaaagtaaattatgaatatgcagaattagggatctgtccatcttggagttgttactctttttgtcttctgtatggcagtgatgaacactaatgctttgacagctttcagcccacccagtggtccaactgattccaattcagtcttccgattcctggttttgttttgtctttccactttttttttcctatcttgattttattgttattgttattgttattattattattattattattattaatattcatgatgtttgttttgatgagggattgggaagtgggagggagtcgaactgagactaggggctgagaggatttttttttttccatctttgcatccaacaggcagaatatggtctgtgtccaaaacggaacttaagtcaggaaggaaaccattcagcataaacaagcacaacatgtagtctgccggctgactggaagcataaataaataaataaataacacatacggaggtgaagatggaatgtgctggattccaagacaatggggcaccaaggcctgagggcctcctcttgactttgctttggttatgtttgttttctttagagatgtcttttctcatgggacttgaagtgactcatctctgtgcagtactggtttcgccatatgctcatttcaagtattatagacatatgtaatggtgaaatatatgaactgtggcctttttcattcttgttacttgtgatgcaattaagtgaagataagaaaaaaaaaaagcagagatttaccatgtatcagtgcctggctttttgttataaagcttcgtctgtctagtgctctttttgctataaaaaatagactgtagtacaccctagtaggaaaaaaaaactaaatttaaaaataaaaaaatatatttggcttatttttcgcaggagtaatccttttataccatggatattacaaaaaaaaatgtcagattctgagtatttcttctttgtagatttttggaatcattatgagtaaaagtttgttactttattttgctatttaaaagatgttattttaccatgtgttactgaaaggaaactgtatggtagagcttctgtttgtttttgttttcaggttttttttgtttgtttgtttttagttgtaggtcgcagtatgaactttttttttgtttctcgttatgttttgttttgtttttgcgactgtacacatagctgcagcattaaaaacttttaaaaaattgtttaaaaaaaaagaaaaaaagggaaaacgttttaaaaaaaaagataaacagttacaccttgttttcaatgtgtggctgagtgcctcaattttttcatgtttttggtgtatttctgatttgtagaagtgtccaaacaggttgtgtgccggacttccttcaagaggcccacagcccagcttggtctagacctgttcccatctgtagttactcgatgaagtcatgtacatgaccgttctgtagcaataaatgtgccatttttataaactgtctctgacacttttttcatttcacctctcgtgcacatag

SEQ ID NO: 15 - DNA, 6317 bp, Homo sapiens
  Human IKZF1 (NM_006060.5)
attgtgaaagaaagctgggaagagctccgcggccaagttagcaggacactctaacaagtgactgcgcggcccgcgcccggggcggtgactgcggcaagccccctgggtccccgcgcggcgcatcccagcctgggcgggacgctcggccgcggcgaggcgggcaagcctggcagggcagagggagccccggctccgaggttgctcttcgcacccgaggatcagtcttggccccaaagcgcgacgcacaaatccacataacctgaggaccatggatgctgatgagggtcaagacatgtcccaagtttcagggaaggaaagcccccctgtaagcgatactccagatgagggcgatgagcccatgccgatccccgaggacctctccaccacctcgggaggacagcaaagctccaagagtgacagagtcgtggccagtaatgttaaagtagagactcagagtgatgaagagaatgggcgtgcctgtgaaatgaatggggaagaatgtgcggaggatttacgaatgcttgatgcctcgggagagaaaatgaatggctcccacagggaccaaggcagctcggctttgtcgggagttggaggcattcgacttcctaacggaaaactaaagtgtgatatctgtgggatcatttgcatcgggcccaatgtgctcatggttcacaaaagaagccacactggagaacggcccttccagtgcaatcagtgcggggcctcattcacccagaagggcaacctgctccggcacatcaagctgcattccggggagaagcccttcaaatgccacctctgcaactacgcctgccgccggagggacgccctcactggccacctgaggacgcactccgttggtaaacctcacaaatgtggatattgtggccgaagctataaacagcgaagctctttagaggaacataaagagcgctgccacaactacttggaaagcatgggccttccgggcacactgtacccagtcattaaagaagaaactaatcacagtgaaatggcagaagacctgtgcaagataggatcagagagatctctcgtgctggacagactagcaagtaacgtcgccaaacgtaagagctctatgcctcagaaatttcttggggacaagggcctgtccgacacgccctacgacagcagcgccagctacgagaaggagaacgaaatgatgaagtcccacgtgatggaccaagccatcaacaacgccatcaactacctgggggccgagtccctgcgcccgctggtgcagacgcccccgggcggttccgaggtggtcccggtcatcagcccgatgtaccagctgcacaagccgctcgcggagggcaccccgcgctccaaccactcggcccaggacagcgccgtggagaacctgctgctgctctccaaggccaagttggtgccctcggagcgcgaggcgtccccgagcaacagctgccaagactccacggacaccgagagcaacaacgaggagcagcgcagcggtctcatctacctgaccaaccacatcgccccgcacgcgcgcaacgggctgtcgctcaaggaggagcaccgcgcctacgacctgctgcgcgccgcctccgagaactcgcaggacgcgctccgcgtggtcagcaccagcggggagcagatgaaggtgtacaagtgcgaacactgccgggtgctcttcctggatcacgtcatgtacaccatccacatgggctgccacggcttccgtgatccttttgagtgcaacatgtgcggctaccacagccaggaccggtacgagttctcgtcgcacataacgcgaggggagcaccgcttccacatgagctaaagccctcccgcgcccccaccccagaccccgagccaccccaggaaaagcacaaggactgccgccttctcgctcccgccagcagcatagactggactggaccagacaatgttgtgtttggatttgtaactgttttttgttttttgtttgagttggttgattggggtttgatttgcttttgaaaagatttttatttttagaggcagggctgcattgggagcatccagaactgctaccttcctagatgtttccccagaccgctggctgagattccctcacctgtcgcttcctagaatccccttctccaaacgattagtctaaattttcagagagaaatagataaaacacgccacagcctgggaaggagcgtgctctaccctgtgctaagcacggggttcgcgcaccaggtgtctttttccagtccccagaagcagagagcacagcccctgctgtgtgggtctgcaggtgagcagacaggacaggtgtgccgccacccaagtgccaagacacagcagggccaacaacctgtgcccaggccagcttcgagctacatgcatctagggcggagaggctgcacttgtgagagaaaatactatttcaagtcatattctgcgtaggaaaatgaattggttggggaaagtcgtgtctgtcagactgccctgggtggagggagacgccgggctagagcctttgggatcgtcctggattcactggctttgcggaggctgctcagatggcctgagcctcccgaggcttgctgccccgtaggaggagactgtcttcccgtgggcatatctggggagccctgttccccgctttttcactcccatacctttaatggcccccaaaatctgtcactacaatttaaacaccagtcccgaaatttggatcttctttctttttgaatctctcaaacggcaacattcctcagaaaccaaagctttatttcaaatctcttccttccctggctggttccatctagtaccagaggcctcttttcctgaagaaatccaatcctagccctcattttaattatgtacatctgtttgtagccacaagcctgaatttctcagtgttggtaagtttctttacctaccctcactatatattattctcgttttaaaacccataaaggagtgatttagaacagtcattaattttcaactcaatgaaatatgtgaagcccagcatctctgttgctaacacacagagctcacctgtttgaaaccaagctttcaaacatgttgaagctctttactgtaaaggcaagccagcatgtgtgtccacacatacataggatggctggctctgcacctgtaggatattggaatgcacagggcaattgagggactgagccagaccttcggagagtaatgccaccagatcccctaggaaagaggaggcaaatggcactgcaggtgagaaccccgcccatccgtgctatgacatggaggcactgaagcccgaggaaggtgtgtggagattctaatcccaacaagcaagggtctccttcaagattaatgctatcaatcattaaggtcattactctcaaccacctaggcaatgaagaatataccatttcaaatatttacagtacttgtcttcaccaacactgtcccaaggtgaaatgaagcaacagagaggaaattgtacataagtacctcagcatttaatccaaacaggggttcttagtctcagcactatgacattttgggctgactacttatttgttaggcgggagctctcctgtgcattgtaggataattagcagtatccctggtggctacccaatagacgccagtagcaccccgaattgacaacccaaactctccagacatcaccaactgtcccctgcgaggagaaatcactcctgggggagaaccactgacccaaatgaattctaaaccaatcaaatgtctgggaagccctccaagaaaaaaaatagaaaagcacttgaagaatattcccaatattcccggtcagcagtatcaaggctgacttgtgttcatgtggagtcattataaattctataaatcaattattccccttcggtcttaaaaatatatttcctcataaacatttgagttttgttgaaaagatggagtttacaaagataccattcttgagtcatggatttctctgctcacagaagggtgtggcatttggaaacgggaataaacaaaattgctgcaccaatgcactgagtgaaggaagagagacagaggatcaagggctttagacagcactccttcaatatgcaatcacagagaaagatgcgccttatccaagttaatatctctaaggtgagagccttcttagagtcagtttgttgcaaatttcacctactctgttcttttccatccatccccctgagtcagttggttgaagggagttattttttcaagtggaattcaaacaaagctcaaaccagaactgtaaatagtgattgcaggaattcttttctaaactgctttgccctttcctctcactgccttttatagccaatataaatgtctctttgcacaccttttgttgtggttttatattgtaacaccatttttctttgaaactattgtatttaaagtaaggtttcatattatgtcagcaagtaattaacttatgtttaaaaggtggccatatcatgtaccaaaagttgctgaagtttctcttctagctggtaaagtaggagtttgcatgacttcacactttttttgcgtagtttcttctgttgtatgatggcgtgagtgtgtgtcttgggtaccgctgtgtactactgtgtgcctagattccatgcactctcgttgtgtttgaagtaaatattggagaccggagggtaacaggttggcctgttgattacagctagtaatcgctgtgtcttgttccgccccctccctgacaccccagcttcccaggatgtggaaagcctggatctcagctccttgccccatatcccttctgtaatttgtacctaaagagtgtgattatcctaattcaagagtcactaaaactcatcacattatcattgcatatcagcaaagggtaaagtcctagcaccaattgcttcacataccagcatgttccatttccaatttagaattagccacataataaaatcttagaatcttccttgagaaagagctgcctgagatgtagttttgttatatggttccccaccgaccatttttgtgcttttttcttgttttgttttgttttgactgcactgtgagttttgtagtgtcctcttcttgccaaaacaaacgcgagatgaactggacttatgtagacaaatcgtgatgccagtgtatccttcctttcttcagttccagcaataatgaatggtcaacttttttaaaatctagatctctctcattcatttcaatgtatttttactttaagatgaaccaaaattattagacttatttaagatgtacaggcatcagaaaaaagaagcacataatgcttttggtgcgatggcactcactgtgaacatgtgtaaccacatattaatatgcaatattgtttccaatactttctaatacagttttttataatgttgtgtgtggtgattgttcaggtcgaatctgttgtatccagtacagctttaggtcttcagctgcccttctggcgagtacatgcacaggattgtaaatgagaaatgcagtcatatttccagtctgcctctatgatgatgttaaattattgctgtttagctgtgaacaagggatgtaccactggaggaatagagtatccttttgtacacattttgaaatgcttcttctgtagtgatagaacaaataaatgcaacgaatactctgtctgccctatcccgtgaagtccacactggcgtaagagaaggcccagcagagcaggaatctgcctagactttctcccaatgagatcccaatatgagagggagaagagatgggcctcaggacagctgcaataccacttgggaacacatgtggtgtcttgatgtggccagcgcagcagttcagcacaacgtacctcccatctacaacagtgctggacgtgggaattctaagtcccagtcttgagggtgggtggagatggagggcaacaagagatacatttccagttctccactgcagcatgcttcagtcattctgtgagtggccgggcccagggccctcacaatttcactaccttgtcttttacatagtcataagaattatcctcaacatagccttttgacgctgtaaatcttgagtattcatttacccttttctgatctcctggaaacagctgcctgcctgcattgcacttctcttcccgaggagtggggtaaatttaaaagtcaagttatagtttggatgttagtatagaattttgaaattgggaattaaaaatcaggactggggactgggagaccaaaaatttctgatcccatttctgatggatgtgtcacaccttttctgtcaaaataaaatgtcttggaggttatgactccttggtgaaaaaaaaaaaaaaaaaa

SEQ ID NO: 16 - DNA, 5451 bp, Mus <mouse, genus>
  Mouse Ikzf1 (NM_001025597.2)
gtcagggtcccgaagccgcgtgccgtgcgcgcaggccgggtgggctgtgggacaagccgagcgggaggcgagtcgcaagcgccaacccaaagtttgcacggtgcggggcgaggggcgcgcgctccgggctgccgcaggtggcggcgcggtgagcccgggccaggtgccccggcagcggggcggcgctgtcgtgcgggacagccgggctgccaggggctcggagccgggtcggagcccgcggggggcggggagtgtggcgagaaatggggaacaatgcgagtgagcaacttgaggaagtcattgtgaaagaaagctgggaattgctccgcagccaacttagcagggcactctaacaagtgcctgcgcggccgcgcccgggccggggacaggggcagcccggcgcagtacagcccatcccgggacgctcggccgcggctgccggagacccggtaggtcccgcggggtgcaggagcccccagatccccggctgctcttcgcgccccaggatcattcttggcccccaaagcgcggcgcacaaatccacataacctgaagacaatggatgtcgatgagggtcaagacatgtcccaagtttcaggaaaggagagccccccagtcagtgacactccagatgaaggggatgagcccatgcctgtccctgaggacctgtccactacctctggagcacagcagaactccaagagtgatcgaggcatggccagtaatgttaaagtagagactcagagtgatgaagagaatgggcgtgcctgtgaaatgaatggggaagaatgtgcagaggatttacgaatgcttgatgcctcgggagagaaaatgaatggctcccacagggaccaaggcagctcggctttgtcaggagttggaggcattcgacttcctaacggaaaactaaagtgtgatatctgtgggatcgtttgcatcgggcccaatgtgctcatggttcacaaaagaagtcatactggtgaacggcctttccagtgcaaccagtgtggggcctcctttacccagaaaggcaacctcctgcggcacatcaagctgcactcgggtgagaagcccttcaaatgccatctttgcaactatgcctgccgccggagggacgccctcaccggccacctgaggacgcactccgttggtaagcctcacaaatgtggatattgtggccggagctataaacagcgaagctctttagaggagcataaagagcgatgccacaactacttggaaagcatgggccttccgggcatgtacccagtcattaaggaagaaactaaccacaacgagatggcagaagacctgtgcaagataggagcagagaggtcccttgtcctggacaggctggcaagcaatgtcgccaaacgtaagagctctatgcctcagaaatttcttggagacaagtgcctgtcagacatgccctatgacagtgccaactatgagaaggaggatatgatgacatcccacgtgatggaccaggccatcaacaatgccatcaactacctgggggctgagtccctgcgcccattggtgcagacaccccccggtagctccgaggtggtgccagtcatcagctccatgtaccagctgcacaagcccccctcagatggccccccacggtccaaccattcagcacaggacgccgtggataacttgctgctgctgtccaaggccaagtctgtgtcatcggagcgagaggcctccccgagcaacagctgccaagactccacagatacagagagcaacgcggaggaacagcgcagcggccttatctacctaaccaaccacatcaacccgcatgcacgcaatgggctggctctcaaggaggagcagcgcgcctacgaggtgctgagggcggcctcagagaactcgcaggatgccttccgtgtggtcagcacgagtggcgagcagctgaaggtgtacaagtgcgaacactgccgcgtgctcttcctggatcacgtcatgtataccattcacatgggctgccatggctttcgggatccctttgagtgtaacatgtgtggttatcacagccaggacaggtacgagttctcatcccatatcacgcggggggagcatcgttaccacctgagctaaacccagccaggccccactgaagcacaaagatagctggttatgcctccttcccggcagctggacccacagcggacaatgttgggagtggatttgcaggcagcatttgttcttttatgttggttgtttggcgtttgatttgcgttggaagataagtttttaatgttagtgacaggattgcattgcatcaggaacattcacaacatccatccttctagccagttttgttcactggtagctgaggtttcccggatatgtggcttcctaacactctccccacccaccccaccccccaaaacagagcctgaatcttcatgaagtgaataaaacaattatccaagaaggagtaaggtggatcttgccctaagcagagtttatgccacaaagattctccaaatcccccaagacagcacagccactggggttgagccatctcagggagctctgcaggtgagccagaggaccagatataaggcagctggggaggagcagggacatcagcctgtgcagagaccaaggccaaaggttgaactttgaaagactattaagtcatatattgtatggcaatatggtgtctggacaagttgtgcaatgtgctgaagggaagggattggagagccttgaagactcttcttcatttgcctgatcaacccgacctccagagggtttgttgcccagtaagacgagctcagtgctcttgtgatcatttttctcttatcgtttccatgccgttgatggccctgaagctcatcactgcattttagaacccaatcctgaaattgggaccttttttttaaacttctgatactgtaaaacttcttggaagccaaagctttcttccaagccccatcctcagttatcctggttcctgttcttccccgagctgatagtaccaggacctgttattccacaaaagcacaggcatccgtcacttcaattcaatccctgttcagattatagatatggactttgctatcttgataaatgtcttctctatgttattttgtctgaaaaacctataaaaccattattaagaatgaccatttttagatggaagaaatgagcccagcatctcagtggctaaaacacaaaatatccatgcttttaaacaaaattgttaaatattccgaagctctctagtataaacaccaagtagcatgtgttttcacataaagaagacaggggccatgcaacctttatcaagtggaggtattagaatgttgtaatgtttggagacacagtgtgaccagtacaggttcccagagaggaatgcccaccatatcacagaaaggtagaggtgggatctggtatagccagaccaagacagggatgtcacgctgaagccaagtcagttagctgaagattctcaacaggaaggcctctcttaagagtcagtaatagggttgttaccatccaccacctcaacaaaacaaaaagcttataattgtaaatgtttacagcactgtcttcgcagaaactttctgaggtgattccaaagaactagaggggagatggtctataacagctcttgaagtaaacgaggttcttagtctcagctctcctgacatatagggcttgatcattactggtagggattgttctgtgaattgcttactactacccctggtctctccccagtagatgccaggaacattctagctgatacctaactgtcttcccaggtgttcgagggagcaaaccactgatctaaactctaaacgctgaagtacgcaggttttctaaaaatgacaagcccttgaaacctttcccagtaggcagcctcgagctggacttgtgtctttggaatgctgatgaattctatagatcagcattgcaaatacacttcaaatacgtctgagttcaagtgcagggactgagttcaccaaggtgtgaaatgtgctcaaaaagttcaaaagtgtgtgtttctttgtttctaaaacattgtggcatctttttcatttgtttctaaaactttttttttagaaacaaatgaagcacttggaaagtgaaagtaaaattacaaatataaggatttacactgaagagagaaaaattttaggaactatagctgtgaaaagattttgttcaaaaggcaggctagccttacccaaattcatatatggcaggtgtcaacctcccaagcttacagttagcaggcagcttttgctcactcatccttagccatgagagccattaagtgtggtccaagaaagatggctccaaaccctacccccgacccaccagtggtattcagagattaaagcagaattgtaaatagtggcttcaggagctcttttttagaatgctttgccccttcctctcactgccttttttagccaatataaatgtcaatttgcacaccttttgttgtggttttatattgtaacagcatttttttgaaactattgtatttaagataaggtttcatattatgtccacaagtaattaaattatgtttgaaggtggctatatgctgtatcagaagttgatgatgtttttctttagctggtaaaggagggttttgcatgacctcactgtttgttctgtggtttgttctgttgtatgatgtgtgtcttgagttttgctgtgtgatgaagtgcgctgagattccagtgccctcaagttgtgttttaagtagctatcagaggcaagagggttcctaagagcaggttgacctgttggcgacagatggcaatcaccatttctcattccttcttctccctgttaccccagcttcctgtcccaggtcccttctgtgattcttaccttagtgtgcatgtgtgtctgtcctggtgagagtcaggagcatcgatatgttatcattgcattatcaccaagggcacgcacagcctagcacctgttgcttcagataccgtcacactctgtttccaatttagatacaaccacataataaaatgttagagtcttcaatgggaagcagaggtgcttgttataaagatgggggcttatgcttgtgtcacattttgtgttcttttcttcttttgtttggttttaacttaattgtgacccttgtaacatcatcttgccaaaaaaaaaaaaaaagttgaactggatttatgtagacatgtcaagacgtactatctatttctttgtcagttatagcaataagagtggataaactctaaaatccagatctcccacaatgaacatccgtgttctttctatgatttttctttctttatggtgagccacaattaaacttgagatgtacagccacccaaacccaggaagctcatgtgcatctggtgctatggcactcactgtgaataagtgtgaccagatattaatatgcaatattgtttccaatcctttctaatacattttttc

SEQ ID NO: 17 - DNA, 1402 bp, Homo sapiens
  Human ID2 (NM_002166.4)
ggggacgaagggaagctccagcgtgtggccccggcgagtgcggataaaagccgccccgccgggctcgggcttcattctgagccgagcccggtgccaagcgcagctagctcagcaggcggcagcggcggcctgagcttcagggcagccagctccctcccggtctcgccttccctcgcggtcagcatgaaagccttcagtcccgtgaggtccgttaggaaaaacagcctgtcggaccacagcctgggcatctcccggagcaaaacccctgtggacgacccgatgagcctgctatacaacatgaacgactgctactccaagctcaaggagctggtgcccagcatcccccagaacaagaaggtgagcaagatggaaatcctgcagcacgtcatcgactacatcttggacctgcagatcgccctggactcgcatcccactattgtcagcctgcatcaccagagacccgggcagaaccaggcgtccaggacgccgctgaccaccctcaacacggatatcagcatcctgtccttgcaggcttctgaattcccttctgagttaatgtcaaatgacagcaaagcactgtgtggctgaataagcggtgttcatgatttcttttattctttgcacaacaacaacaacaacaaattcacggaatcttttaagtgctgaacttatttttcaaccatttcacaaggaggacaagttgaatggacctttttaaaaagaaaaaaaaaatggaaggaaaactaagaatgatcatcttcccagggtgttctcttacttggactgtgatattcgttatttatgaaaaagacttttaaatgccctttctgcagttggaaggttttctttatatactattcccaccatggggagcgaaaacgttaaaatcacaaggaattgcccaatctaagcagactttgccttttttcaaaggtggagcgtgaataccagaaggatccagtattcagtcacttaaatgaagtcttttggtcagaaattacctttttgacacaagcctactgaatgctgtgtatatatttatatataaatatatctatttgagtgaaaccttgtgaactctttaattagagttttcttgtatagtggcagagatgtctatttctgcattcaaaagtgtaatgatgtacttattcatgctaaactttttataaaagtttagttgtaaacttaacccttttatacaaaataaatcaagtgtgtttattgaatggtgattgcctgctttatttcagaggaccagtgctttgatttttattatgctatgttataactgaacccaaataaatacaagttcaaatttatgtagactgtataagattataataaaacatgtctgaagtcaaaaaaaaaaaaaaaaaaaaaaaaaaaaaaaaaaaaaaaa

SEQ ID NO: 18 - DNA, 1289 bp, Mus <mouse, genus>
  Mouse Id2 (NM_010496.3)
tcattctgaaccgagcctggtgccgcgcagtcagctcagccccctgtggcggctccctcccggtcttcctcctacgagcagcatgaaagccttcagtccggtgaggtccgttaggaaaaacagcctgtcggaccacagcttgggcatctcccggagcaaaaccccggtggacgacccgatgagtctgctctacaacatgaacgactgctactccaagctcaaggaactggtgcccagcatcccccagaacaagaaggtgaccaagatggaaatcctgcagcacgtcatcgattacatcttggacctgcagatcgccctggactcgcatcccactatcgtcagcctgcatcaccagagacctggacagaaccaggcgtccaggacgccgctgaccaccctgaacacggacatcagcatcctgtccttgcaggcatctgaattcccttctgagcttatgtcgaatgatagcaaagtactctgtggctaaataaatggcatttggggacttttttttttctttttactttctctttttcttttgcacaagaagaagtctacaagatcttttaagacttttgttatcagccatttcaccaggagaacacgttgaatggacctttttaaaaagaaagcggaaggaaaactaaggatgatcgtcttgcccaggtgtcgttctccggcctggactgtgataccgttatttatgagagactttcagtgccctttctacagttggaaggttttctttatatactattcccaccatggggagcgaaaacgttaaaaaaaaaagaaaaaaatcacaaggaattgcccaatgtaagcagactttgccttttcacaaaggtggagcgtgaataccagaaggacccagtattcggttacttaaatgaagtcttcggtcagaaatggcctttttgacacgagcctactgaatgctgtgtatatatttatatataaatatatatatattgagtgaaccttgtggactctttaattagagttttcttgtatagtggcagaaataacctatttctgcattaaaatgtaatgacgtacttatgctaaactttttataaaagtttagttgtaaacttaacccttttatacaaaataaatcaagtgtgtttattgaatgttgattgcttgctttatttcagacaaccagtgctttgattttttttatgctatgttataactgaacccaaataaataccagttcaaatttatgtagactgtattaagattataataaaatgtgtctgacatcaaaaaaaaaaaaaaaaaaa

SEQ ID NO: 19 - DNA, 5946 bp, Homo sapiens
  Human BCL11A (NM_022893.3)
ttttttttttttttttgcttaaaaaaaagccatgacggctctcccacaattcatcttccctgcgccatctttgtattatttctaatttattttggatgtcaaaaggcactgatgaagatattttctctggagtctccttctttctaacccggctctcccgatgtgaaccgagccgtcgtccgcccgccgccgccgccgccgccgccgccgcccgccccgcagcccaccatgtctcgccgcaagcaaggcaaaccccagcacttaagcaaacgggaattctcgcccgagcctcttgaagccattcttacagatgatgaaccagaccacggcccgttgggagctccagaaggggatcatgacctcctcacctgtgggcagtgccagatgaacttcccattgggggacattcttatttttatcgagcacaaacggaaacaatgcaatggcagcctctgcttagaaaaagctgtggataagccaccttccccttcaccaatcgagatgaaaaaagcatccaatcccgtggaggttggcatccaggtcacgccagaggatgacgattgtttatcaacgtcatctagaggaatttgccccaaacaggaacacatagcagataaacttctgcactggaggggcctctcctcccctcgttctgcacatggagctctaatccccacgcctgggatgagtgcagaatatgccccgcagggtatttgtaaagatgagcccagcagctacacatgtacaacttgcaaacagccattcaccagtgcatggtttctcttgcaacacgcacagaacactcatggattaagaatctacttagaaagcgaacacggaagtcccctgaccccgcgggttggtatcccttcaggactaggtgcagaatgtccttcccagccacctctccatgggattcatattgcagacaataacccctttaacctgctaagaataccaggatcagtatcgagagaggcttccggcctggcagaagggcgctttccacccactccccccctgtttagtccaccaccgagacatcacttggacccccaccgcatagagcgcctgggggcggaagagatggccctggccacccatcacccgagtgcctttgacagggtgctgcggttgaatccaatggctatggagcctcccgccatggatttctctaggagacttagagagctggcagggaacacgtctagcccaccgctgtccccaggccggcccagccctatgcaaaggttactgcaaccattccagccaggtagcaagccgcccttcctggcgacgccccccctccctcctctgcaatccgcccctcctccctcccagcccccggtcaagtccaagtcatgcgagttctgcggcaagacgttcaaatttcagagcaacctggtggtgcaccggcgcagccacacgggcgagaagccctacaagtgcaacctgtgcgaccacgcgtgcacccaggccagcaagctgaagcgccacatgaagacgcacatgcacaaatcgtcccccatgacggtcaagtccgacgacggtctctccaccgccagctccccggaacccggcaccagcgacttggtgggcagcgccagcagcgcgctcaagtccgtggtggccaagttcaagagcgagaacgaccccaacctgatcccggagaacggggacgaggaggaagaggaggacgacgaggaagaggaagaagaggaggaagaggaggaggaggagctgacggagagcgagagggtggactacggcttcgggctgagcctggaggcggcgcgccaccacgagaacagctcgcggggcgcggtcgtgggcgtgggcgacgagagccgcgccctgcccgacgtcatgcagggcatggtgctcagctccatgcagcacttcagcgaggccttccaccaggtcctgggcgagaagcataagcgcggccacctggccgaggccgagggccacagggacacttgcgacgaagactcggtggccggcgagtcggaccgcatagacgatggcactgttaatggccgcggctgctccccgggcgagtcggcctcggggggcctgtccaaaaagctgctgctgggcagccccagctcgctgagccccttctctaagcgcatcaagctcgagaaggagttcgacctgcccccggccgcgatgcccaacacggagaacgtgtactcgcagtggctcgccggctacgcggcctccaggcagctcaaagatcccttccttagcttcggagactccagacaatcgccttttgcctcctcgtcggagcactcctcggagaacgggagtttgcgcttctccacaccgcccggggagctggacggagggatctcggggcgcagcggcacgggaagtggagggagcacgccccatattagtggtccgggcccgggcaggcccagctcaaaagagggcagacgcagcgacacttgtgagtactgtgggaaagtcttcaagaactgtagcaatctcactgtccacaggagaagccacacgggcgaaaggccttataaatgcgagctgtgcaactatgcctgtgcccagagtagcaagctcaccaggcacatgaaaacgcatggccaggtggggaaggacgtttacaaatgtgaaatttgtaagatgccttttagcgtgtacagtaccctggagaaacacatgaaaaaatggcacagtgatcgagtgttgaataatgatataaaaactgaatagaggtatattaatacccctccctcactcccacctgacaccccctttttcaccactccccttccccatcgccctccagccccactccctgtaggatttttttctagtcccatgtgatttaaacaaacaaacaaacaaacagaagtaacgaagctaagaatatgagagtgcttgtcaccagcacacctgttttttttctttttctttttcttttttctttttccttttttttttttttcctttatgttctcaccgtttgaatgcatgatctgtatggggcaatactattgcattttacgcaaactttgagcctttctcttgtgcaataatttacatgttgtgtatgtttttttttaaacttagacagcatgtatggtatgttatggctattttaaattgtccctaattcgttgctgagcaaacatgttgctgtttccagttccgttctgagagaaaaagagagagagagagaaaaagaccatgctgcatacattctgtaatacatatcatgtacagttttattttataacgtgaggaggaaaaacagtctttggattaaccctctatagacagaatagatagcactgaaaaaaaatctctatgagctaaatgtctgtctctaaagggttaaatgtatcaattggaaaggaagaaaaaaggccttgaattgacaaattaacagaaaaacagaacaagtttattctatcatttggttttaaaatatgagtgccttggatctattaaaaccacatcgatggttctttctacttgttataaacttgtagcttaattcagcattgggtgaggtaataaaccttaggaactagcatataattctatattgtatttctcacaacaatggctacctaaaaagatgacccattatgtcctagttaatcatcatttttcctttagtttaattttataaacaaaactgattataccagtataaaagctactttgctcctggtgagagcttaaaagaaatgggctgttttgcccaaagttttattttttttaaacaatgattaaattgaatgtgtaatgtgcaaaagccctggaacgcaattaaatacactagtaaggagttcattttatgaagatatttgctttaataatgtctttttaaaaatactggcaccaaaagaaatagatccagatctacttggttgtcaagtggacaatcaaatgataaactttaagaccttgtataccatattgaaaggaagaggctgacaataaggtttgacagaggggaacagaagaaaataatatgatttattagcacaacgtggtactatttgccatttaaaactagaacaggtatataagctaatattgatacaatgatgattaactatgaattcttaagacttgcatttaaatgtgacattcttaaaaaaagaagagaaagaattttaagagtagcagtatatatgtctgtgctccctaaaagttgtacttcatttcttttccatacactgtgtgctatttgtgttaacatggaagaggattcattgtttttatttttatttttttaattttttcttttttattaagctagcatctgccccagttggtgttcaaatagcacttgactctgcctgtgatatctgtatcttttctctaatcagagatacagaggttgagtataaaataaacctgctcagataggacaattaagtgcactgtacaattttcccagtttacaggtctatacttaagggaaaagttgcaagaatgctgaaaaaaaattgaacacaatctcattgaggagcattttttaaaaactaaaaaaaaaaaaactttgccagccatttacttgactattgagcttacttacttggacgcaacattgcaagcgctgtgaatggaaacagaatacacttaacatagaaatgaatgattgctttcgcttctacagtgcaaggatttttttgtacaaaacttttttaaatataaatgttaagaaaaattttttttaaaaaacacttcattatgtttaggggggaactgcattttagggttccattgtcttggtggtgttacaagacttgttatccatttaaaaatggtagtggaaattctatgccttggatacacaccgctcttcaggttgtaaaaaaaaaaaacatacattggggaaaggtttaagattatatagtacttaaatataggaaaatgcacactcatgttgattcctatgctaaaatacatttatggtcttttttctgtatttctagaatggtatttgaattaaatgttcatctagtgttaggcactatagtatttatattgaagcttgtatttttaactgttgcttgttctcttaaaaggtatcaatgtaccttttttggtagtggaaaaaaaaaagacaggctgccacagtatatttttttaatttggcaggataatatagtgcaaattatttgtatgcttcaaaaaaaaaaaaaagagagaaacaaaaaagtgtgacattacagatgagaagccatataatggcggtttgggggagcctgctagaatgtcacatggatggctgtcataggggttgtacatatccttttttgttcctttttcctgctgccatactgtatgcagtactgcaagctaataacgttggtttgttatgtagtgtgctttttgtccctttccttctatcaccctacattccagcatcttaccttcatatgcagtaaaagaaagaaagaaaaaaaaaggaaaaaaaaaaaaaaaccaatgttttgcagtttttttcattgccaaaaactaaatggtgctttatatttagattggaaagaatttcatatgcaaagcatattaaagagaaagcccgctttagtcaatacttttttgtaaatggcaatgcagaatattttgttattggccttttctattcctgtaatgaaagctgtttgtcgtaacttgaaattttatcttttactatgggagtcactatttattattgcttatgtgccctgttcaaaacagaggcacttaatttgatcttttatttttctttgtttttatttttttttttatttagatgaccaaaggtcattacaacctggctttttattgtatttgtttctggtctttgttaagttctattggaaaaaccactgtctgtgtttttttggcagttgtctgcattaacctgttcatacacccattttgtccctttattgaaaaaataaaaaaaattaaagtaca

SEQ ID NO: 20 - DNA, 3425 bp, Mus <mouse, genus>
  Mouse Bcl11a (NM_016707.3)
gacgttcaagttcgcagggacgtcacgtccgcacttgaacttgcagctcaggggggcttttgccatttttttcatctctctctctccctctatccctcttctctcttcctctctctcttttttttccttaaaaaaaaaaaagccatgacggctctcccacaattcatcttccctgcgccatctttgtattatttctaatttattttggatgtcaaaaggcactgatgaagatattttctctggagtctccttctttctaacccggctctcccgatgtgaaccgagccgtcgtccgcacgccgccgccgccgccgccgcccgccccgcagcccaccatgtctcgccgcaagcaaggcaaaccccagcacttaagcaaacgggaattctcgcccgaacctcttgaagccattcttacagatgatgaaccagaccatggcccgttgggagctccagaaggggaccacgaccttctcacctgtgggcagtgccagatgaatttcccactgggggacattcttatttttatcgagcacaaacggaaacaatgcaatggcagcctctgcttagaaaaaggtgtggataagccgccttccccttctcccatcgagatgaaaaaggcatccaatcctgtggaggttggcatccaggtcacgccagaggatgacgattgtttatcaacgtcatctagaggaatttgccccaaacaggaacacatagcagataaacttctgcactggaggggcctgtcctctcctcggtctgcacacggagctctaatccccacgcccgggatgagtgcagaatatgccccgcagggtatttgtaaagatgagcccagcagctacacatgtacaacttgcaaacagccattcaccagtgcatggtttctcttgcaacacgcacagaacactcatggattaagaatctacttagaaagtgaacacggaagtcccctgaccccgcgggttggtatcccttcaggactaggtgcagaatgtccttcccagccacctctccatgggattcatattgcagacaataacccctttaacctgctaagaataccaggatcagtatcgagagaggcttccggcctggcagaagggcgctttccacccactccccccctgtttagtccaccaccgagacatcacttggacccccaccgcatagagcgcctgggggcggaagagatggccctggccacccatcacccgagtgcctttgacagggtgctgcggttgaatccaatggctatggagcctcccgccatggatttctctaggagacttagagagctggcagggaacacgtctagtccaccgctgtccccaggccggcccagtcctatgcaaaggttactgcaaccattccagccaggtagcaagccacccttcctggcgacgccccccctccctcctctgcaatccgcccctcctccctcccaacccccggtcaagtccaagtcatgcgagttctgcggcaagacgttcaaatttcagagcaacttggtggttcaccgacgcagccatactggtgagaagccctataagtgcaacctgtgcgaccacgcgtgcacacaggccagcaagctgaagcgtcacatgaagacacacatgcacaaatcgtcccccatgacagtcaagtccgacgatggcctctccacagccagctccccggaacctggtaccagcgacctggtgggcagcgccagcagtgcgctcaagtcagtggtggccaagttcaagagtgagaacgaccccaacttgatcccagagaacggggatgaggaggaagaggaggacgacgaggaagaagaagaagaggaggaagaggaggaggaggagctgacggagagcgagagggtggactacggcttcgggctgagcctggaggctgcacgccaccatgagaacagctctcggggcgcagtggtgggcgtgggcgacgagggccgcgccctgcccgatgtcatgcagggcatggtgctcagctccatgcagcacttcagcgaggccttccaccaggtcctgggcgaaaagcataagcgtagccacctggccgaggccgagggccatagggacacttgtgatgaagactcggtggccggtgagtcagaccgcatagacgatggcactgttaatggtcgtggctgctcccccggcgaatcggcttcggggggtctgtccaaaaagctgctgctgggtagccccagctcgctgagccccttctccaagcgcatcaagctggagaaggagtttgacctgcccccggccgcgatgcctaacacggagaacgtgtattcgcagtggctcgctggctatgcggcctccaggcagctcaaagatcccttccttactttcggagactccagacaatcgccttttgcctcctcatcagagcactcctcggagaacgggagcttgcgcttctccacaccgcccggggagctggacggagggatctcagggcgcagcggcacaggaagtggagggagcacgccccatattagtggtccgggcccgggcaggcccagctcaaaagagggcagacgcagcgacacttgtccttcacacacccccgttcggcgtagtaccccgcgagctcaagatgtgtggcagttttcggatggaagctcaagaacccttaagttctgagaaactttgaagcccccaagggcggggcggacatgcgccgcccagccgacgtcaacgtgctccgttatcctgctagattgtgatgttttctgacagtagcctccaagaagacaagagtcctgccgagtcctcccagcctgggcctgcagtgccattttatttatattttttaataaaacgtaaaaacaaaaaaaaccagacccacattggaacagtgaacccgtcccatccagagggccctaggactgccgcagttggagcgacgtccaacccttttgaaaccagccaacctaattacccgtactgtggaaatgagcatgacccctgaccccttgtttctatacattctatgttgtcttttaaaaagtgtgcttaacattgacataataaatgttggagctttaggcggtgtgtgcttgttttttaatttttaatgctcgtaagacaatgtggctgcttcaggctttatgtctgtgtactttttttccttcagaagctcatagggtgagcagaaggaccagactcaagtgccaggcaggagacctagaaaaggaagtaggcttttcagatggcatacattttcaaagaaaatcaaaatgcaaagctaggggataaatcatagtaatatcataattaatgtagtagtattgctgtttattaatgctgacgtgtgtttttcctctctgacttataatttgcataccattaaataatgcataaatatggcacactgaatcctttttcaaatacacgcttttggtgactacc

SEQ ID NO: 21 - DNA, 2297 bp, Homo sapiens
  Human RELB (NM_006509.3)
ggccccgcgccccgcgcagccccgggcgccgcgcgtcctgcccggcctgcggccccagcccttgcgccgctcgtccgacccgcgatcgtccaccagaccgtgcctcccggccgcccggccggcccgcgtgcatgcttcggtctgggccagcctctgggccgtccgtccccactggccgggccatgccgagtcgccgcgtcgccagaccgccggctgcgccggagctgggggccttagggtcccccgacctctcctcactctcgctcgccgtttccaggagcacagatgaattggagatcatcgacgagtacatcaaggagaacggcttcggcctggacgggggacagccgggcccgggcgaggggctgccacgcctggtgtctcgcggggctgcgtccctgagcacggtcaccctgggccctgtggcgcccccagccacgccgccgccttggggctgccccctgggccgactagtgtccccagcgccgggcccgggcccgcagccgcacctggtcatcacggagcagcccaagcagcgcggcatgcgcttccgctacgagtgcgagggccgctcggccggcagcatccttggggagagcagcaccgaggccagcaagacgctgcccgccatcgagctccgggattgtggagggctgcgggaggtggaggtgactgcctgcctggtgtggaaggactggcctcaccgagtccacccccacagcctcgtggggaaagactgcaccgacggcatctgcagggtgcggctccggcctcacgtcagcccccggcacagttttaacaacctgggcatccagtgtgtgaggaagaaggagattgaggctgccattgagcggaagattcaactgggcattgacccctacaacgctgggtccctgaagaaccatcaggaagtagacatgaatgtggtgaggatctgcttccaggcctcatatcgggaccagcagggacagatgcgccggatggatcctgtgctttccgagcccgtctatgacaagaaatccacaaacacatcagagctgcggatttgccgaattaacaaggaaagcgggccgtgcaccggtggcgaggagctctacttgctctgcgacaaggtgcagaaagaggacatatcagtggtgttcagcagggcctcctgggaaggtcgggctgacttctcccaggccgacgtgcaccgccagattgccattgtgttcaagacgccgccctacgaggacctggagattgtcgagcccgtgacagtcaacgtcttcctgcagcggctcaccgatggggtctgcagcgagccattgcctttcacgtacctgcctcgcgaccatgacagctacggcgtggacaagaagcggaaacgggggatgcccgacgtccttggggagctgaacagctctgacccccatggcatcgagagcaaacggcggaagaaaaagccggccatcctggaccacttcctgcccaaccacggctcaggcccgttcctcccgccgtcagccctgctgccagaccctgacttcttctctggcaccgtgtccctgcccggcctggagccccctggcgggcctgacctcctggacgatggctttgcctacgaccctacggcccccacactcttcaccatgctggacctgctgcccccggcaccgccacacgctagcgctgttgtgtgcagcggaggtgccggggccgtggttggggagacccccggccctgaaccactgacactggactcgtaccaggccccgggccccggggatggaggcaccgccagccttgtgggcagcaacatgttccccaatcattaccgcgaggcggcctttgggggcggcctcctatccccggggcctgaagccacgtagccccgcgatgccagaggaggggcactgggtggggagggaggtggaggagccgtgcaatcccaaccaggatgtctagcacccccatccccttggcccttcctcatgcttctgaagtggacatattcagccttggcgagaagctccgttgcacgggtttccccttgagcccattttacagatgaggaaactgagtccggagaggaaaagggacatggctcccgtgcactagcttgttacagctgcctctgtccccacatgtgggggcaccttctccagtaggattcggaaaagattgtacatatgggaggagggggcagattcctggccctccctccccagacttgaaggtggggggtaggttggttgttcagagtcttcccaataaagatgagtttttgagcctccgggaaaaaaaaaaaaaaaaaa

SEQ ID NO: 22 - DNA, 2218 bp, Mus <mouse, genus>
  Mouse RelB (NM_009046.2)
gcccgccgcccgctcggcccggcgccccccgcagccccgggcgccgtgcgtccagcccggccttcggccctagccttgcaccgcttgcccggccggtgatcgtcccagccgaccgggctgtccgactgcccggcttgccctcgtgtgcgctcgccctgagctggccttcgggctgtcggtccctacgggccgggccatgccgagtcgccgcgctgccagagagtccgcgcccgagctaggggccttgggttccagtgacctctcttccctgtcactaacggtctccaggaccacagatgaattggaaatcatcgacgaatacattaaggagaacggctttggcctggacgggacacagctgagtgagatgccgcgcctggtgccccgcgggcccgcctcactgagcagcgtcacgctgggccctgctgcaccaccgcctccggccacgccgtcctggagctgcacactgggcaggctggtgtcacccggcccgtgcccacggccgtacctggtcatcacagagcagccaaagcagcgtggcatgcgcttccgctacgagtgcgagggccgctcggccggcagcatcctcggggagagcagcaccgaagccagcaagaccctgcccgccatcgagcttcgagactgtggcgggctgcgggaggtggaggtgacggcgtgcctggtgtggaaggactggccacaccgggtacacccacatagcctcgtggggaaagactgcacggacggcgtctgcagggtgcggctgcggcctcacgtcagcccccggcacagctttaacaacctgggcatccagtgtgttaggaagaaggaaattgaagctgccattgagcggaagatccagctgggaattgacccctacaatgctggctccctgaagaaccatcaggaggtcgacatgaatgtcgtcaggatctgcttccaggcctcctatcgggaccagcagggacatctgcaccgcatggaccccatcctctctgagcctgtctacgacaagaagtccaccaacacatcggagctgcggatttgccgaatcaacaaggagagcgggccgtgcacaggtggtgaggagctgtacttgctctgtgacaaggtgcaaaaagaggacatatccgtggtgttcagcacagcttcctgggaaggccgtgccgacttctctcaagctgatgtgcaccggcagatcgccattgtgttcaaaacgccaccctacgaggacctggagatctcagagcccgtgactgtcaatgtgttcttgcagcggctcacggatggggtgtgcagcgagccgctgcccttcacgtacctgcctcgggatcatgacagctacggtgtggacaagaagcgaaagcggggactgcctgatgtccttggagagttgagcagctctgatccacatggaatcgagagcaaacgaaggaaaaagaaaccagtgttcttggaccacttcctgcctggccacagctcaggcctgttcctcccaccatcggctctgcagccggcagactctgatttcttccctgcttccatatcccttcctgggctggagcctcctggtggacccgatctcctggacgatggctttgcctatgatccttctgcccccacgctcttcactatgttggacctgctgcccccagcaccaccacttgccagtgctgtggtgggtagcgggggtgcaggggccaccgttgtggagtcttctggcccagagcccctatcactggactcttttgcagcgccgggccccggggatgttggtactgctagccttgtgggcagcaacatgtttcccaaccagtaccgagaggcagctttcgggggtggcctcctatctccagggcctgaagccacgtagcctctgaggtaacagaggaggcactgggtgaggtatgtggtatagcactccattccgaagccaaccttgatcagtcttccagcttcctcatcctgaatcggacatctgcagcgctggtgggaagatggggagcactccggttctctttgagcccattttacagaatgctgagtccgaagaggaaaaggggctcctgcagatggaccccttctcaggacagattctcagagattgtacataggggaggagggagcaggtccccagccttctcccctaatcctgaagaaggcagtggattgttcagttttcccaataaaaattagttttttgaaaaaaaaaaaaaaa

SEQ ID NO: 23 - DNA, 5233 bp, Homo sapiens
  Human ZBTB46 (NM_025224.3)
tgaccttctctcctccctgtgtctttttttttcctttagagatgggggtcttgctctgtcactccagctagagcacagtggtgcaatcggagctcactgactgcagcctgcaactcctgggctcaagtgattctgccgcctcagcctctcaacgtgctgcgattagagagtctgtagaagaggcgacaccagggcttccaaatgaacaaccgaaaggaagatatggaaatcacgtcccactaccggcacctgctgcgggagctcaacgagcagaggcagcacggcgtcctgtgcgacgtctgcgtggtcgtggagggcaaggtcttcaaggcgcacaagaacgtcctgctgggcagcagccgctacttcaagacgctctactgccaggtgcagaagacgtcggagcaggccacggtcacgcacctggacatcgtcacggcccagggcttcaaggccatcatcgacttcatgtactcagcgcacctggcgctcaccagcaggaacgtcatcgaggtgatgtcagccgccagcttcctgcagatgacggacatcgtgcaagcctgccacgacttcatcaaggcggcgctggacatcagcatcaagtcggacgcctcagatgagcttgcggagttcgagatcggcgcctcgtccagcagcagcacggaagctctcatctcggccgtgatggctgggaggagcatctccccgtggctggcacggcgaacgagtcctgccaattcttccggagactcggccatcgccagctgtcacgacggagggagcagctacgggaaagaggatcaggagcccaaggccgatggccctgatgatgtttcttcacagcctctatggcctggagacgtgggctacgggcctctgcgcatcaaggaagagcaggtttcaccgtctcagtacggagggagcgagctgccttctgccaaggacggtgcagtacagaactctttctcagagcagagtgctggtgatgcctggcagcccacgggccgaaggaagaatcggaaaaacaaagagaccgtccggcacatcacacagcaggtggaagatgacagccgggccagctccccggtgccgtccttcctgccgacgtcggggtggccgttcagcagccgagactcaaatgcggacctgtccgtcaccgaagccagcagctccgacagccgaggagagagggccgagctctatgcacaggtggaggagggtctcctgggaggagaagccagctatctgggccctcccctcaccccagagaaggacgacgccctgcatcaggccaccgcggtggccaacctgcgcgcggcgctcatgagtaagaacagcctgctgtcgctgaaggccgacgtgctgggggatgacggctccctgctgttcgagtacctgcccagaggggcccactcgctgtccctgaatgagttcacggtgatcaggaagaagttcaagtgtccgtactgcagcttctcggccatgcaccagtgcatcctcaagcgacacatgcgctcgcacacgggagagcggccctacccctgcgagatctgcgggaagaagttcacgcggcgcgagcacatgaagcgccacacgctggtccacagcaaggacaagaagtatgtgtgcaaggtgtgcagccgcgtcttcatgtccgccgccagcgtgggcatcaggcatggctccaggcgccacggtgtgtgcaccgactgtgctggccgcggcatggccgggcccctggaccatggcggcggaggcggcgagggctctccagaggcgctgttcccaggcgacgggccctatctggaggaccctgaggacccacgaggggaggcggaggagctgggcgaggacgacgagggcctggcccctgaggatgcgctgttggcggacgacaaggatgaggaagactcgccgcggccgcgcagccccccaggaggccctgacaaggacttcgcctggctctcctaggcccgcccgccggcagggtcggtggctgcctcgctccgtccacccgtgtgtgtgtccggtgggtctccactgcggggccagggccacgctcacccctctcgcggcccctcctctgcttccccctgaacccaccccccacggaaaccagccctgcgggctaagcaggtgcgaccccagcaagaggggtgctctgggaccagacatgaagtgagttgggggagggcacagggtgggtttgagtgaagggagagcacggtcctaagtccccagcaggtggtgcgggtgtgtgagtggcccctgtgatggccagcctggcttggacacgtgatgggcctgtggccgggtccagtgggcactgggcggggtggtgtgttcggcccagaggcccctggcctgagcaggtgcagagttttacagacacccggtcagcccggctggagcccgccctcccctcccctagcagccaggtcactgcctgtggctgcagccgtggcccgtggtgcagccgtggcccatggcagcctgtagaatccaggtgcacagagagccctgccaccgtcttacctctgggctttggtgcttaacacacaacacagctgcagaccctgctggaggccgagggctccaggtgctatcttaggtggacacagccctgggggctccttccaggaggggaccctcagccctgtgccccccaccacttcaggccacaccaggttccctctgcaagggcctcggctcagtcgtgtgcacttcctcggagagccttgggctgccacgtccaccccgggctctgcccgtcctgttctgcccatggcccagcccggccgctcctgctgacccctcctggacgggctggagctgggctcctgcctttgctgctaacactggaggcggtgttcctaactgcagtgtgctgcttacacctccccgcgtgggtaaccaaatttttaagtagtcagagacatatcgaggtagttacataaaattattttgtttggcattatttttctcactcgaagaaactatatagggttgtttttcctttagcttgtgctcaagtcctcttgctgtgttttcagaagcactcacatgttctttcttttcctgagtgaaaagcaaaggtcccacggtgtgtgctgtggtgcaccgcctggctttgggggtcccggaggcaggctgcctagactcacagcctcgggaccgttgccacggcctgtcttctcgttcaggcctgcctctgacagcactcaccatgaggacattccatccttcaccccctcctctggcacaggccaccactgcggtgctgtgccttcagatgggaggtgggcgcggtggcctcctccttccctccaggacctgcccgtgtgaagaccccccggagtgctgagcttcagggctgcgtggaaagagtttttactctctttttctagcctgtataccaggcttttccccacattgtcaggtagagcaccagcttccctgaccgctgctgctcggggagggctggggctggccgggggtcctgtggaggagtacatggaggactccaggtacagcgcaggagtcacggcttttgttttttgacattggcccccggttctaccaatgacagggtgccctggctggagctgtcatcacacacacccctcagctcggaggctgtgggctcctcaaagctggagaaagaggccaagatttttctgcacacggagtgtggggataggagccgggccaagcgctggcccctcagcggtgagccctgcccactcttaccgagcaaggtgggtggctctggcacgagtcccccagggggagagcatggctaccagggagctgcagcggagccctccagccctcaccccaggccagccccaccccggcctctttgagaattctcagaactttgtacctttcccctgatttttaaaccctttttctaaacagactgactttcttacaaaatgcatttggaaaccagacctttgctacccaccaatgtctctgggttttgtaccagtccctgctctcaggccaccctgcccaggacccaggcccgcctccccctccacactcaggatgtcctgctccatctggccggctcactccgtgtggcctgcctttgctgaccgttttggggttccccgccggagctacaggggcattttcttccctaaaaccaacagtgtcccactgacctccccaagtgtttgctgcgtggcagatttcctgttcttgttcgcagtttgccgactgaagagtgtgggatttccgaggcccaggtgagcacgtccatctcaggaggcgtggagggaaaagacatgtcatgaagggttttttttatgtgactgatttttttttaaatcgatgttcaaactaataaatatttttttatgaagaggaaaaatgtgtagattacatttcacattttgtatttttgtttgtgtctgtttgtattttggtgtttacaacaccaaagtgggaaatacagtccattggggatggtgttatttgggggcggggagggggcagggacaccacgatttttctgtcaagctctggatcctgaccaggttgtacactggggctctctgagctttgggacacaggacactgccagggctacgtagggaactgactcagaagacgcagcttactgcttccaactttgcacatcttcctctttaaaaaactgagaaaatgcaaaaactggaactttttgcaatattataaaagaagtaatcttattttagctcattctgtgacatgtgcgactcttaagaaagccatacttaatggtggtggttttttttagatcttatattgtgttttgtatgcagcccttttagaactacttgtagtgagggtgctgtgtgtgcttttcttaaatatttatttttttcaacatgctttcaacctgtcaacaaaaacaaaacacacaaaaaaagggcagtgtttgaagattgttgatttttttctggggataatctatattatattgacttcctattacttattataaacctgtgtttgtattggagatgtgtctactattgggggaagaggttctcgtaatcgctcggtgggaaatcatggctctgccgtcctgcctctctgtggccgtgggttcacgtggcctctgcggtgagtctccaagtttctgcctaggcgcctgtgcgtttcctttctgtgacgggattagcttagacatccttgcaaagcgatcactttcaataaattgggaaattgctgctccagc

SEQ ID NO: 24 - DNA, 2014 bp, Mus <mouse, genus>
  Mouse Zbtb46 (NM_027656.2)
agtctatagaagacacagcagcaagactcccagatgaacaaccgaaaggaagatatggaaatcacttctcactaccggcatctgcttcgagagctcaatgagcagaggcagcacggagtcctctgtgatgcgtgcgtcgtggtggagggcaaggtcttcaaggcacataagaacgtcttgcttgggagcagccgctactttaagacgctctactgccaggtacagaagacatctgaccaggccaccgtcactcacttggacattgttacagcccagggcttcaaggccattattgacttcatgtactccgcccatctggctctcactagtaggaatgtcatcgaggtgatgtcagctgccagcttcctacagatgactgacattgtgcaggcctgccatgatttcatcaaggctgcactggacatcagcataaagtcagatgcctccgatgaactctcagaatttgagattggcaccccagccagcaacagtacagaggcgttgatctcagctgtgatggctggaaggagtatctccccatggttggctcggagaacaagtcctgccaattcttctggagactctgccattgccagctgtcatgaaggaggaagcagctatgggaaggaggaccaggaacccaaagctgatggccctgatgacgtttcttcacagtctttgtggcctggagatgtaggctatgggtctctgcgcatcaaggaagaacagatttcaccatcacattatggagggagtgagcttccatcttccaaggacactgcaatacagaattctttatcagaacagggttctggggatggctggcagcccacaggccggaggaagaatcggaaaaacaaagagactgtccgacacatcacccagcaggtggaggaggacagccaggctggctctccagtaccttcattcctacccacatcgggatggcctttcagcagccgagactcaaatgtagacctgacggtcactgaggccagcagcttggacagccgaggcgagagagcagagctctatgctcacatcgatgagggcctactaggaggagaaaccagctacttgggcccacccctcaccccagagaaggaagaagcactacaccaggctactgcagtggccaatcttcgtgctgcactcatgagtaagaacagtctgctgtcactcaaggctgacgtgctcggtgatgatggctcacttctgttcgagtacctgcccaaaggtgcccactcactgtctctgaacgaattcacggtgatcaggaagaagttcaagtgcccctactgcagcttctcagccatgcaccagtgcatccttaagcgacacatgcgctcacatactggagagcggccctacccttgtgagatctgtggcaagaagttcactaggagagagcacatgaagcgacatactctggtccacagcaaggacaagaagtacgtgtgcaaagtgtgcagccgtgtgttcatgtctgcagccagcgtgggcattaagcacggctctcgtcgccatggggtgtgtgcagactgtgctggccggggtgtgggcacgccactggaccatggtggaggtggcgagggctcccctgaggcgctgtttgctggtgaagggccgtacctggaggacccggatgatccacgaggggaggctgaggaggagctggttgaggatgaggatgaggacgtggccaagtggaaggatgacgtgggcttggcccatgaggatgcactgctgggggatgacaaggatgatgaagactctccacaggggcctcacagcccctctggggagcccgataaagactttgcctggatctcctaggggctctgctctagtgggcagggtgagtgatggctgaatcgctttgtccacctgtgtgtgtgtcttagtggatctttacttacccaggagcagggctatgcttactccttgaagctcctcctaaaggcctctcctccatgctatacccctctccattacagaaactggtcctgtgagc

SEQ ID NO: 25 - DNA, 4340 bp, Homo sapiens
  Human RUNX3 (NM_001031680.2)
attcattcattccccgtggcactggaggcggcccactctgctctgtcagcttcggagctcctccaccctggctgccgaaagccccttcccgccatctaatgatacactctgcatacgcttctgttgagaatttgtggctagacattcctgtgggaccgggaatccaaattcttgggtacaaacagaaacttactttccttggggatttttttctctctctcactcacacacactctcgcgttctttccttttttctttttcgtagcagcaggggggaaaaaagagacaaaaacaaaacaaaaaacaacaaaaagcaacaccccccccttttattttcaaaagtagctagaggaaaaaaaaataaaacaacagccaaccaagtgaatcccaacccaaccccctgaagggctgaaaattctcgccttcttcagagcggggcatggcatcgaacagcatcttcgactccttcccgacctactcgccgaccttcatccgcgacccaagcaccagccgccgcttcacacctccctccccggccttcccctgcggcggcggcggcggcaagatgggcgagaacagcggcgcgctgagcgcgcaggcggccgtggggcccggagggcgcgcccggcccgaggtgcgctcgatggtggacgtgctggcggaccacgcaggcgagctcgtgcgcaccgacagccccaacttcctctgctccgtgctgccctcgcactggcgctgcaacaagacgctgcccgtcgccttcaaggtggtggcattgggggacgtgccggatggtacggtggtgactgtgatggcaggcaatgacgagaactactccgctgagctgcgcaatgcctcggccgtcatgaagaaccaggtggccaggttcaacgaccttcgcttcgtgggccgcagtgggcgagggaagagtttcaccctgaccatcactgtgttcaccaaccccacccaagtggcgacctaccaccgagccatcaaggtgaccgtggacggaccccgggagcccagacggcaccggcagaagctggaggaccagaccaagccgttccctgaccgctttggggacctggaacggctgcgcatgcgggtgacaccgagcacacccagcccccgaggctcactcagcaccacaagccacttcagcagccagccccagaccccaatccaaggcacctcggaactgaacccattctccgacccccgccagtttgaccgctccttccccacgctgccaaccctcacggagagccgcttcccagaccccaggatgcattatcccggggccatgtcagctgccttcccctacagcgccacgccctcgggcacgagcatcagcagcctcagcgtggcgggcatgccggccaccagccgcttccaccatacctacctcccgccaccctacccgggggccccgcagaaccagagcgggcccttccaggccaacccgtccccctaccacctctactacgggacatcctctggctcctaccagttctccatggtggccggcagcagcagtgggggcgaccgctcacctacccgcatgctggcctcttgcaccagcagcgctgcctctgtcgccgccggcaacctcatgaaccccagcctgggcggccagagtgatggcgtggaggccgacggcagccacagcaactcacccacggccctgagcacgccaggccgcatggatgaggccgtgtggcggccctactgaccgccctggtggactcctcccgctggaggcggggaccctaacaaccttcaagaccagtgatgggccggctccgaggctccgggcgggaatgggacctgcgctccagggtggtctcggtcccagggtggtcccagctggtgggagcctctggctgcatctgtgcagccacatccttgtacagaggcataggttaccacccccaccccggcccgggatactgcccccggcccagatcctggccgtctcatcccatacttctgtggggaatcagcctcctgccacccccccggaaggacctcactgtctccagctatgcccagtgctgcatgggacccatgtctcctgggacagaggccatctctcttccagagagaggcagcattggcccacaggataagcctcaggccctgggaaacctcccgacccctgcaccttcgttggagcccctgcatcccctgggtccagccccctctgcatttacacagatttgagtcagaactggaaagtgtcccccacccccaccaccctcgagcggggttcccctcattgtacagatggggcaggacccagcacgctgctggcagagatggtttgagaacacatccaagccagtccccccagcccagcttcccctccgttcctaactgttggctttcccccagccgcacgggtcccaggccccagagaagatgagtctatggcatcaggttcttaaacccaggaaagcacctacagaccggctcctccatgcactttaccagctcaacgcatccactctctgttctcttggcagggcgggggaggggggataggaggtcccctttcccctaggtggtctcataattccatttgtggagagaacaggagggccagatagataggtcctagcagaaggcattgaggtgagggatcattttgggtcagacatcaatgtccctgtcccccctgggtccagccaagctgtgccccatcccccaagcctcctgggaggatccagccaaatcttgcgactcctggcacacacctgtctgtaacctgttttgtgctctgaaagcaaatagtcctgagcaaaaaaaaaaaaaaaacaaaaaaacaaaaaaaaaacaaaacagtttttaaaactgattttagaaaaagaagcttaatctaacgttttcaaacacaaggtctcttacaggtatagttccgtgattatgatagctctgtgattataagcaacatccccgccccctctcccccccgcggacccccagctgcctcctgagggtgtggggttattagggtctcaatactttctcaaggggctacactccccatcaggcagcatcccaccagcctgcaccacaggctcccctgggaggacgagggaaacgctgatgagacgctgggcatctctcctctgtggctctaggacatctgtccaggaggctgggcggaggtgggcaggatgtgagaggtggggagtactggctgtgcgtggcaggacagaagcactgtaaagggctctccagccgcagctcagctgcactgcgttccgaggtgaagtcttgcccctgaattttgcaaaatgggaaagtgggcgcttgcccaagggccaggctgcatggattctcacatcagagttctctggccctagaaaggcttagaaaaggcgtaagggaactcataaaggctagcagcatgcggtattttaactttctgcctcggcctctgtggatgcagaaatctgccctacaaaatgctcttcattggttgtctctgtgagagcactgtccccacccaacctgtcacaacggccagaaccatacaccagagacacactggcaggttaggcagtccttctggtgatcctattccattccctcctgctgcggtttctcttggcctgtcctcactggaaaaacagtctccatctcctcaaaatagttgctgactccctgcacccaaggggcctctccatgccttcttaggaagcagctatgaatccattgtccttgtagtttcttccctcctgttctctggttatagctggtcccaggtcagcgtgggaggcacctttgggttcccagtgcccagcactttgtagtctcatcccagattactaacccttcctgatcctggagaggcagggatagtaaataaattgctcttcctaccccatcccccatcccctgacaaaaagtgacggcagccgtactgagtctgtaaggcccaaagtgggtacagacagcctgggctggtaaaagtaggtccttatttacaaggctgcgttaaagttgtactaggcaaacacactgatgtaggaagcacgaggaaaggaagacgttttgatatagtgttactgtgagcctgtcagtagtgggtaccaatcttttgtgacatattgtcatgctgaggtgtgacacctgctgcactcatctgatgtaaaaccatcccagagctggcgagaggatggagctgggtggaaactgctttgcactatcgtttgcttggtgtttgtttttaacgcacaacttgcttgtacagtaaactgtcttctgtactatttaactgtaaaatggaattttgactgatttgttacaataatataactctgagatgtgtggaagga

SEQ ID NO: 26 - DNA, 3891 bp, Mus <mouse, genus>
  Mouse Runx3 (NM_019732.2)
attcattcattcatccaggctgctgagtctggactggctgctgcagccccgggctcctccgccctgactgcccagagccccttcccaccatttaatgatactctgcacatagtgctgttgaaaatttgtggctagacattcctgtgggactgggaagccaaattcttgggtacaaaccgaaactttctttccttggagattttcttctctctcgcccacagacgctctcgcgttctttccccattttttttctttctcttcttttttttctttttttttttttttttgtagcagcagggggagaaaaaaagaaaccaaactttaaaaaaaaaaagtcaacacctccccttttttattttcgaaagcaacttgaaaaaatatatataacaaaacagcagccaaccaagtgggtctgaacccaaccccctgaggccgagtccttgccactgtcagcgtgcgacatggcttccaacagcatctttgactccttccccaactatacaccaaccttcatacgagacccgagcaccagccgccgcttcactcccccctccacggccttcccctgcggcggcggcggcggcggcaagatgggcgagaacagcggcgcgctaagcgcgcaggcaaccgcgggccccggcggccgcacccggcccgaagtgcgctcgatggtggacgtgctggccgaccacgcgggagagctcgtgcgcaccgacagccccaacttcctctgctccgtgctgccctcgcactggcgctgcaacaagacgctgccggtcgccttcaaggtggtggccctgggggatgtgccggatggaacggtggtgaccgtgatggccggcaatgatgagaactactccgccgagctgcgcaacgcttccgctgtcatgaagaaccaagtggccaggttcaacgaccttcgattcgtgggccgcagtgggcgagggaagagtttcacgctcacaatcaccgtgttcaccaaccctacccaagtggctacctaccaccgagccatcaaggtcactgtggatggaccccgggaaccccgacggcaccggcagaagatagaagaccagaccaaggccttccccgaccgctttggagacctgcgcatgcgtgtaacaccaagcacacccagcccccgtggctctctcagcaccacgagccacttcagcagccaggcccagaccccaatccaaggctcctcagacctgaaccccttctccgacccccgccagtttgaccgctccttccctacgctgcagagcctcacagagagccgcttcccggaccccaggatgcactacccgggagccatgtctgccgccttcccctacagcgccacaccatcgggcaccagcctgggcagcctgagcgtggcgggcatgccggccagcagccgcttccaccacacctacctccctccgccctaccccggggccccacagagccagagcgggccctttcaggccaaccccgcgccctaccacctcttttacggcgcctcctccggctcctaccagttctccatggcagccgcgggaggtggtgagcgctcgcccacccgcatgctgacctcctgccccagcggcgcttcggtgtcagcaggcaacctcatgaaccccagcctgggccaggctgatggcgtggaagccgacggcagccacagcaactcgcccacggccctgagcacgccgggccgcatggacgaggccgtgtggcggccctactaagcaccctggagactctcgggccagccgaatccttccctccagcccgagactacaagaagaaacagactttggcctggtcccaggggccagagctggcagtggctcccagagctctgtccagccacaagtttgagcagaggatgtggggacctcccacaggacactgctccaacccaaatcaatgtcctctctagctgtgcatcccaaacccacctcttgtctccagccatgcccaggatcaattctagaatcagaggctacccctgcctgtgtggggagggcctttgctggcaagagaagctcaggctcagagatgtctggactttctctccctccctctctctctctctctctctctctctctctctctctctctctctctctctcacacacacacacacacacacacacacacacacacacacacactgccctggggaccatccatgcccatcaaaccaaagggaaactcaaacccctgggaaggtttcactcccctgaagagagagaggagccatatctctctttcacatacacacacacacacacacacacacacacacacacacacgtccccaacttgacttccccctggtcccaggccagcagcccctgatcagtcctaacttacctgaaaacaccaggccccagagcagactcatccggggtggcaggtccctaaagcaaggaaggcctcacactgtccagcatactccagcctgaattgcctactgggttctcagggggcagacaggtcctggccgaaagtcttaccatggggatcgatagggtggttagccctgcgcactaggtccagccaatctgtgctctgggccttgcctcccaggccacagtcctgctcccaacttgtttgtccctagaagcagacaactttgaaccaaaagcatctcagtcaagcatctaaaacagggggcagtctgtgtatacaagagcccacctcctgctgtgtgatgtcatcaggacacccccaccctcaccccaccaccagggtcctgacttcacattcttcacagaaggggacaagacctccaggaggccctgtggagtctctggtgaggtgtgcgatggcagagcagcatccaagcagagatcagatgtcctcttcagtctgtgggcgggcgattgtcagtgggattggttaaaaagctcttaccagagctggctggcccacggctggtttttcaaactgagtgagccccgtagtgatggcctctgccttgtgcttggccttccccattgcctgcacctgaaacagccacccacatacacactctggtaggtcagggggtccccgacaatcctggacaatcctgagcagaatacctcctgttacagtgtctcttgtcccacccttactggaggaaaaaaaaaaaaaaaactctatctcttggaagtagctgaggtaaccttccagctccctgcacccagagggggccttctcacctcttctcaggaagcagctacgacccattgccctcctacctgcttcgctactggtccatggtacagactgttccagatcaccaagaaaggtactttcaggatcccagtgcctagcactgggtaagctaccccagacaactagccttccttatacccaaacgctggtcggtggaaatagaaagtcacccctcccccatcgcctctttctcatccctgattaacagtgaagtttgagtcttgtcgtgagtcctacagtgagcacaggcagctggggctaataaaaaaagaagaagaagaagaaaaaggagaggagagaaaaaaaacaaaaatgaaaggaaaagggtccttatttgcaaggctactttaaagtgctacttgaaagcacaggctagacagaaagcacaaggaacctagggggttgatacaatgttactgtaattgtgtgggtgggtgtcatcctttgtgacattgttaccctgaggtatactccctgcagtgagctggtcttcctgaagtgggcctgctttgcactataggctgcttgtatgtttggtttgttgtttttgtttttttgttttttttaatgcacaacttgcttgtacaggtcaactgtccatcttgggtactatttaactgtcaaacagaggaatctgtgtttgttacaataatataacagatgccttgaaggacccgc

SEQ ID NO: 27 - DNA, 2802 bp, Homo sapiens
  Human GFI1 (NM_005263.3)
gagggtgcgcccaccggtcccgccgggcgcccgcgggacgcgccgccagggccctctccgccgggggctcggcgctcgcccacctcttccaaatttaaccattacctaaatccgaagggaaatgagcaaacctctcggattgggtgtcaaggtctcctccgggctggggctgagcaagccctcggagtgaccgtgggtgacagcggctccagggactcttggggcgcagtggggaaagtgccggaccaccatgccgcgctcatttctcgtcaaaagcaagaaggctcacagctaccaccagccgcgctccccaggaccagactattccctccgtttagagaatgtaccggcgcctagccgagcagacagcacttcaaatgcaggcggggcgaaggcggagccccgggaccgtttgtcccccgaatcgcagctgaccgaagccccagacagagcctccgcatccccagacagctgcgaaggcagcgtctgcgaacggagctcggagtttgaggacttctggaggcccccgtcaccctccgcgtctccagcctcggagaagtcaatgtgcccatcgctggacgaagcccagcccttccccctgcctttcaaaccgtactcatggagcggcctggcgggttctgacctgcggcacctggtgcagagctaccgaccgtgtggggccctggagcgtggcgctggcctgggcctcttctgcgaacccgccccggagcctggccacccggccgcgctgtacggcccgaagcgggctgccggcggcgcgggggccggggcgccagggagctgcagcgcaggggccggtgccaccgctggccctggcctagggctctacggcgacttcgggtctgcggcagccgggctgtatgagaggcccacggcagcggcgggcttgctgtaccccgagcgtggccacgggctgcacgcagacaagggcgctggcgtcaaggtggagtcggagctgctgtgcacccgcctgctgctgggcggcggctcctacaagtgcatcaagtgcagcaaggtgttctccacgccgcacgggctcgaggtgcacgtgcgcaggtcccacagcggtaccagaccctttgcctgcgagatgtgcggcaagaccttcgggcacgcggtgagcctggagcagcacaaagccgtgcactcgcaggaacggagctttgactgtaagatctgtgggaagagcttcaagaggtcatccacactgtccacacacctgcttatccactcagacactcggccctacccctgtcagtactgtggcaagaggttccaccagaagtcagacatgaagaaacacactttcatccacactggtgagaagcctcacaagtgccaggtgtgcggcaaggcattcagccagagctccaacctcatcacccacagccgcaaacacacaggcttcaagcccttcggctgcgacctctgtgggaagggtttccagaggaaggtggacctccgaaggcaccgggagacgcagcatgggctcaaatgagcaccctggctggctgcaagcagcagctacacaacactacagagggcagcctccctgcttgccaccactctgctccctgcttgcctccactcccttctgactttccagaccccaggtccagtctgcagatcctaccaggttgctcctccttcgccttacctcctggagctgccagaagaaatgaggtaccttttcaaagtgcagccgagagtgagaaccaagtgactctctaggcttcggacacaaataggctcctctacacctgaagacaaaggcaaagtcaaatggggaccagaataaatcttagaccccacagtccttcccatttccagccctaatctacagacaggaatgcccttcaggtttcttccctcccccctcttgacctaccccagatatttgtgtggaagaggaggaatcaccatttacaaggtggacaaatgctaatatttttatctagaaagaagagtgagtgttaacttttatttttttccttctggggggtctgttgactcctttcttttgggtgctgcctataaatcttggaggaatcatttctcctcctcaaaaactgattcagaaactgacttggggaaggaatttaatactttgaagtcatgagatgcaccatcgaggctacccccaagaagaagcagaagagaagttggtaatgagaggggattagaggtcctcccttcagtagggctgtgaaaacctcatcactggaggtaaaagcacaagcaatgcctgtggacaagatgtcattcattcactcagcaaatgttcatggatcaccggctaccaaggtaccaggcaccatgctaggtattggggaagagagactgaagtcacaacccctgactgctcctcaaaagctaacggttgcacctccaagtggctgggtctgttcttactcttggagggaattctgagaagacagcacagaattgtaaaccttcccttttgacccttttggattttatcaggtgtaaacaaaaagctgaacagttacttcaaagatatgtgtgtatattcagttttttattgttaagctgatattttaaagatttctgagctagcaggcatgtgggaaggaaggctctgtcttcaactctttgaccctccatgtgtaccatagaggggggaaaggtggtattttcactttgatgaggttggtaaatgtttttagatcttctggtaagcattatgtttgttaatacatatttattagagtgatgttttaagttaataaagtattaagagtattaaaaaaaaaaaaaaaa

SEQ ID NO: 28 - DNA, 2862 bp, Mus <mouse, genus>
  Mouse GFI1 (NM_010278.2)
ctccaagccccttccgggtcccaaacactgatgccccctgactggctaaactaagccacgcatccctggcgtgagccacaacccagaagggagcaggtgggcttgcagggttgacttgggataacggaccagttgtggactactgctctcaggagagtgatgatctagctttggtagggaaggggaggggctgaggcgtgggcagggcagagcaaagggaccagagccagagcctggggacaggttttaccactgagctgttgcagtggcggcggaggccgggattcgtgccacctgtccgagtgccacctggtgagcgtggcgcctgggtccaggcccctcctcccgcggcttccctctctcctccctggcccacactcttccttggcctgggaacctaccacaaccgccatcggtgctgaccctcgtttccacccaattttcccccttctctcagaactcagagtatccgagggtccaaacattcgtccagcggctgaccaccatgccgcgctcattcctggtcaagagcaagaaggcgcacagctatcaccagccgcgttctccggggccggactactccctgcgcctggagaccgtgcctgcgccgggcagagcagagggcggcgctgtgagtgcaggcgagtcgaaaatggagccccgagagcgtttgtcccccgactctcagcttaccgaggctcccgacagggcctccgcgtcccccaacagctgcgaaggcagcgtttgtgacccctgctccgagttcgaggacttttggaggcccccttctccctccgtgtctccagcgtcggagaagtcactgtgccgctctctggacgaagcccagccctacacgctgcctttcaagccctatgcatggagcggtcttgctgggtctgacctgcggcacctggtgcagagctatcggcagtgcagcgcgctggagcgcagcgcgggcctgagcctcttctgcgagcgcggctcggagccgggccgcccggcagcgcgctacggccccgagcaggctgcgggcggagccggtgcgggacagccagggagctgcggggtcgccgggggcgccaccagcgctgcgggcctggggctctacggcgacttcgcgcctgcggcggccgggctgtacgagcggccgagcacagcagcaggccggctgtaccaagatcatggccacgagctgcacgcggacaagagcgtgggcgtcaaggtggagtcggagctgctttgcacccgtctgctgctgggcggcggctcctacaaatgcatcaaatgcagcaaggtgttctccacaccgcacgggctggaggtgcacgtgcgccggtcccacagcggcacaagaccctttgcgtgcgagatgtgcggcaagaccttcgggcacgcggtgagcctggagcaacacaaggcagtgcactcccaggaacgcagctttgactgtaagatctgtggcaagagcttcaagaggtcatccacgctgtccacacatctgctcattcactcggacacccggccctatccctgtcagtactgtggcaaaagattccaccagaagtcagatatgaagaaacacaccttcatccacacaggtgagaagccccacaaatgccaggtgtgcggcaaagccttcagtcagagctccaacctcatcactcatagcagaaagcacacaggcttcaagccctttggctgtgacctgtgtgggaagggcttccagaggaaggtggatctcaggaggcaccgagagactcagcatggactcaaatgagtaccctggcagcccgcaacaccagctgtgtaacactaccgtgagggatgtcttccctgcctccctccagccccttctcaggccctgagtccagtgtgcaaagctcatcatggttagtccccttcaccttccttcccggagctgctggaggagatgaactcccgtttctaaggtcaacccagagtgggaaccgcagcagcagcagcagtcgtctgtgctttgggcttccctacagctgaagatggggatcaaatgagatcttgcacctcccagttcttcccttttttgctgtctcacaggccagaatgaactctgggcagctgctacaagaggaggcatcacctcttaagctttgagcgccactgatgcatttattgagaacgaatgaacattaattttctcttctggggagactgctgactcctttatcctccaccagactctggtttagggaaggaacctcgttcctttgaaatcatcagatgcaccatcaagcctgccacgagaagaaggggacttggtgatgagagggagtcagaggtcctgtggtgccatcagaggaggtgaagctgtggagcagctccggggaacagggtcttcacttactcagcgagtgattattggccgcaggttatcagagtaaggaactgtgctaggtatgggagagccagagattaaagtcataggccctaacccccaaaagctatcagttggacttcaacatagctagagcctgtgttctgtgcttccaagggagttctgaagaaggccacacaaacattgggacttctttttgacacttacggagtttttcaagtgtaaacaaataggaactggaggattatttctaaagttcatgagtaaatccagcttttattgttaggtgggactttattagatgcctgcgctgggagatgtggggtgaaggctatggcctcagctcctgccccttatcatcttaggaacaacttatttttcctgtgagggttgtagacgttcctaaatcttcttgagtgcattatgtattagcataatcatatttattagaatgttgttttaacttaataaagtattaagattattac

SEQ ID NO: 29 - DNA, 2302 bp, Homo sapiens
  Human IRF2 (NM_002199.3)
agccgcggctcttcgcagtttcctctccttgttttgctttcgatctggactgttctcaggcaagccggggagtaacttttagttttgctcctgcgattattcaactgacgggctttcatttccatttcacataccctagcaacacttataccttgcggaattgtattggtagcgtgaaaaaagcacactgagagggcaccatgccggtggaaaggatgcgcatgcgcccgtggctggaggagcagataaactccaacacgatcccggggctcaagtggcttaacaaggaaaagaagatttttcagatcccctggatgcatgcggctagacatgggtgggatgtggaaaaagatgcaccactctttagaaactgggcaatccatacaggaaagcatcaaccaggagtagataaacctgatcccaaaacatggaaggcgaatttcagatgcgccatgaattccttgcctgatattgaagaagtcaaggataaaagcataaagaaaggaaataatgccttcagggtctaccgaatgctgcccctatcagaacggccttctaagaaaggaaagaaaccaaagacagaaaaagaagacaaagttaagcacatcaagcaagaaccagttgagtcatctctggggcttagtaatggagtaagtgatctttctcctgagtatgcggtcctgacttcaactataaaaaatgaagtggatagtacggtgaacatcatagttgtaggacagtcccatctggacagcaacattgagaatcaagagattgtcaccaatccgccagacatttgccaagttgtagaggtgaccactgagagcgacgagcagccggtcagcatgagcgagctctaccctctgcagatctcccccgtgtcttcctatgcagaaagcgaaacgactgatagtgtgcccagcgatgaagagagtgccgaggggcggccacactggcggaagaggaatattgaaggcaaacagtacctcagcaacatggggactcgaggctcctacctgctgcccggcatggcgtccttcgtcacttccaacaaaccggacctccaggtcaccatcaaagaggagagcaatccggtgccttacaacagctcctggcccccttttcaagacctccccctttcttcctccatgaccccagcatccagcagcagtcggccagaccgggagacccgggccagcgtcatcaagaaaacatcggatatcacccaggcccgcgtcaagagctgttaagcctctgactctccgcggtggttgttggggcttcttggctttgttttgttgtttgtttgtattttatttttttctctctgacacctattttagacaaatctaagggaaaaagccttgacaatagaacattgattgctgtgtccaactccagtactggagcttctctttaactcaggactccagcccattggtagacgtgtgtttctagagcctgctggatctcccagggctactcactcaagttcaaggaccaacaagggcagtggaggtgctgcattgcctgcggtcaaggccagcaaggtggagtggatgcctcagaacggacgagataatgtgaactagctggaattttttattcttgtgaatatgtacataggcagcactagcgacattgcagtctgcttctgcaccttatcttaaagcacttacagataggccttcttgtgatcttgctctatctcacagcacactcagcacccccttctctgcccattccccagcctctcttcctatcccatcccatcccatcccatcccatcccatcccatcccgctcttttcctacttttccttccctcaaagcttccattccacatccggaggagaagaaggaaatgaatttctctacagatgtcccattttcagactgctttaaaaaaaatccttctaatctgctatgcttgaatgccacgcggtacaaaggaaaaagtatcatggaaatattatgcaaattcccagatttgaagacaaaaatactctaattctaaccagagcaagcttttttattttttatacaggggaatattttattcaaggtaaaattctaaataaaatataattgttttttatcttttctacagcaaatttataattttaagattccttttcttgtttatcagcagttgttattacatccttgtggcacatttttttttttaattttgtaaaggtgaaaaaagcttttatgagctcatgtagcaatcagattttcctgtggattgataataaatgaatatgatatatagttaaatttttaaaaaaaaaaaaaaaaaa

SEQ ID NO: 30 - DNA, 2484 bp, Mus <mouse, genus>
  Mouse Irf2 (NM_008391.4)
gctcctcgcagtttcctctccttgttttgctttcgatctggactgttctcaggcaagccggggactaacttttagttttgctcctgcgattattcaactgacgggctttcatttccattttacacaccctaacaacactcacaccttgcgggattgtattggtagcgtggaaaaaaaaaagcacattgagagggtaccatgccggtggaacggatgcgaatgcgcccgtggctggaggagcagataaattccaatacgataccagggctaaagtggctgaacaaggagaagaagattttccagatcccctggatgcatgcggctcggcacggatgggacgtggaaaaggatgctccgctcttcagaaactgggcgatccatacaggaaagcatcaaccaggaatagataaaccagatccaaaaacatggaaagcaaattttcgatgtgccatgaattccctgcccgacattgaggaagtgaaggacagaagcataaagaaaggaaacaacgccttcagagtctaccggatgctgcccttatccgaacgaccttccaagaaaggaaagaaaccaaagacagaaaaagaagagagagttaagcacatcaagcaagaaccagttgagtcatctttggggcttagtaatggagtaagtggcttttctcctgagtatgcggtcctgacttcagctataaaaaatgaagtggatagtacggtgaacatcatagttgtaggacagtcccatctggacagcaacattgaagatcaagagatcgtcactaacccgccagacatctgccaggttgtagaagtgaccactgagagtgatgaccagccagtcagcatgagtgagctctaccctctacagatttctcctgtgtcttcctacgcagaaagcgaaactaccgacagtgtggccagtgatgaagagaacgcagaggggagaccacactggaggaagaggagcatcgaaggcaagcagtacctcagcaacatggggacacggaacacctatctgctgcccagcatggcgacctttgtcacctccaacaagccagatctgcaggtcaccatcaaagaggatagctgtccgatgccttacaacagctcctggcccccatttacagaccttccccttcctgccccagtgacccccacgcccagcagcagtcggccagaccgggagacccgggccagtgtcatcaagaagacatctgatatcacccaggcccgtgtcaagagctgttaagcctttgactctccctggtggttgttgggatttcttagctttgtgttgttctttgtttgtattatattattttttttctctatgatacctatcttagacacatctaagggagaaagccttgacgatagattattgattgctgtgtccaactccagagctggagcttcttcttaactcaggactccagccccccccccccctcggtagatgcgtatctctagaacctgctggatctgccagggctactccctcaagttcaaggaccaacagccacacgggcagtggaggtgctgcgttgcctacggtcaaggccagcatggtggagtggatgcctcagaacggaggagaaaatgtgaactagctggaatttttttattcttgtgaatatgtacatagggcagtacgagcaatgtcgcgggctgcttctgcaccttatcttgaagcacttacaataggccttcttgtaatcttgctctccttcacagcacactcggcgaccccttctgtgtccactaccccactacccacccctccctcctcaacccctccatcccggtcctctatgcgccccttccccccaaccaatcccatcacaacctcttacctatcctttccctcccaaccccttctatcccagcccaccacctaccccactcctccccaactcctccattctagcccattacccacgcctctctcctcagcccagcctaccccatcccaccctgttcctttcctccagtttcctctcctcaaaggcaaggctctacatcttggaggaggaggaggagaagaaaatgagtttcttcaccgctgtcccattttaagactgcttgaataataaaaaaaaaatctttctaatctgctatgcttgaatggcacgcggtacaaaggaaaactgtcatggaaatattatgcaaattcccagatctgaagacggaaaatactctaattctaaccagagcaagcttttttatttttttatacaaggggaatattttattcaaggtaaaaaaattctaaataaaatataattgttttttatcttttctacagcaaatttataattttaagattccttttcctgttcatcagcagttgttattacatcccttgtggcacattttttttttaattttgtaaaggtgaaaaaaaaacttttatgagctcatgtagcaatcaaattatcctgtggattgataataaatgaatatggtatatagttaaagattttaa

SEQ ID NO: 31 - DNA, 2247 bp, Homo sapiens
  Human NFIL3 (NM_001289999.1)
aattgtgcagggggcggtgtttgtgcgtggagctttccctcccggctccgggccgtcgcggctctcgggagaggcgccgggacattttaatcgctgcctccgccgcgcagccctgcgcagctgcccggccgcgccaaccccttccccgccgcagcgcgccccgagtgttggcagcttgccagccgccaccccccgccttccctcctgcccaccccaaggtagagggctcctctcgggagtgtgcggggaaggggaggccgaggtccgggccacgcccgggtagccgcaacccgcagtgctcagtcggcaacaggtagcccagcaggctgcggctctcaggaagacaaaaagcgcctctgcgagcaaataacgaaggaggcccaacttcattcaataaggagcctgacggatttatcccagacggtagaacaaaaggaagaatattgatggattttaaaccagagtttttaaagagcttgagaatacggggaaattaatttgttctcctacacacatagatagggtaaggttgtttctgatgcagctgagaaaaatgcagaccgtcaaaaaggagcaggcgtctcttgatgccagtagcaatgtggacaagatgatggtccttaattctgctttaacggaagtgtcagaagactccacaacaggtgaggagctgcttctcagtgaaggaagtgtggggaagaacaaatcttctgcatgtcggaggaaacgggaattcattcctgatgaaaagaaagatgctatgtattgggaaaaaaggcggaaaaataatgaagctgccaaaagatctcgtgagaagcgtcgactgaatgacctggttttagagaacaaactaattgcactgggagaagaaaacgccactttaaaagctgagctgctttcactaaaattaaagtttggtttaattagctccacagcatatgctcaagagattcagaaactcagtaattctacagctgtgtactttcaagattaccagacttccaaatccaatgtgagttcatttgtggacgagcacgaaccctcgatggtgtcaagtagttgtatttctgtcattaaacactctccacaaagctcgctgtccgatgtttcagaagtgtcctcagtagaacacacgcaggagagctctgtgcagggaagctgcagaagtcctgaaaacaagttccagattatcaagcaagagccgatggaattagagagctacacaagggagccaagagatgaccgaggctcttacacagcgtccatctatcaaaactatatggggaattctttctctgggtactcacactctcccccactactgcaagtcaaccgatcctccagcaactccccgagaacgtcggaaactgatgatggtgtggtaggaaagtcatctgatggagaagacgagcaacaggtccccaagggccccatccattctccagttgaactcaagcatgtgcatgcaactgtggttaaagttccagaagtgaattcctctgccttgccacacaagctccggatcaaagccaaagccatgcagatcaaagtagaagcctttgataatgaatttgaggccacgcaaaaactttcctcacctattgacatgacatctaaaagacatttcgaactcgaaaagcatagtgccccaagtatggtacattcttctcttactcctttctcagtgcaagtgactaacattcaagattggtctctcaaatcggagcactggcatcaaaaagaactgagtggcaaaactcagaatagtttcaaaactggagttgttgaaatgaaagacagtggctacaaagtttctgacccagagaacttgtatttgaagcaggggatagcaaacttatctgcagaggttgtctcactcaagagacttatagccacacaaccaatctctgcttcagactctgggtaaattactactgagtaagagctgggcatttagaaagatgtcatttgcaatagagcagtccattttgtattatgctgaattttcactggacctgtgatgtcatttcactgtgatgtgcacatgttgtctgtttggtgtctttttgtgcacagattatgatgaagattagattgtgttatcactctgcctgtgtatagtcagatagtccatgcgaaggctgtatatattgaacattatttttgttgttctattataaagtgtgtaagttaccagtttcaataaaggattggtgacaaacacagaaaaaaaaaaaaaaaaaaaaa

SEQ ID NO: 32 - DNA, 2019 bp, Mus <mouse, genus>
  Mouse Nfil3 (NM_017373.3)
acacatctctcggcgcggccacggcgcccgcggacccggcgcgcccgctcgtctcccgcgccgcgccctcgccaccgcccgctgagggcccggcggagcttgaatcgcgccccggcgccgccagcccggttacagccgccctttcttttccccctcacggaccagggagcagaaccacgataacccatgaaaggctcctgacagatttaccctgtgccggacaacagaaggacccattgatggatgagaggctgaagtccttaagacctgaaagaagactggggaagtgatttgtctcctccatccggtctgtaggacgaggaggtcctttctgatgcagctgagaaaaatgcagaccatcaaaaaggagcccgcacccctagatcctaccagcagctcagacaagatgctgctgctgaactctgccttagctgaggtggccgaggacctagcctcaggtgaagatttgctcctgaacgaagggagcatggggaaaaacaaatcctcggcgtgtcggagaaaacgggaattcattccggacgagaagaaagacgccatgtattgggagaaacggcggaaaaacaacgaagctgccaaaagatctcgggagaagcgccgcctcaatgacctggttttggagaacaagctgatcgccctgggagaagaaaatgccactttaaaagctgagctgctctccctgaaattaaagtttggtttaattagctccacggcgtatgcccaagaaatccagaaactcagtaattccacagctgtctactttcaggactaccagacatccaaggctgccgtgagctcttttgtggacgagcatgagcctgcgatggtagccggaagttgcatctcagtcatcaagcactctccccagagctcgctctccgatgtgtcagaggtgtcctcggtggagcacactcaggaaagccccgcacagggaggctgccggagccctgagaacaagttccctgtgatcaagcaggagcccgtggagttggagagctttgccagggaggccagggaggagcggggcacgtattccacctccatctaccagagctacatgggaagctctttctccacttactcccactccccacccctcttgcaggtccatgggtccactagcaactccccaagaacctcagaggccgatgagggtgtagtgggcaagtcttctgatggggaagacgaacaacaggtccctaagggccccatccattctccagtggagctgcaacgggtccacgccacggtggtgaaggttccggaagtgaacccttctgccttaccgcacaagcttcggattaaagccaaggccatgcaggtcaaagtggaggctttggacagcgagtttgaaggcatgcagaaactctcttcacccgccgatgcgatcgccaaaagacattttgacctggagaaacatggaacctcgggtatggcccattcctccctccctcctttctcagtgcaggtgacgaacattcaagattggtccctcaaatcggaacactggcatcacaaagaactgagcagcaaaactcagagtagcttcaaaacaggtgtggtggaagtcaaagacggtggctataaggtttccgaagctgagaatttgtatttgaagcagggaatagcaaacttatctgcagaggtggtctcgctcaagagattcatagccacacaaccgatctcggcttcggactccaggtaaatggctgctgaccgagctatgcatggaggaggaggctgttggtaccatactgaatttccactggacctctaaagtcatttcactgtagtgtgcacaacggcgtctgtctgggtgtccttgtgtgcacgcgctgaagacttgatgccctcactctgcctggcgtgtagtcagatagccccccacagaggctgtacatactgaacgttatttttgctctattataaagtgtgtatgttgccagtttcaataaaggattggtggcaagcacaaaaaaaaaaaaaaaaaaaaaaaaaaaa

SEQ ID NO: 33 - DNA, 3575 bp, Homo sapiens
  Human BCL6 (NM_001706.4)
accatcgtcttgggcccggggagggagagccaccttcaggcccctcgagcctcgaaccggaacctccaaatccgagacgctctgcttatgaggacctcgaaatatgccggccagtgaaaaaatcttgtggctttgagggcttttggttggccaggggcagtaaaaatctcggagagctgacaccaagtcctcccctgccacgtagcagtggtaaagtccgaagctcaaattccgagaattgagctctgttgattcttagaactggggttcttagaagtggtgatgcaagaagtttctaggaaaggccggacaccaggttttgagcaaaattttggactgtgaagcaaggcattggtgaagacaaaatggcctcgccggctgacagctgtatccagttcacccgccatgccagtgatgttcttctcaaccttaatcgtctccggagtcgagacatcttgactgatgttgtcattgttgtgagccgtgagcagtttagagcccataaaacggtcctcatggcctgcagtggcctgttctatagcatctttacagaccagttgaaatgcaaccttagtgtgatcaatctagatcctgagatcaaccctgagggattctgcatcctcctggacttcatgtacacatctcggctcaatttgcgggagggcaacatcatggctgtgatggccacggctatgtacctgcagatggagcatgttgtggacacttgccggaagtttattaaggccagtgaagcagagatggtttctgccatcaagcctcctcgtgaagagttcctcaacagccggatgctgatgccccaagacatcatggcctatcggggtcgtgaggtggtggagaacaacctgccactgaggagcgcccctgggtgtgagagcagagcctttgcccccagcctgtacagtggcctgtccacaccgccagcctcttattccatgtacagccacctccctgtcagcagcctcctcttctccgatgaggagtttcgggatgtccggatgcctgtggccaaccccttccccaaggagcgggcactcccatgtgatagtgccaggccagtccctggtgagtacagccggccgactttggaggtgtcccccaatgtgtgccacagcaatatctattcacccaaggaaacaatcccagaagaggcacgaagtgatatgcactacagtgtggctgagggcctcaaacctgctgccccctcagcccgaaatgccccctacttcccttgtgacaaggccagcaaagaagaagagagaccctcctcggaagatgagattgccctgcatttcgagccccccaatgcacccctgaaccggaagggtctggttagtccacagagcccccagaaatctgactgccagcccaactcgcccacagagtcctgcagcagtaagaatgcctgcatcctccaggcttctggctcccctccagccaagagccccactgaccccaaagcctgcaactggaagaaatacaagttcatcgtgctcaacagcctcaaccagaatgccaaaccagaggggcctgagcaggctgagctgggccgcctttccccacgagcctacacggccccacctgcctgccagccacccatggagcctgagaaccttgacctccagtccccaaccaagctgagtgccagcggggaggactccaccatcccacaagccagccggctcaataacatcgttaacaggtccatgacgggctctccccgcagcagcagcgagagccactcaccactctacatgcaccccccgaagtgcacgtcctgcggctctcagtccccacagcatgcagagatgtgcctccacaccgctggccccacgttccctgaggagatgggagagacccagtctgagtactcagattctagctgtgagaacggggccttcttctgcaatgagtgtgactgccgcttctctgaggaggcctcactcaagaggcacacgctgcagacccacagtgacaaaccctacaagtgtgaccgctgccaggcctccttccgctacaagggcaacctcgccagccacaagaccgtccataccggtgagaaaccctatcgttgcaacatctgtggggcccagttcaaccggccagccaacctgaaaacccacactcgaattcactctggagagaagccctacaaatgcgaaacctgcggagccagatttgtacaggtggcccacctccgtgcccatgtgcttatccacactggtgagaagccctatccctgtgaaatctgtggcacccgtttccggcaccttcagactctgaagagccacctgcgaatccacacaggagagaaaccttaccattgtgagaagtgtaacctgcatttccgtcacaaaagccagctgcgacttcacttgcgccagaagcatggcgccatcaccaacaccaaggtgcaataccgcgtgtcagccactgacctgcctccggagctccccaaagcctgctgaagcatggagtgttgatgctttcgtctccagccccttctcagaatctacccaaaggatactgtaacactttacaatgttcatcccatgatgtagtgcctctttcatccactagtgcaaatcatagctgggggttgggggtggtgggggtcggggcctgggggactgggagccgcagcagctccccctcccccactgccataaaacattaagaaaatcatattgcttcttctcctatgtgtaaggtgaaccatgtcagcaaaaagcaaaatcattttatatgtcaaagcaggggagtatgcaaaagttctgacttgactttagtctgcaaaatgaggaatgtatatgttttgtgggaacagatgtttcttttgtatgtaaatgtgcattcttttaaaagacaagacttcagtatgttgtcaaagagagggctttaatttttttaaccaaaggtgaaggaatatatggcagagttgtaaatatataaatatatatatatataaaataaatatatataaacctaaaaaagatatattaaaaatataaaactgcgttaaaggctcgattttgtatctgcaggcagacacggatctgagaatctttattgagaaagagcacttaagagaatattttaagtattgcatctgtataagtaagaaaatattttgtctaaaatgcctcagtgtatttgtatttttttgcaagtgaaggtttacaatttacaaagtgtgtattaaaaaaaacaaaaagaacaaaaaaatctgcagaaggaaaaatgtgtaattttgttctagttttcagtttgtatatacccgtacaacgtgtcctcacggtgccttttttcacggaagttttcaatgatgggcgagcgtgcaccatccctttttgaagtgtaggcagacacagggacttgaagttgttactaactaaactctctttgggaatgtttgtctcatcccattctgcgtcatgcttgtgttataactactccggagacagggtttggctgtgtctaaactgcattaccgcgttgtaaaatatagctgtacaaatataagaataaaatgttgaaaagtcaaactggaaaaaaaa

SEQ ID NO: 34 - DNA, 3527 bp, Mus <mouse, genus>
  Mouse Bcl6 (NM_009744.4)
gtagccgcgcgcgcccgcctcgggacccccggtgttccgggcggcggtgctgcgggaaccacgatccgcactatagggcggcgagcggcgcggccccgaggcattctgccggccgggagggcgctgcggagcgcgccgctgccaccgagtcctcccctgctgcggagcaatggtaaagcccgcagctcaaattccgagaattgagctctgttgattcttagaactggggttcttagaagtggtgatgcaagaagtttctaggaaaggccggacaccagttttaaagcaaaattttggactgtgaagcaaggcactgggcaaacacaacatggcctccccggctgacagctgtatccagtttacccggcacgctagtgatgttcttctcaaccttaatcgcctccggagtcgggacatcttgacggacgttgtcatcgtggtgagccgtgagcagtttagagcccataagacagtgctcatggcctgcagcggcctgttctacagtatcttcactgaccagttgaaatgcaaccttagtgtaatcaatctagatcctgaaatcagccctgaggggttttgcatcctcctggacttcatgtacacatctaggctcaacctgagggaaggcaatatcatggcggtgatgaccacagccatgtacctgcagatggagcatgttgtcgacacatgcaggaagttcatcaaggccagtgaagcagaaatggcccctgcacttaaacctccccgtgaagagttcctgaacagccggatgctgatgccccatgacatcatggcctaccgaggtcgtgaggtcgtggagaacaatatgccactgagaaatactcccgggtgtgagagcagagcttttgctcctcctctgtacagtggcctgtcaacaccaccagcctcttatcccatgtacagccatctcccgctcagcaccttcctcttctctgatgaggagctccgagatgccccccgaatgcctgtggccaacccttttcccaaggagcgtgccctcccctgcgacagtgccaggcaagtccctaatgagtatagcaggccagccatggaggtgtcccccagtttgtgtcacagcaacatctactcgcccaaggaggcagtcccagaggaggctcggagtgacatacactacagtgtgcctgagggccccaagcctgctgtcccttctgctcggaatgctccatacttcccctgtgacaaagccagcaaagaagaagagagaccttcttcggaggatgagattgccctgcatttcgagccccccaatgcacccttgaaccggaagggtctggttagtccccagagtccccagaaatccgactgccagcccaactcacccacagagtcctgcagcagcaagaacgcctgcatccttcaggcctctggctctccgccagccaagagccccactgacccgaaagcctgcaactggaagaagtataagttcatcgttctcaacagcctcaatcagaatgccaaacccgagggctctgagcaggcagagctgggtcgcctctcccctcgagcctaccctgcaccgcccgcttgccagccgcctatggagcccgcgaaccttgatctccagtccccgaccaagctcagtgccagtggggaggactctaccatcccccaagccagccggctcaataatctcgtgaacaggtccctggcaggctccccccgaagcagcagtgagagtcactcaccactctacatgcaccccccaaagtgcacatcctgcggctctcagtccccacagcatacagagatgtgcctccatactgctgggcccacgttcccggaggagatgggggaaacccagtcagagtattcggattctagctgtgagaatgggaccttcttctgcaacgaatgtgactgccgtttctctgaggaggcctcgctcaagaggcacacgctgcagacgcacagtgacaaaccatacaaatgtgatcgctgccaggcctccttccgctacaagggcaacctcgccagccacaagactgtccacacgggtgagaaaccctatcgctgtaacatttgtggagcgcagttcaatcggccagccaacctgaagacccacactcgaattcactctggagaaaagccctacaaatgtgaaacctgtggggccaggtttgttcaggtggcccacctccgtgcccacgtgctcatccacactggagagaagccgtacccctgtgaaatctgtggcactcgcttccggcaccttcagactctgaagagccatctgcgcatccacacaggagagaaaccttaccattgtgagaagtgtaacctgcactttcgtcacaaaagccaactgcgacttcatttgcgccagaagcacggcgccatcaccaacaccaaggtgcaataccgcgtgtcggccgctgacctgcctccggagctccccaaagcctgctgaatgaagcatggagtgttcctcgccctttcctctccagccccttctcagaatctacccaaaggatgctgtaacactttatacaaaggtcatcccatgatgtagtgcctctctcatccactagtgcaaatcatagttggggtgggggtgggggtggggtttgcgggaccgggagccaaggcagctccccttcccacactgccataaaacattaagaaaatactattgcttcttctcctatgtgtaaggcaaaccctgtcagcaaaaagcaaattcattttctatatcaaagtaggggagaatgcagaagttctgacttgacaggttgcaaccgaggaatgtaaatgatgtgtgggaacagaggtctcttttgtatgtaaatgtgtattgttttaaaagacaagacttcagtatgctgtcaaagagaaggctttaatttttttaaccaaaggtgaaggaatatatggcagagttgtaaatatataaatatatatatatataatataaatatataaacctaaaaagatatattgaaaatataaaactgtgttaaaggctcgattttgtatctgcaggcagacacggatctgagaatctttattgagaaagagcacttaagagactattttaagtattgcgtctgtataagtaagaaaatattttgtctaaaatgcctccgtgtatttgtatttttttgcaagtgaaggtttacaaatttacaaagtgtgtattaaaaacaaaaagaacaaaaaaaaaagctgcagaaggagaaatgtatacttttgttccagttttcagtttgtacatacctgtaatgtgtcctcacggtgcctttttacacggaagttttcaatgatggacgggtgtgcgccatccctttttgaagtgtaggcagacacagggacttgaagttgtcactaactaaactctctttgggaatgtttgactcctcccacattctgcgtcatgcttgtcgttataattactccggagacagggtttggctgtgtctaaactgcattagtgcgttgtaaaatagagctgtacaaaacataagaataaaacattgaaaagtcga

SEQ ID NO: 35 - DNA, 3623 bp, Homo sapiens
  Human L-MYC (NM_001033081.2)
aatgcgcctgcagctcgcgctcccgcgccgatcccgagagcgtccgggccgccgtgcgcgagcgagggagggcgcgcgcgcggggggggcgcgcttgtgagtgcgggccgcgctctcggcggcgcgcatgtgcgtgtgtgctggctgccgggctgccccgagccggcggggagccggtccgctccaggtggcgggcggctggagcgagggaggctgcgggtggccagggcacgggcgcgggtcccgcggtgcgggctggctgcaggctgccttctgggcacggcgcgcccccgcccggccccgccgggccctgggagctgcgctccgggcggcgctggcaaagtttgctttgaactcgctgcccacagtcgggtccgcgcgctgcgattggcttcccctaccactctgacccggggcccggcttcccgggacgcgaggactgggcgcaggctgcaagctggtggggttggggaggaacgagagcccggcagccgactgtgccgagggacccggggacacctccttcgcccggccggcacccggtcagcacgtccccccttccctcccgcagggagcggacatggactacgactcgtaccagcactatttctacgactatgactgcggggaggatttctaccgctccacggcgcccagcgaggacatctggaagaaattcgagctggtgccatcgccccccacgtcgccgccctggggcttgggtcccggcgcaggggacccggcccccgggattggtcccccggagccgtggcccggagggtgcaccggagacgaagcggaatcccggggccactcgaaaggctggggcaggaactacgcctccatcatacgccgtgactgcatgtggagcggcttctcggcccgggaacggctggagagagctgtgagcgaccggctcgctcctggcgcgccccgggggaacccgcccaaggcgtccgccgccccggactgcactcccagcctcgaagccggcaacccggcgcccgccgccccctgtccgctgggcgaacccaagacccaggcctgctccgggtccgagagcccaagcgactcggagaatgaagaaattgatgttgtgacagtagagaagaggcagtctctgggtattcggaagccggtcaccatcacggtgcgagcagaccccctggatccctgcatgaagcatttccacatctccatccatcagcaacagcacaactatgctgcccgttttcctccagaaagctgctcccaagaagaggcttcagagaggggtccccaagaagaggttctggagagagatgctgcaggggaaaaggaagatgaggaggatgaagagattgtgagtcccccacctgtagaaagtgaggctgcccagtcctgccaccccaaacctgtcagttctgatactgaggatgtgaccaagaggaagaatcacaacttcctggagcgcaagaggcggaatgacctgcgttcgcgattcttggcgctgagggaccaggtgcccaccctggccagctgctccaaggcccccaaagtagtgatcctaagcaaggccttggaatacttgcaagccctggtgggggctgagaagaggatggctacagagaaaagacagctccgatgccggcagcagcagttgcagaaaagaattgcatacctcactggctactaactgaccaaaaagcctgacagttctgtcttacgaagacacaagtttattttttaacctccctctcccctttagtaatttgcacattttggttatggtgggacagtctggacagtagatcccagaatgcattgcagccggtgcacacacaataaaggcttgcattcttggaaaccttgaaacccagctctccctcttccctgactcatgggagtgctgtatgttctctggcgcctttggcttcccagcaggcagctgactgaggagccttggggtctgcctagctcactagctctgaagaaaaggctgacagatgctatgcaacaggtggtggatgttgtcaggggctccagcctgcatgaaatctcacactctgcatgagctttaggctaggaaaggatgctcccaactggtgtctctggggtgatgcaaggacagctgggcctggatgctctccctgaggctcctttttccagaagacacacgagctgtcttgggtgaagacaagcttgcagacttgatcaacattgaccattacctcactgtcagacactttacagtagccaaggagttggaaacctttatatattatgatgttagctgacccccttcctcccactcccaatgctgcgaccctgggaacacttaaaaagcttggcctctagattctttgtctcagagccctctgggctctctcctctgagggagggacctttctttcctcacaagggacttttttgttccattatgccttgttatgcaatgggctctacagcaccctttcccacaggtcagaaatatttccccaagacacagggaaatcggtcctagcctggggcctggggatagcttggagtcctggcccatgaacttgatccctgcccaggtgttttccgaggggcacttgaggcccagtcttttctcaaggcaggtgtaagacacctcagagggagaactgtactgctgcctctttcccacctgcctcatctcaatccttgagcggcaagtttgaagttcttctggaaccatgcaaatctgtcctcctcatgcaattccaaggagcttgctggctctgcagccacccttgggccccttccagcctgccatgaatcagatatctttcccagaatctgggcgtttctgaagttttggggagagctgttgggactcatccagtgctccagaaggtggacttgcttctggtgggttttaaaggagcctccaggagatatgcttagccaaccatgatggattttaccccagctggactcggcagctccaagtggaatccacgtgcagcttctagtctgggaaagtcacccaacctagcagttgtcatgtgggtaacctcaggcacctctaagcctgtcctggaagaaggaccagcagcccctccagaactctgcccaggacagcaggtgcctgctggctctgggtttggaagttggggtgggtagggggtggtaagtactatatatggctctggaaaaccagctgctacttccaaatctattgtccataatggtttctttctgaggttgcttcttggcctcagaggaccccaggggatgtttggaaatagcctctctacccttctggagcatggtttacaaaagccagctgacttctggaattgtctatggaggacagtttgggtgtaggttactgatgtctcaactgaatagcttgtgttttataagctgctgttggctattatgctgggggagtcttttttttttatattgtatttttgtatgccttttgcaaagtggtgttaactgtttttgtacaaggaaaaaaactcttggggcaatttcctgttgcaagggtctgatttattttgaaaggcaagttcacctgaaattttgtatttagttgtgattactgattgcctgattttaaaatgttgccttctgggacatcttctaataaaagatttctcaaacatgtc

SEQ ID NO: 36 - DNA, 3686 bp, Mus <mouse, genus>
  Mouse L-myc (NM_008506.3)
agtcgggaaacaatgcgcctgcagatcgcgctcccgcgtcgatcccgggagcgtcctggctgccgtgtgcgagcgaggcggggggcgcgcgcacggggggcgcgctcgtgagtgcggggccgcgcgctcggtggcgcgcatgtgtgtgtgtgcgggctgccgggcttccccgagccggcggggagccgctccgctccaggtggcgggcggcgggagcgaggtgaggctgcgggtggcccgggcaggggtccccaggggactggcgggctgcaaggctgcagactgccttcgagacagcgcgcccccgcccggccctgctgtgcccccggagctgagctccgggcggtgctggcaaagtttgctttgaactcgctcccctcagcctggtcggcccgttgcgagctgccctgagcgagctgaccccaggccaggcttcccaggagcagggaccagggcgcgggctgcaagctggtgggcctggggagagaccagagccccgcagccagctgcagcgagggactcggagccgcctcttccctcggcgggcaccgcagtcagctcgtctcccccttccctcccgcagggagcggacatggacttcgactcgtatcagcactatttctacgactatgactgcggagaggatttctaccgctccacggcgcccagcgaggacatctggaagaaattcgagctggtgccgtcgccccccacgtcgccgccctggggctccggtcccggcgccgtggacccagcctctgggattaatcccggggagccgtggcctggagggggtgccggggacgaggcggaatctcggggccattcgaaagcctggggcaggaattatgcttccatcattcgccgtgactgcatgtggagcggcttctccgcccgagaacggctggagagagtggtgagcgacaggctggccccaggcgcgccccgggggaacccgcccaaagcgcccgctaccccggacggcactcctagtctggaagccagtaacccggcgcccgccacccaatgtcagctgggcgagcccaagactcaggcctgctccgggtccgagagccccagcgattctgaaggtgaagagattgacgtggtgaccgtggagaagaggcgatctctggacatccgaaagccagtcaccatcacggtgcgagcagaccccctggacccctgcatgaagcacttccatatctctatccaccaacagcagcataactatgctgcccgttttcctccagaaagttgctctcaagagggggatcctgagccaggtccccaggaagaggctccggagatagaagctcccaaggagaaagaggaggaggaagaggaagaggaggaagaagagattgtgagccccccacctgtcggaagtgaggctccccagtcctgccaccccaaacctgtcagttctgacactgaggacgtgaccaagaggaagaaccataacttcttggaacgaaaaaggaggaatgacctccgctcccggttcctagccctgcgggaccaggttcccaccctggccagctgctctaaggcccccaaagtcgtgatcctcagcaaggcgttagaatacttgcaggctttggtgggggctgaaaagaaaatggctacagagaaaaggcagctccggtgtcggcaacagcaactgcaaaagagaatcgcgtacctcagtggctactaaccgaccagaacgcctgacttcttggtctcacagacacaagcttattgtttaacctctctctcccttttagtaatttgcacattttggttacagcggggggggcagtctggacagtagatcccagaatgcattgcagccggtgtgcgcacacaataagggcttgcattcttggtaacctcgaaacccaattctccctcttccccgaccgactcatgggaatgctgtccttctctggcgcctttggcttctcagcaggcagctactgaggagatttggggtctgcttagctcactagctcctgacgaaaggctgacagatgctatgcaacaggtggtggacgttgttggggctgcagcctacgtgaaatctcacactgtgctggggcttcaggctaggaaaggatgctgctctcactgctgtctctggggatgatctgaggacagctgggcctggatactgtcccccaggctccgttttccaggaggcaagcgagctgtcccgggcgaagacaagctcgcagacttgatcagcatggagcattacctcaccgtcagacactttacagtagctgtggagtggaaacctttaagatagatttggatggtaggccacacccttccctgcacgctcaatgctatgactttgagaaagggcttggcctctatgtagagtctttgtctcagagttctctgggccttctcagagagggacctttctatcctcacaagggacctttttgtttcttcctgcctttgttatgcaatggccaccacagcaccctttcacaccgaccagaaatatttccccaggacatagggaaatgggtcacagcccaggacctggggaagccttggcatccccactcatgaccaacggtccttgcccaggttttctgcagggctatttgaggcccagcttggaaccttttctcgaggcagatagttacaaggtgcctctgaaggacaagccctatcgcttcctctttcccacctgcctctctgtcagatcttgactctgtctacaatctgctggaacagtgcaaacctgtccttctcgagcaactttgctggctctgcagccaccatcctgattctctgccggcctgagtcacatcctttcccctggaatctgggccttacagagagattcagaggggcaccgcttgcattcacctgatgcccccagaaggtaaacttacttcctggtgggttgtcagtgtacctctaggaacgctactcagccaacaaggagagtttgctccagctgtgttctgcaactccctgtggaatcaaagtacagccctctatcctgggaaagtcaccaagctagcagccgtcacgtgagcatctttcaggagatcctaagctttgcctgaaagaagagccagcctttccagaactctacccaggaaagcagatctgttcctgctggccctgggcttggaagtaggggtacagtgtgggggacagacagtaagtaacaacatgtggctctcaaaaaccagctaccacttccaaattggctcccaactgtgatggcctccaattacttcctggcctcaagtcctagaggaagcttcggaagttgctgttgtacctgttggggcaggacttctaggcaccaagggactcctggaactatcttgggaggacaagtggtgaacaggctaaagtctcatctgaatggcttgtgttttataagctgctgcggggttgtatgctgtgggcgtcttttgtttttgtttttgcttttttttttaatactgtatttttgtatgcttttttgcaaagtggtgttaactgtttttgtataagaaaaacaaaaaacaaaaaccctcctgttgcaagggtctggtttattttgaaaggtgcatttacctgaaattttgtatttagttgtaatcattaattgcttgattttaaactgttgccttctgggacatcttctaataaaaagatttctcaaaaaaaaaaaaaaaaaaaaaaaa

SEQ ID NO: 37 - DNA, 5635 bp, Homo sapiens
  Human NR4A3 (NM_006981.3)
ataaatgacgtgccgagagagcgagcgaacgcgcagccgggagagcggagtctcctgcctcccgccccccacccctccagctcctgctcctcctccgctccccatacacagacgcgctcacacccgctccctcactcgcacacacagacacaagcgcgcacacaggctccgcacacacacttcgctctcccgcgcgctcacacccctcttgccctgagcccttgccggtgcagcgcggcgccgcagctggacgcccctcccgggctcactttgcaacgctgacggtgccggcagtggccgtggaggtgggaacagcggcggcatcctcccccctggtcacagcccaagccaggacgcccgcggaacctctcggctgtgctctcccatgagtcgggatcgcagcatcccccaccagccgctcaccgcctccgggagccgctgggcttgtacaccgcagcccttccgggacagcagctgtgactcccccccagtgcagatttcgggacagctctctagaaactcgctctaaagacggaaccgccacagcactcaaagcccactgcggaagagggcagcccggcaagcccgggccctgagcctggacccttagcggtgccgggcagcactgccggcgcttcgcctcgccggacgtccgctcctcctacactctcagcctccgctggagagacccccagccccaccattcagcgcgcaagataccctccagatatgccctgcgtccaagcccaatatagcccttcccctccaggttccagttatgcggcgcagacatacagctcggaatacaccacggagatcatgaaccccgactacaccaagctgaccatggaccttggcagcactgagatcacggctacagccaccacgtccctgcccagcatcagtaccttcgtggagggctactcgagcaactacgaactcaagccttcctgcgtgtaccaaatgcagcggcccttgatcaaagtggaggaggggcgggcgcccagctaccatcaccatcaccaccaccaccaccaccaccaccaccatcaccagcagcagcatcagcagccatccattcctccagcctccagcccggaggacgaggtgctgcccagcacctccatgtacttcaagcagtccccaccgtccacccccaccacgccggccttccccccgcaggcgggggcgttatgggacgaggcactgccctcggcgcccggctgcatcgcacccggcccgctgctggacccgccgatgaaggcggtccccacggtggccggcgcgcgcttcccgctcttccacttcaagccctcgccgccgcatccccccgcgcccagcccggccggcggccaccacctcggctacgacccgacggccgctgccgcgctcagcctgccgctgggagccgcagccgccgcgggcagccaggccgccgcgcttgagagccacccgtacgggctgccgctggccaagagggcggccccgctggccttcccgcctctcggcctcacgccctcccctaccgcgtccagcctgctgggcgagagtcccagcctgccgtcgccgcccagcaggagctcgtcgtctggcgagggcacgtgtgccgtgtgcggggacaacgccgcctgccagcactacggcgtgcgaacctgcgagggctgcaagggctttttcaagagaacagtgcagaaaaatgcaaaatatgtttgcctggcaaataaaaactgcccagtagacaagagacgtcgaaaccgatgtcagtactgtcgatttcagaagtgtctcagtgttggaatggtaaaagaagttgtccgtacagatagtctgaaagggaggagaggtcgtctgccttccaaaccaaagagcccattacaacaggaaccttctcagccctctccaccttctcctccaatctgcatgatgaatgcccttgtccgagctttaacagactcaacacccagagatcttgattattccagatactgtcccactgaccaggctgctgcaggcacagatgctgagcatgtgcaacaattctacaacctcctgacagcctccattgatgtatccagaagctgggcagaaaagattccgggatttactgatctccccaaagaagatcagacattacttattgaatcagcctttttggagctgtttgtcctcagactttccatcaggtcaaacactgctgaagataagtttgtgttctgcaatggacttgtcctgcatcgacttcagtgccttcgtggatttggggagtggctcgactctattaaagacttttccttaaatttgcagagcctgaaccttgatatccaagccttagcctgcctgtcagcactgagcatgatcacagaaagacatgggttaaaagaaccaaagagagtcgaagagctatgcaacaagatcacaagcagtttaaaagaccaccagagtaagggacaggctctggagcccaccgagtccaaggtcctgggtgccctggtagaactgaggaagatctgcaccctgggcctccagcgcatcttctacctgaagctggaagacttggtgtctccaccttccatcattgacaagctcttcctggacaccctacctttctaatcaggagcagtggagcagtgagctgcctcctctcctagcacctgcttgctacgcagcaaagggataggtttggaaacctatcatttcctgtccttccttaagaggaaaagcagctcctgtagaaagcaaagactttcttttttttctggctcttttccttacaacctaaagccagaaaacttgcagagtattgtgttggggttgtgttttatatttaggcattgggggatggggtgggagggggttatagttcatgagggttttctaagaaattgctaacaaagcacttttggacaatgctatcccagcaggaaaaaaaaggataatataactgttttaaaactctttctggggaatccaattatagttgctttgtatttaaaaacaagaacagccaagggttgttcgccagggtaggatgtgtcttaaagattggtcccttgaaaatatgcttcctgtatcaaaggtacgtatgtggtgcaaacaaggcagaaacttccttttaatttccttcttcctttattttaacaaatggtgaaagatggaggattacctacaaatcagacatggcaaaacaataatggctgtttgcttccataaacaagtgcaattttttaaagtgctgtcttactaagtcttgtttattaactctcctttattctatatggaaataaaaaggaggcagtcatgttagcaaatgacacgttaatatccctagcagaggctgtgttcaccttccctgtcgatcccttctgaggtatggcccatccaagacttttaggccattcttgatggaaccagatccctgccctgactgtccagctatcctgaaagtggatcagattataaactggattacatgtaactgttttggttgtgttctatcaaccccaccagagttccctaaacttgcttcagttatagtaactgactggtatattcattcagaagcgccataagtcagttgagtatttgatccctagataagaacatgcaaatcagcaggaactggtcatacagggtaagcaccagggacaataaggatttttatagatataatttaatttttgttattggttaaggagacaattttggagagcaagcaaatctttttaaaaaatagtatgaatgtgaatactagaaaagatttaaaaaatagtatgagtgtgagtactaggaaggattagtgggctgcgtttcaacattccgtgttcgtactcccttttgtatgtttctactgttaatgccatattactatgagataatttgttgcatagtgtccttatttgtataaacatttgtatgcacgttatattgtaatagctttgcctgtatttattgcaagaccaccagctcctggaagctgagttacagagtaattaaatggggtgttcacagtgacttggatacaccaattagaaattaaataagcaaatatatatatatatataaatatagcaggttacatatatatatttataatgtgtctttttattaaccatttgtacaataaatgtcacttcccatgccgttattttatggttcatttgcagtgacttttaaggcagtactgtttagcactttgatattaaaattttgcttatgttttgctaaattcgaataatgtttgaagatttttaggtctaaaagtctttatattatatactctgtatcaagtcaaaatatctttggccattttgctaagaaacaaactttgaatgtcaaactgatgtcacagtagtttttgttagctttaaatcatttttgctttagtctttttaaaggaaaataacaaaactatgctgtttatattgtcattaaattatacaatcaaacaaatgccaaatgaattgcctaattgctgcaaagtataacccagataggaaatcatatgtttttttccaagagtcattctaatatttgattatgttatgtgtgcttttatgaaagattgttatttttatatatcaagatgatagaacctggaatgttaggattttgaaatgttagacttggaaggggcctggtctgtcaactagtccaaccccttaaaattcatagaggagcaaactggggcccattgaagggtgaagagttactcaaggtcaaacagctggtaacagaatcaagactaagacctaatttacctttccatactctttttttttctcaacttcatctatataaaatcaggcttttaaacataaccactaatatttacctgaagataaccatgagtaaagtatacttttgcattaattttttgagcttatatgcaaacataataaatattattaaatatcaggaaagctaacatttcatacaagatagcttcagaccaaattcaaattgaatttgaataaattagaaatactgtgcatacataaccttcttgtgcaccatgagtatttggaaagttaatccttgtttttgtcgtgtctataaaggaagaacaaaacaaaataaaaacagagccctagagaaatgctgttactttttatttttacacccatcagatttaaggaaaagactttttagccattataatctagtggttggaaggaatgaagaagcttttttagtaataggtccagatatgagtgctaaaaataaagatgatagcatgttcttctgtcttccatagttattacaactatgagagcctcccaagtcatcttatcaactcaactcccttttttttgtcttaatgttgcacataagtttatacagagtggatgaccacactagcacagaagagaacaacatgtattaaagcaggtgattcctccccttggcgggagagctctctcagtgtgaacatgccttctgtgggcggaaatcaggaagccaccagctgttaatggagagtgccttgcttttatttcagacagcagagttttccaaagtttctctgctcctctaacagcattgctctttagtgtgtgttaacctgtggtttgaaagaaatgctcttgtacattaacaatgtaaatttaaatgattaaattacattttatcaatggca

SEQ ID NO: 38 - DNA, 5573 bp, Mus <mouse, genus>
  Mouse Nr4a3 (NM_015743.3)
cacacgcgcgctcacacgctccgcacacacactccactctctcccgcgcgctcacacccctctcacccggctccctcgccagtgtcgcgccgcgccgcgccgcagccggacgcccctccagggctcactttgcaacgctgacagagcccgcagtgtccgtggaggtgggaaacgtggcgacatcctaccccctggtcgcagccggagactggatgcctgcggaacctctcggcggcgctctcccatgagttgggatcgcagcatcccccgccagccgctcaccgcctctgggagccgctgggtttgtgcaccgcagcccttccgggacagcagctgtgactctcccccaatccagatttcggggtcgctctctagaaactcgctctaaagacggaaccgccacagcacccaaagcccactgcgggagagcgcagcccgacaagcccgggcgctgagcctggaccctcagcagagcgggccagcacagcggctgctgcttcgcctatcccgacgtccccgcctcctacactctcagcctccgctggagagacccccagccccaccattcagcgcgcaagataccctccagatatgccctgcgtgcaagcccagtatagcccttcacctccggggtccacttacgccacgcagacttatggctcggaatacaccacagaaatcatgaaccccgactacaccaagctgaccatggacctcggtagcacggggatcatggccaccgccactacatccctgcccagcttcagtaccttcatggagggctaccccagcagctgcgaactcaagccctcctgcctgtaccaaatgccgccttctgggcctcggcctttgatcaagatggaagagggtcgcgagcatggctaccaccaccaccatcaccatcaccatcatcaccaccaccaccagcaacagcagccgtccattcctcctccctccggccccgaggacgaggtactgcccagcacctccatgtacttcaagcagtctccgccttctacaccgaccactccaggcttccccccgcaggcgggggcgctgtgggacgacgagctgccctctgcgcctggctgcatcgctccgggaccgctgctggacccgcagatgaaggcggtaccccccatggccgctgctgcgcgcttcccgatcttcttcaagccctcaccgccacaccctcccgcgcccagtccagccggcggccaccacctcggctatgaccccacggccgcagctgcactcagtctgcccctgggagccgcggccgcagcaggcagccaagctgctgcgctcgagggccacccatacgggctcccgctggccaagaggacggccacgctgaccttccctccgctgggcctcacagcctcccccaccgcgtccagcctgctgggagagagccccagcctcccatcgccacccaataggagctcatcatctggggaaggcacatgtgccgtgtgcggcgacaacgctgcctgccagcactacggagtccgcacctgcgagggctgcaagggcttcttcaagagaacggtgcagaaaaatgcaaaatatgtttgcctggcaaataaaaactgcccagtggacaagagacgccgaaaccgatgtcagtactgcagatttcagaagtgtctcagtgtcgggatggttaaggaagttgtgcgtacagacagtctgaaagggaggagaggtcgtctgccttccaaaccaaagagcccactacaacaggagccctcgcagccctccccgccatctcctccgatctgtatgatgaatgcccttgtccgagctttaacagatgcaacacccagagatcttgattattccagatactgtcccaccgaccaggccactgcaggcacagatgctgagcacgtgcaacagttctacaaccttctgacggcctccattgacgtgtccagaagctgggcagaaaagatcccaggattcactgatctccccaaagaagatcagacgttacttatagaatcagcctttttggagctgtttgttcttagactttccatcaggtcaaacactgctgaagataagtttgtgttctgcaatggacttgtcctgcatcgacttcagtgccttcgaggatttggggagtggctcgactccattaaagacttttctttaaacttgcagagcctgaaccttgatatccaagccttagcctgcctgtcagcactgagtatgatcacagagcgacatgggttaaaagaaccaaagagagtggaggagctatgcaccaagatcacaagcagcttaaaggaccaccagaggaagggacaggctctggagccctcggagcctaaggtcctgcgcgcgctggtagaactgagaaagatctgtacccagggcctccagcgcatcttctacctgaagctagaggacttggtacctccaccttctgtcatcgacaagctcttccttgacaccctgcctttctgagcaggggaagcctgagcagagagctacttgctctgctggcacctgatcattaagtgagcaaaagaatgggtttgaacaccttccacactcactgtccttccttcaggggaaaagcagctcccgtagaaagcaaagacttttttttcttttcctggcacctttccttacaacctaaagccagaaaccttgcagagtatcgtgttggggttgtgttttatatttaggctttggtgggtgggttgggagggggtaaatagttcatgaggcttttctaagaaattgctgacaaagcacttttggatgatgctatcccagcagtggggtggggagaaaggataatataactgttttgtttttgtttttgtttttgtttttaaaaaaaaactctttctggggaatatgattatggttgctttgtatttaaaaataagaacagccaagggctgttcaccagggtagggctgtgtcctacgacggatccctttaggatatacttcctgtgtcaagggtagatacgtggtgcaaatgaggcagaaaattcccttttcttcatttctttcttaaaaaaatggcaaaagatgaaagattatctacaaatcagacttagcaaaaatgataatggctatttgcttccatatacaagtgcaattttttagagtgctgtcttactaagtcttgtttgtgaactcccccttattttacatgaaaataagaaggaggcagtcatgctatgaaatggcgcgctcattttcctagctaaggcttgatccacctgccctgtagaacccttcggaggtgtggcccttctaagactttcaggccattctcgatggaattcgacccctgatgactatccagccatcctgaagggggatcgggttataaagtggattgcatacaactgtcttcgctgtgttttgtcaacctggacagagttctctaaacctacttcagttgtagcaagttcctgattcatccactcagaagcccaatgagcactggttgactcaatcaagtgttaaccctaggagaacaagcaaataagtaggaactgggtcatacagggtaaacaccagagatgataaggatatatatatatatatatatatatatatatatatatatatgtatatgtatatatatatacatattaatttttgttattggttagagacaattttggaaagcaagagaatcatctttttttaaaaaagagagaagaagaagaagaaaagatagtattaacgtgagttctagagaaggttagtgggttgcggttcaaaattccgtgtttgtgcccccttttatatgtttctactgttgatgccatattattatgaaatgatttgttgcatagtgtccttatttgtatgaacatttgtatgcacgttatattgtaatagctttgcctgtatttattgcaagaccaccagctcctggaggctgagatacagagtaatcaaatggggtgttcgtggtgacttggatacaccaattagaaattaaataagcatatatatatataaacatagccggttacatatatatttataatgtgtctttttattaaccatttgtacaagaaatgtcacttcccacgcagttactttacccttcacttgcagtgacctttaaggcagcactgtttagcactttgatatgaaatttttgcttatgttttgctaaattctaataatgtttgaagattttaaggtctaaaagtctttatattatatactctgtatcaagtcaagatccctttggccgttttgctaagactcaaaaactttgaatgtcaaactgatgtcacagtagcttttgttagcttttaatcatttttgctttagttttttttttaaaaaaaataacaaactatactgtttatattgtcattaaattatacaatcaaacaaatgccaaatgaattgcctaattgctgcaaagtgtaacccagataacaaatcatattctctcctctttttgcaactcattcagatgtttgatcttgtgttttgtttgtataaagattgtatgaactatatcaccttcctatcaaggtgacagggcttgagatgttaagatttttgaacttcagacttggaaggggcctggctcatcatctggtcagatctattaaaattcacaaaggagaaaagtgggggcccgttgcagggcaaacagctagcaacaggataaaggctcagacttaattcaccttcccttagtctcccccacatcttactgcatctgtaggaaaataaacttttaaacatagtcacgcatactaacactttaccagcagacagccttgaataaagtagtactttggcattaatttgttgagcttatatgcaaacataataaacattattaaatatcaggaaagctaacatttcacacgagatcgcttcagaccaaattcaatttgaatttgaataaattagaagtactgagcgtacgtaaccttcttgtgcaccttgagtattgcaaagttgctccttggttgttggttttttttgttgtttcttttcgtcctgtctgaaaggcaaagcaaaacagcagcacggtgctctgggaaatgctgttcccccttctgtcctcacacccacagattgaagggaaagaactgtctaagcatctatctgctggtttgaagaatgatgaagccgttttagttaagggccagacactagtgctgaaagaaaagactatacagccagtgttcttctgtcttccatagttatcacaactatgagagcctcttaggtcatcattttgaaatgttgacacccaagtgtacccagagtggaaggcacactagctctgcagaggacaagcattaatgcaggtgattcctcccgctgactggagtgcagtctcagtgtgaacccgccctcagcaggaaatgggaatccacttgctgttcctggagagtgccttgcttttgtttcaaatggccgagtctcccaagcccttctcctctaacagcattgctttttagtaagtgtgtgttaacctgtggtttgaaagaaatgctcttgtacattaacaatgtaaatttaaatgattaaattaaattacattttaccaatggaaaa

SEQ ID NO: 39 - DNA, 5989 bp, Homo sapiens
  Human ETV6 (NM_001987.4)
gcgtcccgggtccccgcgccgcgccgcgacctgcagaccccgccgccgcgctcgggcccgtctcccacgcccccgccgccccgcgcgcccaactccgccggccgccccgccccgccccgcgcgctccagacccccggggcggctgccgggagagatgctggaagaaacttcttaaatgaccgcgtctggctggccgtggagcctttctgggttggggagaggaaaggaaagtggaaaaaacctgagaacttcctgatctctctcgctgtgagacatgtctgagactcctgctcagtgtagcattaagcaggaacgaatttcatatacacctccagagagcccagtgccgagttacgcttcctcgacgccacttcatgttccagtgcctcgagcgctcaggatggaggaagactcgatccgcctgcctgcgcacctgcgcttgcagccaatttactggagcagggatgacgtagcccagtggctcaagtgggctgaaaatgagttttctttaaggccaattgacagcaacacgtttgaaatgaatggcaaagctctcctgctgctgaccaaagaggactttcgctatcgatctcctcattcaggtgatgtgctctatgaactccttcagcatattctgaagcagaggaaacctcggattcttttttcaccattcttccaccctggaaactctatacacacacagccggaggtcatactgcatcagaaccatgaagaagataactgtgtccagaggacccccaggccatccgtggataatgtgcaccataaccctcccaccattgaactgttgcaccgctccaggtcacctatcacgacaaatcaccggccttctcctgaccccgagcagcggcccctccggtcccccctggacaacatgatccgccgcctctccccggctgagagagctcagggacccaggccgcaccaggagaacaaccaccaggagtcctaccctctgtcagtgtctcccatggagaataatcactgcccagcgtcctccgagtcccacccgaagccatccagcccccggcaggagagcacacgcgtgatccagctgatgcccagccccatcatgcaccctctgatcctgaacccccggcactccgtggatttcaaacagtccaggctctccgaggacgggctgcatagggaagggaagcccatcaacctctctcatcgggaagacctggcttacatgaaccacatcatggtctctgtctccccgcctgaagagcacgccatgcccattgggagaatagcagactgtagactgctttgggattacgtctatcagttgctttctgacagccggtacgaaaacttcatccgatgggaggacaaagaatccaaaatattccggatagtggatcccaacggactggctcgactgtggggaaaccataagaacagaacaaacatgacctatgagaaaatgtccagagccctgcgccactactacaaactaaacattatcaggaaggagccaggacaaaggcttttgttcaggtttatgaaaaccccagatgaaatcatgagtggccgaacagaccgtctggagcacctagagtcccaggagctggatgaacaaatataccaagaagatgaatgctgaaggaaccaacagtccacctcagcgggccagcagcccagggaacccctgcccaccaggattgctggaagtgtgacggagcaggcgggctgaggagagtggaaaaggaagcgacccagaaatggcagggacacttctcttgcagaccaagagggaccctggagcaccttagacaaactacccagcacaggcggggctggaattctggcggagggcatgagcctgggactccatgtcacgtttccttctgatttggaatctctccatctgtaattcctcaccctcacccttccaccgttgttagtatcatggtgtttttgtttttgtttttgttttaagaacctgcagtttgactcttcatcgttcatctaggggaagacatctgatgttgttttcctatggaaatatatatctattatatatatattttttgcaaatctcacaaagtgcggcaagcccagctggtcaggaaagagaatacttgcagaggggttcaggttcctctttttcctgccacgtggatcaggtctgttcctgttactgttgggtcttggctgaaaaaaaaaaatgcttttaaaaaagataaaatgaaaaggagagctctctttttctctctcttgctctgttcttcccttggtcccctctgtcctcccgccctgcctgcagttgagattcagatgccttctgacagagttcagcctcttggagagtcttggggattgttggcacctaaacagaatcagtgacccgggtgctttgtggccagcagcacagaatcaaacccgcatcccagcattgggccacccatctgagggaggccaaaatcatcacagatgctgctgtgctgcagacagatacatgctagtccagagagccgcccctgagatggctgtgagaaccatgtgtctaaggcgtaagataaggatggaaggctgtccaagttatttggaaggcctcggcagcttgggattagcttgggagcgcagcgctgcaaagtggaaaatatgaaaagaccacacaggcccagcagtccagaaactgggcaaaaatattctgcagtggggatttatttttccaaagcaggtaacagaggctagtgagaaagaaaagctcctctctgctccattccaaaggccatcttgtggtcagtttcatgccctcacctgatttttttttttttttttttttttcaattcctaaccttttttaaagtttcctggtctccactggacacagagctttggagacggaggatcccagagggcagtctcagttgcaatcagtgtgtgcccagcctgggcagacaggaaattcctcggatacattattttttctttctttcatagctgtgtctcagaaaggacccatttgtggctctttttcacctcaaaataagatcgatggtatcttgtaaaatgagggtagtgccacttcttagtatttttgaaagctgttttagattttttttttttttccttttctagccatctaaattgactcttccaatataggtctcagaaatccaatatttggagtacaatttcttttaatccagattacacctgccttacaaagcaccccctccttgttcccctctgtttcctctactcagttgggggagaaactcacagctcctccgggatacatatgtgccctcagcagcagctcccaggtgaagttaccagacccctgggcttctccccagctttttctgagttgagtcagacatgtagagtttgggtcacacaggcaagaggaattttccctcggccttactgacaaggacaccaacctagggtgcaaacagatggactatggttcaaggacactggaattgaggagctgatcaaggctctcttcagccttgctctgtccctgcctcttatcagagcacaggtagacacacgggcatagccagcccactcctactgtcacaggcgccccaccattcaaccttccgggaggtcagggaccttctatatgaggcgagtgggtctcagtctgcttgaatggtgatgagattctgctggatctcagcacgctgcaggtgtcttttgagagcattcagtaggacatggtgatccctatttcagcctctaagatgactggtattctatctgaaatgcagagattaagccaaatacctgatgtattgtgaaagccactgattttaagaatggagagaaagggattttttactgcatccctctgtatgaatatgaaatcagagaccagggcatgatgttgctaggattagagcctctcagtctggcctcttcacccaagtgcaagaactcagtctcttactgttcaaagaatcttaacagttgaattatggagggaaattcccttttgccccaagcatttctatatttaaagcaatatcccaggagaatatgttagacttaggatgataccttcagccacttgaagaagaaatagaaggcgctcattccaatatagtctttatttcccattcagatacaggttgagcatccctaatctgaacagttaaaacccccaaatgccccaaaatccaaaccttcctgaacgctatgacaccatgagtggaaaattccacacctaacaaacacatttgctttcttatggttcaatgtacacaaactgttttatatagaaaatgatttcaaatatcataaaattaccttcaggctatgtgtataaagtatatatgagccataaatgaattttgtgtttagactttgtgtccatccccaagatctctcattttatatatatatatatatatatatatatatatatatatatatatatatacacacacacacacatacacaaatattccaggatacaaaaaaaaacatttaaaaatccgagacccagaacacttctggtcccaagcatttcagataagggatatcaatctgtactaccaataaggatttcgtaattcccctaactgcaaatgtcctcttcatttgttctttatgagaaaacccgggtagtgccagcacctggatacagtatttacaccctgcagaccctaaagatttcagattcagttagcaaaccttgatgaagcacctgctggacactgagggacccaaagctcaatcagccataatccctgctttcagagtttatattgtacctgcctaatccacccggcgtgactcatttcaacactaagtactaggggtgttgtcaggagacaaatctgaagtcaggagaggaaaatgcaaaggagccctgccgtgtgatggatgtgcattctcacttgggtcttgaagttctcattcctacatctcaagctagccaggcagtctcctctctatcagaagaaagcactggtaattggctagactggctatgttgaaggtaacatgaactctaagatcttgacccagggcgacttggttttgcttaaggtggcatcaccaatgttccaaatcctttagggagatgagggtatccccacagaaaaagaggaataatagaccaatggattttctcctttcaccagtatgtttggaaccctctgatccaatgtcttttgatactgatctcttgtccaaatgagaatgtcgctttagctgaaattcaaatggctgtgacaatttaccgaaatgatgaagtaaccaccattcccacctttcactgcctaggctccaagtctgaatacatttttgaaataggaactcccttttgcaaaaaagaaacctgggtgtcagggaggtgaagtgacttgccctaggagcagacagcatgccaagaatggaattaggctcaggatccagcctgggctcaccctgtgtggctcattcccacccaggaaactgaagataaaagatttgggaaaacacaccaagaaaaaggggcagttttctttgcccaagcatttggtgctagttagaggctgttcactctctcctgctcctcttcggagtagaaataaaggctgtgacacaaggaagccagtggggtgggagggaggcaccataatccctccctaaaacccacagaagactaacctgatactcttttgacccaactgcatcaacactaaacagctgcagaccccctgaatctttcacacatgccaagtgaacattcttgatgatttctctttgtgaccgcaaccacctgcaaaccagaacgactctagaatttccttccccgcccccctttttgtttagtttctaatctcttgtttatgaggtgtggggtttataagggactgaatcaaatgaatgtaacaaaaaagaaaaaaaaaacaaaaaaaaatgccttttctcagggccagtgagttgcaaataatttttaaagaaaagcctataattacatcatctcaataaattttttataaaaaaaaaaaaa

SEQ ID NO: 40 - DNA, 5548 bp, Mus <mouse, genus>
  Mouse ETV6 (NM_007961.4)
ttctgcctttcagtttctctcttccaggaaggaaaacattcgagaaagagagagggagggagggagcgagggagcgagagagcgagcgagcgagcgccgcgggagggcgggcgcgccggccgcgggtgggaggagacacgccaggccggcctgctgcgcccgggtcgccgcgccgcgacccgcacaccccacgccgtgctcgccggctcctacgcccccgcacctcgcgcccaatccgcgcgttgagaagagccccccctccccctcgggcggccgccgccagcgatgctgcaagaaacttcttaaacgaccgcatcccgctgccccgccgagcgtttctgggttggggagaggaaaggaaagtggaaaaaaactgagaacttcctgatccctttcgctgtgagacatgtctgagactcctgctcagtctagcattaagcaggaacgaatttcatacacgcccccagagagtccagtggcaagccaccgttcctcgactccgcttcatgttcacacagtgcctcgagcgctcaggatggaggaagactcgatccacctgccaacacacctgcgtttgcagccgatttactggagcagagatgacgtagcccagtggctcaagtgggcagaaaatgagttttctttaaggcccattgagagcaacaagttcgaaatgaatggcaaggccctcctgctgctgaccaaagaggatttccgctaccgatctcctcattcaggcgacgtgctctatgaactccttcagcatatcctgaagcagaggaaatctcgaatgctcttctcaccattcttcccccctggggactctatccacaccaagccagaggtcctcctgcatcagaaccatgacgaagataactgtgtccagaggacacccaggacgcccgcggagagcgtgcaccacaaccctcccaccatcgaactcttacatcgccctaggtcacccatcaccacaaaccacaggccttctcctgaccccgaacagcagcggccccagcggtcccccctagacaacatgagccgccgcctctcgccagtggagaaagcccaggggcccaggctacagcaggagaacaaccaccaggaaacgtaccccctgtcagtgtctcctgtcgagaataatcactgcctgccctcaagcccctggcaggagagcactcgagtgatccagctgatgcccagccccatcatgcaccctttgatcctgaacccccggcactcgcactcggtggacttcaaacagtcccggcactccgaggatgggatgaatcgggaagggaagcccatcaacctgtctcatcgggaggacctggcttacttgaaccacatcatggtctctatgtccccaccggaagagcacgccatgcccattgggagaatagcagactgtagactgctttgggattatgtctatcagttgctgtctgacagccggtacgaaaacttcatccgatgggaggacaaagaatccaaaatattccggatagtggatcccaacggactggctcgactctggggaaaccataagaacagaacaaacatgacctatgagaaaatgtccagagccctgcgccactactacaaactaaacattatcaggaaggagcccggacaaaggcttttgttcaggttcatgaaaaccccagatgagatcatgagtggccggacagaccgtctagaacacctcgagtctcaagtgctggatgaacaaacgtaccaagaggatgaacctaccatagcctcaccggtgggctggccaagaggaaacctgcccacggggaccgcaggaggcgtgatggaagcaggcgagctaggggtggctgtaaaggaagagacccgggaatagcagggacacttctcctgccgatcaagagggacccagagcaccttagacaagccaccgagcaatggcagggctgaagttctggcggagggcacaagcctgagactcacacgtcacgttcgcttctccttctgatctcttgtctgtaactctcaccctctcccttcccctacacctgttgtagtctcatggtgtttctggtttcgttttttgtttttgttttttaagaacatgcagtttgactattcattgttcatacagggaagacatcacatgttgttttcctatggaaatatatctattatatatatattattaatttttttgttgttgttgcaaatctcaccaagtacggccagcttggctggtcaggaaagagaaaacttgcagaaggaatcaggttcctctttttcctgccacatagatctggtgtgtcctgtccaagtcaggtcttagatgagaaaggaaaacaaaatgagagagatactttcaaacaatggaaaagaagagttctgtctccatctccctctctcgccgctcatccccgcccctttctccttcccccttctctgcctgctatgcacttcacaggcttttcatcagagctagcctcactagcacctgaactacacagtgacccggctgctctgtgacagtcagaccccttgggcacccatctgaggaaggccagacatctccccccaccaaatgctgctgtattctagaaagaacaatgggaggatcgagcataagataggacagagggtggccacaggatttgcaaggcccaggcagtttgggattgtcctgaaagtgctacacattaggaaaatatgagagaccacacaggcctggtagtttaggagcaagaacaggtcaccaatgttgtcccaagacatcatgcccttgtgggattgtcaccaccccacacacacactccaagtcctagcctttttcttctatgctggtcctcatggaacacagaacacacatgagggaggatgctggaatttagtctcaggcacagccggtatttgcgcagacaggaaattcctcagatttagactttttccttttttccgtctgtcatggctgtatttcaggaggacatatctgtggctcttctccacctcgacataaggtcagtagcatcttccaagatgagggtaatgctattccttaggatttttgatagcagggattttattttatttatttatttatttttgggatttttttttttgagacagggtttttctgtgtatccctggaattcactctgtagaccagactaggactcagagatctacctgcctctgcctcccaagcactgagattaaaggtgtgcgcccccatgcttagctttttttccttttctagccatctaagtggactctttgaagttcactgttttaaaacccagataatgaggcctgcctttcaaaaccaccccttgtccttcctgtgttctcccacatcatggaatgagcctctcccagccctcctgggtgtgtctctgcttggtcagacgcaggacacaggtgaggctgacagaccagagctgacctacaactactcctaagtggggcacatagaggctaggaggacctggacaagtcactctcccgacgtcagctcacaggcggactgtggttcacagacactggaattgagttgactgggtatctttagtcttgctgtgacttccccgtgcctcccccacaacccacaatctgccttcaaagaggtcagtgacctgggtgaggggttccctcttaatattcatggggaatgatgagagtcacgtgctatgtgtttcttgaaagcatgacaggggttcctttttttggcctctaaaaatgactggtaccttatatcaaatggggagattaagccaaatacttgtgttgtatgagccactgggaggaagagcaagtgagaaagggtgtgctttttgtttttgttttgactgaggtcctttgtgtgaatataaaatgagaaactacaacacttcatactggccactttgcccatgcgtagaactcagtcctttaactgcccaaagaattgtccatatgaactgtgtaaggaaattcctctgttccctaaggagtcttggatgacagctttggccacttacgttagaaatgctcatggcagtgccgtctttatttcacacctggtgttgccataattgatttctttgattctcttacctgcaaaagcccttgtttgttttttggagagaaaatatggccagggttgtctgggttgtcagggttgtgcagtgctctcaggcttcagactcacagaatttagatttagccaatcagaccttggaggaaacaccacaatgggggtcctgttttgtctttttggtttttgagttttggttttttgtttgtttgtttttttacaatcaactatgatcttctagatcgacattaaagcgacattaagttcaagaggtgatagaaggaatctaaaagctcctttagtggcctttttctgcagccattgtgggttgagtcaggaaaggaatttgcagggaagcattgccatgtggaggatgggcattgccacctaggtcctgggattctgtcctgagtcctcggccgggctgtcttcaggtctccttcagcagaaaccaggggcagctggtcagatgttgacagcagcttctcttccgataattttcatccaaggccacttagtgccacttggagacagggtccctgatgtcccatatctggttttggaaagagaatggtcctcataagaaaagaacaaaacaggcttcttgcctagtacattcaggtccctctgatccagcatctttttacactaataccttgtccagataagaatgtcactccagctgacatctagatgtctgtgaggagtccctggaatgaccactcttgtcttttcacactgttcgggatccaaccataaacacagtttggcccattcactgttgttggcagaagacaacctgagagaggtcgtgtcactttccgtgggagcagacagcatgacacacagttgggatcagtatctagccggcctgcacttagcagcaggataagcgttcagaaggcagttagaaattattctggtttaaacccccatttgatccatccccggcaaagagacgaaagatgccaagggtggtttttactgcccagtcattcggtgctagttagagctgctgtgcgttctcagcctgctcctcttctgaacagaaaccaaaattggacgtcatgagaaacccagtggagcaggggtacagagggacaccccagaaccctgcctatcaacaaggcacacgggactcacccagcactcttttggccccatccgcatcaacactaaacaacttcaaatgcgcccgactcttttcaccctcacaggtgaaccctcttctggagacttctctttgtgacggcacccacctgcaagccagatgaatctagaatgactttttgttgttgttgttgtttagtttctaatctcttgtttatgaggtgtggggtttataagggactgaatcaaatgaatgtaacaaaaaaagaaaaaaaaacaaacaaaaaatgccttttctcagggccagtgagttgcaaataatttttaaagaaaaacctataattacatcatctcaataaattttttataaaaaaaaaaaaa

SEQ ID NO: 41 - DNA, 5967 bp, Homo sapiens
  Human RUNX1 (NM_001754.4)
ctttgggcctcataaacaaccacagaaccacaagttgggtagcctggcagtgtcagaagtctgaacccagcatagtggtcagcaggcaggacgaatcacactgaatgcaaaccacagggtttcgcagcgtggtaaaagaaatcattgagtcccccgccttcagaagagggtgcattttcaggaggaagcgatggcttcagacagcatatttgagtcatttccttcgtacccacagtgcttcatgagagaatgcatacttggaatgaatccttctagagacgtccacgatgccagcacgagccgccgcttcacgccgccttccaccgcgctgagcccaggcaagatgagcgaggcgttgccgctgggcgccccggacgccggcgctgccctggccggcaagctgaggagcggcgaccgcagcatggtggaggtgctggccgaccacccgggcgagctggtgcgcaccgacagccccaacttcctctgctccgtgctgcctacgcactggcgctgcaacaagaccctgcccatcgctttcaaggtggtggccctaggggatgttccagatggcactctggtcactgtgatggctggcaatgatgaaaactactcggctgagctgagaaatgctaccgcagccatgaagaaccaggttgcaagatttaatgacctcaggtttgtcggtcgaagtggaagagggaaaagcttcactctgaccatcactgtcttcacaaacccaccgcaagtcgccacctaccacagagccatcaaaatcacagtggatgggccccgagaacctcgaagacatcggcagaaactagatgatcagaccaagcccgggagcttgtccttttccgagcggctcagtgaactggagcagctgcggcgcacagccatgagggtcagcccacaccacccagcccccacgcccaaccctcgtgcctccctgaaccactccactgcctttaaccctcagcctcagagtcagatgcaggatacaaggcagatccaaccatccccaccgtggtcctacgatcagtcctaccaatacctgggatccattgcctctccttctgtgcacccagcaacgcccatttcacctggacgtgccagcggcatgacaaccctctctgcagaactttccagtcgactctcaacggcacccgacctgacagcgttcagcgacccgcgccagttccccgcgctgccctccatctccgacccccgcatgcactatccaggcgccttcacctactccccgacgccggtcacctcgggcatcggcatcggcatgtcggccatgggctcggccacgcgctaccacacctacctgccgccgccctaccccggctcgtcgcaagcgcagggaggcccgttccaagccagctcgccctcctaccacctgtactacggcgcctcggccggctcctaccagttctccatggtgggcggcgagcgctcgccgccgcgcatcctgccgccctgcaccaacgcctccaccggctccgcgctgctcaaccccagcctcccgaaccagagcgacgtggtggaggccgagggcagccacagcaactcccccaccaacatggcgccctccgcgcgcctggaggaggccgtgtggaggccctactgaggcgccaggcctggcccggctgggccccgcgggccgccgccttcgcctccgggcgcgcgggcctcctgttcgcgacaagcccgccgggatcccgggccctgggcccggccaccgtcctggggccgagggcgcccgacggccaggatctcgctgtaggtcaggcccgcgcagcctcctgcgcccagaagcccacgccgccgccgtctgctggcgccccggccctcgcggaggtgtccgaggcgacgcacctcgagggtgtccgccggccccagcacccaggggacgcgctggaaagcaaacaggaagattcccggagggaaactgtgaatgcttctgatttagcaatgctgtgaataaaaagaaagattttatacccttgacttaactttttaaccaagttgtttattccaaagagtgtggaattttggttggggtggggggagaggagggatgcaactcgccctgtttggcatctaattcttatttttaatttttccgcaccttatcaattgcaaaatgcgtatttgcatttgggtggtttttatttttatatacgtttatataaatatatataaattgagcttgcttctttcttgctttgaccatggaaagaaatatgattcccttttctttaagttttatttaacttttcttttggacttttgggtagttgtttttttttgttttgttttgtttttttgagaaacagctacagctttgggtcatttttaactactgtattcccacaaggaatccccagatatttatgtatcttgatgttcagacatttatgtgttgataattttttaattatttaaatgtacttatattaagaaaaatatcaagtactacattttcttttgttcttgatagtagccaaagttaaatgtatcacattgaagaaggctagaaaaaaagaatgagtaatgtgatcgcttggttatccagaagtattgtttacattaaactccctttcatgttaatcaaacaagtgagtagctcacgcagcaacgtttttaataggatttttagacactgagggtcactccaaggatcagaagtatggaattttctgccaggctcaacaagggtctcatatctaacttcctccttaaaacagagaaggtcaatctagttccagagggttgaggcaggtgccaataattacatctttggagaggatttgatttctgcccagggatttgctcaccccaaggtcatctgataatttcacagatgctgtgtaacagaacacagccaaagtaaactgtgtaggggagccacatttacataggaaccaaatcaatgaatttaggggttacgattatagcaatttaagggcccaccagaagcaggcctcgaggagtcaatttgcctctgtgtgcctcagtggagacaagtgggaaaacatggtcccacctgtgcgagaccccctgtcctgtgctgctcactcaacaacatctttgtgttgctttcaccaggctgagaccctaccctatggggtatatgggcttttacctgtgcaccagtgtgacaggaaagattcatgtcactactgtccgtggctacaattcaaaggtatccaatgtcgctgtaaattttatggcactatttttattggaggatttggtcagaatgcagttgttgtacaactcataaatactaactgctgattttgacacatgtgtgctccaaatgatctggtggttatttaacgtacctcttaaaattcgttgaaacgatttcaggtcaactctgaagagtatttgaaagcaggacttcagaacagtgtttgatttttattttataaatttaagcattcaaattaggcaaatctttggctgcaggcagcaaaaacagctggacttatttaaaacaacttgtttttgagttttcttatatatatattgattatttgttttacacacatgcagtagcactttggtaagagttaaagagtaaagcagcttatgttgtcaggtcgttcttatctagagaagagctatagcagatctcggacaaactcagaatatattcactttcatttttgacaggattccctccacaactcagtttcatatattattccgtattacatttttgcagctaaattaccataaaatgtcagcaaatgtaaaaatttaatttctgaaaagcaccattagcccatttcccccaaattaaacgtaaatgttttttttcagcacatgttaccatgtctgacctgcaaaaatgctggagaaaaatgaaggaaaaaattatgtttttcagtttaattctgttaactgaagatattccaactcaaaaccagcctcatgctctgattagataatcttttacattgaacctttactctcaaagccatgtgtggagggggcttgtcactattgtaggctcactggattggtcatttagagtttcacagactcttaccagcatatatagtatttaattgtttcaaaaaaaatcaaactgtagttgttttggcgataggtctcacgcaacacatttttgtatgtgtgtgtgtgtgcgtgtgtgtgtgtgtgtgtgaaaaattgcattcattgacttcaggtagattaaggtatctttttattcattgccctcaggaaagttaaggtatcaatgagacccttaagccaatcatgtaataactgcatgtgtctggtccaggagaagtattgaataagccatttctactgcttactcatgtccctatttatgatttcaacatggatacatatttcagttctttctttttctcactatctgaaaatacatttccctccctctcttccccccaatatctccctttttttctctcttcctctatcttccaaaccccactttctccctcctccttttcctgtgttctcttaagcagatagcacatacccccacccagtaccaaatttcagaacacaagaaggtccagttcttcccccttcacataaaggaacatggtttgtcagcctttctcctgtttatgggtttcttccagcagaacagagacattgccaaccatattggatctgcttgctgtccaaaccagcaaactttcctgggcaaatcacaatcagtgagtaaatagacagcctttctgctgccttgggtttctgtgcagataaacagaaatgctctgattagaaaggaaatgaatggttccactcaaatgtcctgcaatttaggattgcagatttctgccttgaaatacctgtttctttgggacattccgtcctgatgatttttatttttgttggtttttatttttggggggaatgacatgtttgggtcttttatacatgaaaatttgtttgacaataatctcacaaaacatattttacatctgaacaaaatgcctttttgtttaccgtagcgtatacatttgttttgggatttttgtgtgtttgttgggaattttgtttttagccaggtcagtattgatgaggctgatcatttggctctttttttccttccagaagagttgcatcaacaaagttaattgtatttatgtatgtaaatagattttaagcttcattataaaatattgttaatgcctataactttttttcaatttttttgtgtgtgtttctaaggactttttcttaggtttgctaaatactgtagggaaaaaaatgcttctttctactttgtttattttagactttaaaatgagctacttcttattcacttttgtaaacagctaatagcatggttccaattttttttaagttcactttttttgttctaggggaaatgaatgtgcaaaaaaagaaaaagaactgttggttatttgtgttattctggatgtataaaaatcaatggaaaaaaataaactttcaaattgaaatgacggtataacacatctactgaaaaagcaacgggaaatgtggtcctatttaagccagcccccacctagggtctatttgtgtggcagttattgggtttggtcacaaaacatcctgaaaattcgtgcgtgggcttctttctccctggtacaaacgtatggaatgcttcttaaaggggaactgtcaagctggtgtcttcagccagatgacatgagagaatatcccagaaccctctctccaaggtgtttctagatagcacaggagagcaggcactgcactgtccacagtccacggtacacagtcgggtgggccgcctcccctctcctgggagcattcgtcgtgcccagcctgagcagggcagctggactgctgctgttcaggagccaccagagccttcctctctttgtaccacagtttcttctgtaaatccagtgttacaatcagtgtgaatggcaaataaacagtttgacaagtacatacaccata

SEQ ID NO: 42 - DNA, 5803 bp, Mus <mouse, genus>
  Mouse Runx1 (NM_001111021.2)
gtgaaaacttctttggacctcataaacaaccacagaaccacaagttgggtagcctggcagtgtcagaagtgtaagcccagcacagtggtcagcaggcaggacgaatcacactgaatgcaaaccacaggctttcgcagagcggtgaaagaaattatagaatcccccgccttcaggagaggtgcgttttcgaaaggaaacgatggcttcagacagcatttttgagtcatttccttcatatccacagtgcttcatgagagatgccagcacgagccgccgcttcacgccgccttccaccgcgctgagccccggcaagatgagcgaggcgctgccgctgggcgccccggatggcggcgccgccctggccagcaagctgaggagcggcgaccgcagcatggtggaggtactagctgaccaccctggcgagctagtgcgcaccgacagccccaacttcctctgctccgtgctacccactcactggcgctgcaacaagaccctgcccatcgctttcaaggtggtggcactgggggacgtcccggatggcactctggtcaccgtcatggcaggcaacgatgaaaactactcggcagaactgagaaatgctaccgcggccatgaagaaccaggtagcgagattcaacgacctcaggtttgtcgggcggagcggtagaggcaagagcttcactctgaccatcaccgtctttacaaatccgccacaagttgccacctaccatagagccatcaaaatcacagtggacggcccccgagaaccccgaagacatcggcagaaactagatgatcagaccaagcccgggagtttgtccttttccgagcggctcagtgaattggagcagctgcggcgcacggccatgagggtcagcccgcaccacccagcccccacgcccaaccctcgggcctccttgaaccactccactgcctttaaccctcagcctcaaagtcagatgcaggatgccaggcagatccagccatccccaccgtggtcctatgaccagtcctaccagtacctgggatccatcacctcttcctctgtccacccagcgacacccatttcacccggccgtgccagcggcatgaccagcctctctgcagaactttccagtcgactctcaacggctccggacctgaccgccttcggcgacccacgccagttccctactctgccgtccatctccgacccgcgcatgcactacccaggcgccttcacctactcgccgcccgtcacgtcgggcatcggcatcggcatgtcagccatgagctcggcctctcgctaccacacctacctgccgccgccctaccccggctcatcacaggcgcaggccgggcccttccagaccggctcgccctcctaccatctatactacggcgcctcggccggttcctaccagttctccatggtgggcggagagagatcgcccccgcgcatcctgccgccctgcaccaacgcatccaccggcgccgcgctgctcaaccccagcctccccagccagagcgacgtggtggagaccgagggcagccatagcaactcgcccaccaacatgccccccgcgcgcctggaggaggccgtgtggcggccctactgagctgagcgccatcgccatcgagggactgggcctgccgtccatgcacagaccccgccaggagggcccttggaggccaccaggaagaatcccggagggaaactgtgaatgcttctgatttagcaatgctgtgaataaaagaaagattttatacccttgacttcactttttaaccacgttgtttattccaaagagtgtggaatgttttcggttcggggtggggaagacgcagcccatcctgtttggcatctatttcttatttcggagttttcttttccgcaccttatcgattgcaaaaatgcctgtttgcatctgggtggtcatttatttttaagtgtgtatagatttgagcttgcttttttttcttcctttgaccaactcaaagaaataaaattcccttctctgtaaggtttatttaacttttagactttcatgtagctgggggttttatttgtgtttggtttttgtttttatttttaaagagacagctacagctttgggtcattttttaactactgtatttccacaaagaaatccctagatatttatgtatcttgatgtttgaacatttacatatgtgttgatacttttttaattatttaaatgtacttatattaagaaagatatcaagtactacatttttctttataatagccaaagttaaatattattgcgttgaagatgtctggaaaaaaaagagatcgcttggttaactagaaatattgtttacattaaactccctttatgttattcaaacaagttggtaggtaacgcagcaatgtttttaattggattgtagacactgagggtcactccaaggtcagaagtacaaaattttctgctaggctcaacaaatagtctcatacctggctccttcccttcaaaaagagaggcaaactctgtcctgaaagggttcagagaggtgccaaggatttgctctgaagaggatttcattttggcctggagatatacttgccccaaggcctcctcattctggcatgctttatcacagagctcaaccaagtaagctgttggtcaggggtttacttacatagtatttacatagacccaaaccactgaatgtgatttttaaattgccttccattaatagtacccgttcattgatgaaaaccaaaacttgaggctgtaccccaaagatccaaatagaagagttaagaccaggtgtctttgaggcctaaaggctgagttttaagagagtgtaccccaaaagtctgaaggagccggtttccttctcccagtcttagtggaatcagtcatgggaggcagatgccacgcccacctgtgcaggatgctcctcagaagctgccccttcaccagcatcttctcccaccaggccgagcccctgacctttggggtgcatcagtgtgatagatcctggtctctgcagtccgccatggctacggttcagatgtgcatcgtgtcactgtaaatgtaatggtactgttgttacagtggaggacttggtcaaaatccagttgttctacaacgtatgaagcctaaccgctggttctgacatacatgtgctcaaaatgatctggttgtttggatttttcttttgttgttttgttttttaatgtacctcttaaattagttgaagtgatgtcaggtcaactccgaagagcgtttgaaagcaggacttcagcacagtgtttgatttttttattattattaatattattttataaatttaagcattcagattagatctttggctgcaggcagcaaaaacggctggacttatttaaaaaaaatacagcttgttttttgagttatctatatctatatctatatgttgattctttgtcttacatagagcagcagcactttggtaacctgtgataccaggttgctcttgtctggagaagagcgctagcaggattcagagaaactcagaatagatcttcatatcagccataccttcctcctccatccggtctccactcagttattccacagaacactttgacagctgtgttgtcagaaaaataaaaaaaaatttaatttctcaaaaggagtttgtttctccaacattagatgttcctcttaccataggctgccgtatctggcctgagaaaacggtagggaaggacgaaggaaagagatttctattttttcatattaattttgatatctaaagatacgctagccctcagaggagcagataatctcacacattgaattttcgccctgggcaccatgcatcaagaaggcttgtcactgtgttagagccatttagtgcttcctaaacttttatcaacataggcagtatttagtctcagagaaaaaaaaatccatcaggcacatgtagtcttggagatagattccacggggcaggtatttctctacctgagaaattgtgttcattgccttcgggtgcttccagcggtctcctcattcgctgtcttcaaggaagacccataagccaattctgagataatggagctgttgggaatactggtccagagaaagaaaaatgggataagccattcttactgcttattcaagcccctatttataattttaacacactttccattccttctggttttctcgccgtctatatcctcccaatagcccttctcacttttcttttccctcctgcaaacacacacacacacacacacacacacacacataaggcacacacacacacatcctctcccccataccaagtgtccagaacacagaaagtccagttcttctccgtttattaaagaacagggtgagtcagccattctcttgctcacgggtttttttccccaacagaacagaggcgttgccagccattttgggtctgctttctgtccagatactgcagcaaaaactcttgaggatcacaacccgttggctgagcagctgtgctgctgcccaaacgtcctgcgcagacaaacgcacgctgggaccggaaggggtgtctctccttctgcctcttttctttcatacgtttctctcgaaaggcctcaactgaggactgcaaatttctttcttgaaataactttcccccagggacattcggtcttagggattttttggttttgatgggttttgttttgttttggtttttttggttcttctcattttctttgtaggagaaggcatgagatgttgagggtctttcatacatgaaaataaatagtttgacagcaatctcagaatatattttttccttatttgaacaaagtactgttttgtttactctacagtacacctttatttggtgggtttggctgttggtcggaaatgccttccctctttcagccaggtcggtatagccaaagctgatcatttgtctgttttttcttttttttcctcagaagagttgtatccacaaactcaattgtatttatgtatgtaaatagatttcatgcttcattataaaatattgttaatgcctgtaataacttttttcacattttgtgtgtgtttctaaggactttttcttatgttcgctaaatattgtagaagaaaaatgcttctcttaacttgtttattttagattttaaaaaaaccaagctacttcttactcacttttataaacataataaacaagcatggttccaatgggttttttttaagttcaccttatgttctaggagaaatgaatgtgcaaaaaaaaaaatcaatcttcaaatgaactgttgggtatttctgttactctggatggaaaaagatcaatggaaaacaaaaaacaaaaaaacaaacttccaaattgaaatagcagtaaaacacatgtattgggggtaaaaaaaaaaaaaaaaaacacacctcagaaaatgcagttctccagcctccagctactgcccacacatgtggcaagtgttagatgtggtcgtgaggaatcccaaaatcagtgcccgggccttttccttcctggtactaacattaagaacacctcctaaggggcactgtcaggctcaggtcttaaagcacatagataagagagaatgtcccagaacgattctcagtagcccaggccagcaggtactcacggcactgcacctgctcactgcacacagtcgctgaggcagacccctctcctgggggccatgcagagccagggcagggcagccctaagctactgatgttttctttcctttgtactatggtcttttctgtaactccaatattcaaacccatgtgaatggcaaataaacaatttgacaagcacctaaaaaaaaaaaaaaaaaa

SEQ ID NO: 43 - DNA, 2475 bp, Homo sapiens
  Human GFI-1B (NM_004188.6)
ctttattgcgaggctgagtatgatgggctccatccagcacgaacacaaagccctgtgagaggaggcagagtgagatgaagtcgaactgtgggatatgaaaggcattttgaaggagtaggcatcaggctggtttttgttcgaggaaagctactcaggagcttgggaggattgcttgagaccaggagttcaagaccagcctgggctacagagcaagaccccatctttttgaaacttcctgcaactcgcatctggaaaagtgctgttatttgaaagggtgccgacattgtgaaaaacacggagtattgatctctgaagctgagatttttgtcctaaagaatactcaagatgtgtccctggctgggcacagcagctcgtgcctgtaatcccagcactttgggaggctgaggcaggaggatcgcttgaggccaggagttcaagaccagcctattgtgaatagtaccactataaatagagaaagcgtgccgctccaagtgtcgagggttagaaatgagaattcgaagtcttgtgtcctggaaagttttgataagcaaatacggctgagctcccgcgctctcttcattggctgcttgttcaccgccagattttgacacaaataatcagattgaaaatcagggaggggaacagaagaggaaaaacacacagagagacagagcaaaaaggagaagtatctatttgtgcaaagagtcacacagttgacagagtggaggccagtcccgagagaggctttgcagttcccacctcgggaagctccggcagaacccaggcgagggacagctccggacaggtgtggggtgcacactgaaaatgccacgctccttcctggtgaagagcaagaaggctcacacctaccaccagccccgtgtgcaggaagatgaaccgctctggcctcctgcccttaccccggtgcccagagaccaggctccaagcaacagccctgtccttagcactctattcccaaaccagtgcctggactggaccaacctcaaacgagagccggagctggagcaggaccagaacttggccaggatggccccggcaccagagggccccattgtgctgtcccgaccccaggatggggactctccactgtccgactcacccccattctacaagcctagcttctcctgggacaccttggccacaacctatggccacagctaccggcaggccccctccaccatgcagtcagccttcctggagcactccgtcagcctgtacggcagtcctcttgtgcccagcactgagcccgccttggacttcagcctccgctactccccaggcatggatgcgtaccactgtgtgaagtgcaacaaggtcttctccacccctcacgggctcgaagtgcatgtgcgacgctcccatagtgggacccggcccttcgcctgtgacatctgcggcaaaaccttcggccacgctgtgagcctggagcagcacacgcacgtccactcccaggagcgcagcttcgagtgccgcatgtgcggcaaggccttcaagcgctcgtccacgctgtccacccacctgctcatccactcagacacgcggccctacccctgccagttctgcggcaagcgtttccaccagaagtccgacatgaagaagcacacctacatccacacaggtgagaagccgcacaagtgccaggtgtgcggaaaggccttcagccagagctccaacctcatcacccacagccgcaagcacacaggcttcaagcccttcagctgtgagctgtgcaccaaaggcttccagcgcaaggtggacctgcggcggcaccgcgagagccagcacaatctcaagtgaggctgcgccggctcccagctcctggccagcctgccctgcggtcctgtcacctggaggccagcctcacatgcccaaatctccagtctcctggaggtgggactggacaggagtctaccagcttgttttgagactcatgaaattgctgtgtgaccttgggcaagtcacttaccctgtctggatcaacatttctcctgctgccaagtgtgggagcctggctgggtctttctcagcagaagttgtttccaggtgtgctcaagtgccttcctctagcagagcacagaaagctagaatacccccagggagacagggatgccaagagtagaccagagctgggacccacagacagaacctccacctgcctgctgcccactgagctgggacctggtcaccttggattttagccggcctctttctggctataacaggcagagtcggagctgcctcccaccccagtcagaagcctggcaccccctctgcttcggccagatgtgctggctgactccgacttccgaccagcactcagctggcctctggggattctagctccacaaccaggccgtgaggctggagaaactggcagttattgctgtcaaaagcctgttctctcaactgctgtcaataaaattaaagatacagatttgctgccaaaaaaaaaaa

SEQ ID NO: 44 - DNA, 1724 bp, Mus <mouse, genus>
  Mouse Gfi-1b (NM_008114.3)
cacagaaacgaaaaggagaagtgtctgtctgtgcagagactcataacgttgaccgagccgagagcagtccccagggacagtgtggaggttcgtggctctcgggcagaactcagaagagggacagctccctgacggtgtggcgtgcacgcagaaaaatgccacggtcctttctagtgaagagtaagaaggcacacacttaccaccagccccgggcacagggtgatgagctggtctggcctcctgctgtaattcctgtggcaaaagagcatagccagagtgccagccctcttctcagcacaccgcttccaagccagaccttggactggaacacaatcaaacaggagcgggagatgttgctgaaccagagccttcccaagatggcctcagccccagaggggcctctcgtgacaccccaaccccaggatggggaatcaccactctctgagtcaccccctttctacaagcccagcttctcctgggataccttggcctcctcctacagccacagctacacacagaccccctccaccatgcagtccgccttcctggagcgctccgtgaggctgtacggcagccccctcgtgcccagcacagagtctcccttggacttccgcctccgctactctccaggcatggacacttaccactgtgtcaagtgcaacaaggtgttctccacccctcatgggctagaagtgcatgtccgccgctctcacagcggaacccggccctttgcctgtgatgtctgtggcaaaacctttggccacgctgtgagcttggagcagcatactcacgtccactcacaggagcgaagcttcgagtgccggatgtgtggcaaagccttcaagcgttcatccaccctgtccacccacctgctcatccactcggacactcggccctacccctgccagttctgtgggaagcgcttccaccagaagtcggacatgaagaaacacacctacatccacacaggtgagaagccccacaagtgccaggtgtgtgggaaagccttcagccagagctccaacctcatcacccacagccgcaagcacacaggcttcaagccgttcagctgtgagctgtgcaccaagggcttccagcgcaaggtggacctgcgacgtcaccgtgagagtcaacacaatctcaagtgagacggttggccgcctgctttagtgtgtctcgcctgaaggccagcctctcctttccaatcctgatcccagtcctcctggaagcagcattgcccatgagcctctctgcttcttttgagactggatgacctcaaccaagccacactcctcctctgaccacagctgatgtgggagtcagttcgggcctttctgaactgaggcagtcacagacatgctctggtctcattcaatgccagagcacagacagctacaaagccctcgtggacatggcaaaaccaggcaagagccaggatccacagagaaaccctcttgcttgcttctctgggtctagtgactgaatttttagggattctctttttggctgccacagtcagagttgtcccctggcctagaggtctggcgcccctctgcttcggccagatgtgctctctgtcccccacctctcaccacatccatccgcccactgggagtcaggctcctgaggtgagccacgaggctatgaaatcagccatgatagtagaagcctgctcctatcagttgatgtaaatgtaaataaaggtgggtttatttacatgtgaa

SEQ ID NO: 45 - DNA, 2076 bp, Homo sapiens
  Human HOX-A9 (NM_152739.3)
agttgttacatgaaatctgcagtttcataatttccgtgggtcgggccgggcgggccaggcgctgggcacggtgatggccaccactggggccctgggcaactactacgtggactcgttcctgctgggcgccgacgccgcggatgagctgagcgttggccgctatgcgccggggaccctgggccagcctccccggcaggcggcgacgctggccgagcaccccgacttcagcccgtgcagcttccagtccaaggcgacggtgtttggcgcctcgtggaacccagtgcacgcggcgggcgccaacgctgtacccgctgcggtgtaccaccaccatcaccaccacccctacgtgcacccccaggcgcccgtggcggcggcggcgccggacggcaggtacatgcgctcctggctggagcccacgcccggtgcgctctccttcgcgggcttgccctccagccggccttatggcattaaacctgaaccgctgtcggccagaaggggtgactgtcccacgcttgacactcacactttgtccctgactgactatgcttgtggttctcctccagttgatagagaaaaacaacccagcgaaggcgccttctctgaaaacaatgctgagaatgagagcggcggagacaagccccccatcgatcccaataacccagcagccaactggcttcatgcgcgctccactcggaaaaagcggtgcccctatacaaaacaccagaccctggaactggagaaagagtttctgttcaacatgtacctcaccagggaccgcaggtacgaggtggctcgactgctcaacctcaccgagaggcaggtcaagatctggttccagaaccgcaggatgaaaatgaagaaaatcaacaaagaccgagcaaaagacgagtgatgccatttgggcttatttagaaaaaagggtaagctagagagaaaaagaaagaactgtccgtcccccttccgccttctcccttctctcacccccaccctagcctccaccatccccgcacaaagcggctctaaacctcaggccacatcttttccaaggcaaaccctgttcaggctggctcgtaggcctgccgctttgatggaggaggtattgtaagctttccattttctataagaaaaaggaaaagttgaggggggggcattagtgctgatagctgtgtgtgttagcttgtatatatatttttaaaaatctacctgttcctgacttaaaacaaaaggaaagaaactacctttttataatgcacaactgttgatggtaggctgtatagtttttagtctgtgtagttaatttaatttgcagtttgtgcggcagattgctctgccaagatacttgaacactgtgttttattgtggtaattatgttttgtgattcaaacttctgtgtactgggtgatgcacccattgtgattgtggaagatagaattcaatttgaactcaggttgtttatgaggggaaaaaaacagttgcatagagtatagctctgtagtggaatatgtcttctgtataactaggctgttaacctatgattgtaaagtagctgtaagaatttcccagtgaaataaaaaaaaattttaagtgttctcggggatgcatagattcatcattttctccaccttaaaaatgcgggcatttaagtctgtccattatctatatagtcctgtcttgtctattgtatatataatctatatgattaaagaaaatatgcataatcagacaagcttgaatattgtttttgcaccagacgaacagtgaggaaattcggagctatacatatgtgcagaaggttactacctagggtttatgcttaattttaattggaggaaatgaatgctgattgtaacggagttaattttattgataataaattatacactatgaaaccgccattgggctactgtagatttgtatccttgatgaatctggggtttccatcagactgaacttacactgtatattttgcaatagttacctcaaggcctactgaccaaattgttgtgttgagatgatatttaactttttgccaaataaaatatattgattcttttctaaaaaaaaaaaaaaaaaaaa

SEQ ID NO: 46 - DNA, 3229 bp, Mus <mouse, genus>
  Mouse HOX-A9 (NM_010456.3)
gaaaaaacagaagagggaaggataccagagcggttcatacagggcccagaaactaggcgaggtgacccctcagcaagacaaacacctcttgatgttgactggcgattttccccatctccagtctggggagcgggactaggcatacagatgatggagcttagaacccgctggctagggaataaaattcgctgggcagtttgtgctcaaagaagtgggccagggcgcttgtgacacaatcagggcgtttgtgacacaaacccttgagggttggcagttctctccttggcggttgctctggttgctctgtggggccttccctgtggagcaagggtgatctggccgatgtgcaagcgcctggctggctttccagtctgactagggtcggtagcccattttaggtggttgtatcatcgacggtgcgtcgcgacaggggcggtggtcactctgtttgaggtggagagagccttgtatttgacttttctaggccggccctgggggcgcgcgcgggcggggggctcacatctctgaggactgcaaggattatttacagggtattcaccaaccaaacacaacagtctaatttaacctttccaagtcctcataaatttttacagggagccacagcgaggcaaacgaatctgttggtcgctcctgactttccaccagcctgtgtggcttccgaaacaataactccttatgaaatatcataaatatagatttaaatacagtagagtgagaatgcgatttggctgcttttttatggcttcaattattgtctaattttatgtgaggggctctgctggccgtgctcacacgcgggacccgcgccttcctgatggcgtgattaattgtgatataaaatagtccgcttaagaagtgtgtgtgtctggtatgtgtgtgtgttgggggggtggcaagggagagtacagaggcaaggccagatttgatcttttaatcttcgttggccacaattaaaacaaaccagatcgtggagctgcgcgatccctttgcataaaaacatatggcttttgctataaaaattatgactgcaaaacaccgggccattaatagcgtgcggagtgatttacgcgttattgttctgccgggcggacacgtgacgcgcgtggccaatgggggcgcgggcgccggcaacttattaggtgactgtacttcacccccccctggtgccaccaagttgttacatgaaatctgcagtttcataatttcggcgggtcgggctgggccggccaggcgcgggctactgcaatggccaccaccggggccctgggcaactactatgtggactccttcctgctgggcgccgacgctgctgatgagctgggtgcgggacgctacgctccagggaccctgggtcaacccccaaggcaggcggcagctctggccgaacaccccgacttcagtccttgcagcttccagtccaaggcggcggtgtttggtgcctcgtggaacccagtgcacgcggcgggcgccaatgcggtgcctgctgcagtgtatcatcaccaccaccacccctacgtgcatccccaggcgcccgtggcggcggcggcgccggacggcaggtatatgcgctcctggctggaacccacgcccggtgcgctctccttcgcgggcttaccctccagccggccttatggcattaaacctgaaccgctctcggccagaaggggtgactgtcccacgcttgacactcacactttgtccctgactgactatgcttgtggttctcctccagttgatagagaaaaacaacccagcgaaggcgccttctccgaaaacaatgccgagaatgagagcggcggagacaagccccccatcgatcccaataacccggctgccaactggctacatgctcgctccactcggaagaagcgatgcccctacacaaaacaccagacgctggaactggagaaggagtttctgtttaacatgtacctcacacgggaccgcaggtacgaggtggcccggctgctcaacctcaccgaaaggcaggtcaagatctggttccagaaccgcaggatgaaaatgaagaaaatcaacaaggaccgagcaaaagacgagtgagccttttaggggctcatttaaaaagagagcaagctagaaagaaaaagaaaggactgtccgtctccctctgtctcctctcccccaaacccagcctccacccgcacaaaggggctctaaatcccaggcctcatctccccactggcagtccgtgctcaggctggctcttaggcctgcggctttgatggaggaggtattgtaagctttccattttatagaaggcacacacacacacaagggagggcattagcgctattggctgtatgtgctagcttgtatatatatatatatatttaaaaaaaatctacctgcttctgactttaagcaaaaggaaagaaaactacctttttatataatgcacaactgttgatgactggctgtatagtttttagtctctgtagctaatttaatttgctcttcgtgtggcagatcattctgccaaaatacttgaacactgtgttttattgtggtaattatgttttgtgactcaaacttctgtgctgggtgaagtacccattgtgattgtggaagctagaattcaatttgaactcaggttgtttatggggggagagaagctgtggcataatgtatagctctgtagtcttctgtgtagctagactgttaacctacgattgtaaactagctgtaaggatttcccagtgaaatcagatttggaaagaaaagagagatagttctccgggatgcatagattcatgatttatctacttttgaaatgtgggcttcttcatctttacgttctagactccaattttgtccaatgtatatagaatctccatattaaagaaatattcataatcagaaagcttgaatattgtttttgcaccagaggagaagtgaggaaattcggagctatacgtgtgtgcagagggttgctacctatgggtttacgcttaattttaattgggagaaagtgagtgcttattgtaatggagttaattttattgataataaattatacaccatgaaactgctcttgggctactgtagatttgtatccttggtgaatttggggttcccatcggattgaacatacactgtatattttgcaatagttacctcaaggcctactgaccaaattgttgtgtcgagatatttaacttttgccaaataaaatatattgattctttta

SEQ ID NO: 47 - DNA, 3484 bp, Homo sapiens
  Human GATA2 (NM_001145661.1)
actgggtcaagcacagccctgagcggccgcgtgtccgaggcccaggtgccctctagagccctgtagttcctgcccctctctgcccctctcggctcctgctgttccgccgctgtcgtccgaaccatcccaacccccagtccacccagacagcgcccgagctaggggagggaacggtctgggagtcggcagctggcgccagggcggccggaggatgccgaggggccggagccgggagggcccgaggccgaggcgcactctacccccagctcctaccctgtaagccccgccagcctccggacgtgctgtccctgggcccgtcgccctcggggctcccgccggaactccttcactctcagaggccgagtccctcccctccccacggctgcgtgtggccgttgccgtctgcacccagaccctgagccgccgccgccggccatggaggtggcgcccgagcagccgcgctggatggcgcacccggccgtgctgaatgcgcagcaccccgactcacaccacccgggcctggcgcacaactacatggaacccgcgcagctgctgcctccagacgaggtggacgtcttcttcaatcacctcgactcgcagggcaacccctactatgccaaccccgctcacgcgcgggcgcgcgtctcctacagccccgcgcacgcccgcctgaccggaggccagatgtgccgcccacacttgttgcacagcccgggtttgccctggctggacgggggcaaagcagccctctctgccgctgcggcccaccaccacaacccctggaccgtgagccccttctccaagacgccactgcacccctcagctgctggaggccctggaggcccactctctgtgtacccaggggctgggggtgggagcgggggaggcagcgggagctcagtggcctccctcacccctacagcagcccactctggctcccaccttttcggcttcccacccacgccacccaaagaagtgtctcctgaccctagcaccacgggggctgcgtctccagcctcatcttccgcggggggtagtgcagcccgaggagaggacaaggacggcgtcaagtaccaggtgtcactgacggagagcatgaagatggaaagtggcagtcccctgcgcccaggcctagctactatgggcacccagcctgctacacaccaccccatccccacctacccctcctatgtgccggcggctgcccacgactacagcagcggactcttccaccccggaggcttcctggggggaccggcctccagcttcacccctaagcagcgcagcaaggctcgttcctgttcagaaggccgggagtgtgtcaactgtggggccacagccacccctctctggcggcgggacggcaccggccactacctgtgcaatgcctgtggcctctaccacaagatgaatgggcagaaccgaccactcatcaagcccaagcgaagactgtcggccgccagaagagccggcacctgttgtgcaaattgtcagacgacaaccaccaccttatggcgccgaaacgccaacggggaccctgtctgcaacgcctgtggcctctactacaagctgcacaatgttaacaggccactgaccatgaagaaggaagggatccagactcggaaccggaagatgtccaacaagtccaagaagagcaagaaaggggcggagtgcttcgaggagctgtcaaagtgcatgcaggagaagtcatcccccttcagtgcagctgccctggctggacacatggcacctgtgggccacctcccgcccttcagccactccggacacatcctgcccactccgacgcccatccacccctcctccagcctctccttcggccacccccacccgtccagcatggtgaccgccatgggctagggaacagatggacgtcgaggaccgggcactcccgggatgggtggaccaaacccttagcagcccagcatttcccgaaggccgacaccactcctgccagcccggctcggcccagcaccccctctcctggagggcgcccagcagcctgccagcagttactgtgaatgttccccaccgctgagaggctgcctccgcacctgaccgctgcccaggtggggtttcctgcatggacagttgtttggagaacaacaaggacaactttatgtagagaaaaggaggggacgggacagacgaaggcaaccatttttagaaggaaaaaggattaggcaaaaataatttattttgctcttgtttctaacaaggacttggagacttggtggtctgagctgtcccaagtcctccggttcttcctcgggattggcgggtccacttgccagggctctgggggcagatttgtggggacctcagcctgcaccctcttctcctctggcttccctctctgaaatagccgaactccaggctgggctgagccaaagccagagtggccacggcccagggagggtgagctggtgcctgctttgacgggccaggccctggagggcagagacaatcacgggcggtcctgcacagattcccaggccagggctgggtcacaggaaggaaacaacattttcttgaaaggggaaacgtctcccagatcgctcccttggctttgaggccgaagctgctgtgactgtgtccccttactgagcgcaagccacagcctgtcttgtcaggtggaccctgtaaatacatcctttttctgctaacccttcaaccccctcgcctcctactctgagacaaaagaaaaaatattaaaaaaatgcataggcttaactcgctgatgagttaattgttttatttttaaactctttttgggtccagttgattgtacgtagccacaggagccctgctatgaaaggaataaaacctacacacaaggttggagctttgcaattctttttggaaaagagctgggatcccacagccctagtatgaaagctgggggtggggaggggcctttgctgcccttggtttctgggggctggttggcatttgctggcctggcagggggtgaaggcaggagttgggggcaggtcaggaccaggacccagggagaggctgtgtccctgctggggtctcaggtccagctttactgtggctgtctggatccttcccaaggtacagctgtatataaacgtgtcccgagcttagattctgtatgcggtgacggcggggtgtggtggcctgtgaggggcccctggcccaggaggaggattgtgctgatgtagtgaccaagtgcaatatgggcgggcagtcgctgcagggagcaccacggccagaagtaacttattttgtactagtgtccgcataagaaaaagaatcggcagtattttctgtttttatgttttatttggcttgttttattttggattagtgaactaagttattgttaattatgtacaacatttatatattgtctgtaaaaaatgtatgctatcctcttattcctttaaagtgagtactgttaagaataataaaatactttttgtgaatgcccaaaaaaaaa

SEQ ID NO: 48 - DNA, 3258 bp, Mus <mouse, genus>
  Mouse Gata2 (NM_008090.5)
gtctgtgcaggagtcggcagctggcgccagggcggccggaggatgcagaggggccggagccgggcgggccggaggccgagacgcgcgctgtcccccacccctatcccgtgaatccgccggccctggaacgcgctgtcgctgggcccgccgtacccgggctctcctggtgtctcttactctctactgctgagccctccccttcccgcgccgctgcgagtggccgccccaccttcgcctggttcccaagacacagtagtggaccatggaggtggcgcctgagcagcctcgctggatggcgcaccccgccgtattgaatgcgcagcaccccgactcgcaccatccgggcctggcgcataactacatggagccagcacagctgctgcctcccgacgaggtggatgtcttcttcaaccatctcgactcgcagggcaacccttactacgccaacccggcccacgcgcgcgcgcgcgtttcctacagcccggcgcatgcccgtctcaccggaggccagatgtgccgaccacacttgttgcacagcccaggcttgccgtggctggacgggggcaaagcagctctctctgccgccgctgcccatcaccacagtccctggaccgtcagcccgttctccaagaccccgctgcacccctcagctgctggagcacccggagggcctctgtctgtttacccaggggctgcgggtgggagcgggggaggcagtgggagctccgtggcctccctcacccccactgcagcccactcgggctcccatctcttcggcttcccacccacgccacccaaagaagtgtctccagaccccagcacaacaggagctgcttccccggcctcttcttctgcagggggtagtgtagcccggggtgaggacaaggatggcgtcaagtaccaagtgtcactctccgagagcatgaagatggaaggcggcagtcccctgcgcccgggcctagctaccatgggcacccagcctgcaacacaccacccgatacccacctatccctcctatgtgcccgccgcagctcatgactatggcagcagtctcttccatccaggaggcttcctgggtggccccgcctccagcttcacccctaagcagagaagcaaggctcgctcctgctcagaaggccgggagtgtgtcaactgtggtgccacagccacccctctctggcgacgagatggcacgggccactacctgtgcaatgcctgtgggctctaccacaagatgaatggacagaaccggccgctcatcaagcccaagcggaggctgtctgctgccagaagagcgggcacctgttgtgcaaattgtcagacgacaaccaccaccttatggcgccggaacgccaacggggaccctgtgtgcaacgcctgtggcctctactacaagctgcacaatgttaacaggccactgaccatgaagaaggaagggatccagacccggaatcggaagatgtccagcaaatccaagaagagcaagaaaggggctgaatgtttcgaggagctctccaagtgcatgcaagagaagtcaccgcccttcagtgcggctgccctggctggacacatggcacctgtgggacacctcccaccttttagtcactctggacacatcctacccacgcccacgcctatccacccttcctccagtctctcttttggccacccccacccgtccagcatggtgactgccatgggctaggcaagcctcccactggacagacatggacatcaagggtggtttggcagaaccagagcgaggctgggcactcccaggatgggtggaacatactcttggctcccgcccatcccaagagacccacttcctcctgccagcctagcctggccgaagccacctctccttggaggactcccagccttgtgccgccattactgtgaatatttctaactgggctgcagctcgcgtgtgcccggggtgctgcccagaaaagtgttttcacggagagtgtttgtttggagagcaaaatggacaggtttacagatttatagcaagaagagactggggatagaaaaatgaaacctttttttttctttttctttttttcttcttctgttttatttttttgatggagaaaggagtaggcaagaagaaaaataatttattttgctcttatttcttacaagaacgtgaagacatggaggcgtgtgctatttgtgttcttggggtccttctttgggacctcctgccaccagtcagggctctcgggggcagacttagaggtcctcagcctgagcctccttcaccccagcctgcctgcagggtagcccctgccctgacgcagccctagagggcagagacaattgcaggcggtcctgcgcagattcccaggccagggctgggtcacaggaaggaaacattctctggaaaggggaaacgtctcccagatcattcccctggcttccagaggccaaagctggtgtgacccaaatgggccagagctgcagcctgtgctctaggccagtcggacccctgtaaatacaaccttcttttctgctaaaccctcggccccctccccctctaagataaataagaaaatactcaaagcgaaaaccaaactgcataagcttaacccgctgatgagtggttttattttgaaactcgttttttgggtccagtcaattgtacgttgccacagaagccccgctatggaaaaaaataaataaaacctacaaaccaggcctgagcttcacagtcctttgagtggttcttgggtcccacagccctggcagggggctcgggacaagggggaatcttatgctcttggtttctgggagacagggggcaggcaggcagtggccctgtgatcccaggcttctgttctgctgtggctggctgaatccttcaaggtacagttgtacataaaaagtgtcccaagcttcgattctgtgtgtggtggtggcagtggtgcagcagccagcaagggggccccgagtgagcccagggagacgattgtgctgagtcaaccaagtgcaatatcggtgtccagttgctgcagagcaccctaaccggaagtaacttattttgtgctagtacccgcataagagaagaatcggcagtattttctgtttttatgttttgggcttgttttattttgaattagtgacctaagttattgttaactgtgtacaacatttaaatattgtctgtaaaaattgtatgctaccctcttattcctttaaagtgaatactgttaaaaataataaaatactttttgtgaaaaaaaaaaaaaaaaa

SEQ ID NO: 49 - DNA, 3198 bp, Homo sapiens
  Human MEIS1 (NM_002398.2)
atttgaggtgttctgaccagaagaagacagagcggatgatcattcattcaccacgttgacaacctcgcctgtgattgacagctggagtggcagaaagccatgagatttggtagttgggtctgaggggcgctcttttttttccttttctttctttctttctttttttttttttaaactgatttttgggggagagaagatctgcttttttttgcccccgctgctgtcttggaaacggagcgcttttatgctcagtgactcgggcgctttgcttcaggtcccgtagaccgaagatctgggaccagtagctcacgttgctggagacgttaagggatttttcgtcgtgcttttttttttttttttttttttttccgggggagtttgaatatttgtttcttttcacactggccttaaagaggatatattagaagttgaagtaggaagggagccagagaggccgatggcgcaaaggtacgacgatctaccccattacgggggcatggatggagtaggcatcccctccacgatgtatggggacccgcatgcagccaggtccatgcagccggtccaccacctgaaccacgggcctcctctgcactcgcatcagtacccgcacacagctcataccaacgccatggcccccagcatgggctcctctgtcaatgacgctttaaagagagataaagatgccatttatggacaccccctcttccctctcttagcactgatttttgagaaatgtgaattagctacttgtaccccccgcgagccgggggtggcgggcggggacgtctgctcgtcagagtcattcaatgaagatatagccgtgttcgccaaacagattcgcgcagaaaaacctctattttcttctaatccagaactggataacttgatgattcaagccatacaagtattaaggtttcatctattggaattagagaaggtacacgaattatgtgacaatttctgccaccggtatattagctgtttgaaagggaaaatgcctatcgatttggtgatagacgatagagaaggaggatcaaaatcagacagtgaagatataacaagatcagcaaatctaactgaccagccctcttggaacagagatcatgatgacacggcatctactcgttcaggaggaaccccaggcccttccagcggtggccacacgtcacacagtggggacaacagcagtgagcaaggtgatggcttggacaacagtgtagcttcccccagcacaggtgacgatgatgaccctgataaggacaaaaagcgtcacaaaaagcgtggcatctttcccaaagtagccacaaatatcatgagggcgtggctgttccagcatctaacacacccttacccttctgaagaacagaaaaagcagttggcacaagacacgggactcaccatccttcaagtgaacaattggtttattaatgcccggagaagaatagtgcagcccatgatagaccagtccaaccgagcagtaagtcaaggaacaccttataatcctgatggacagcccatgggaggtttcgtaatggacggtcagcaacatatgggaattagagcaccaggacctatgagtggaatgggcatgaatatgggcatggaggggcagtggcactacatgtaaccttcatctagttaaccaatcgcaaagcaagggggaaggctgcaaagtatgccaggggagtatgtagcccggggtggtccaatgggtgtgagtatgggacagccaagttatacccaaccccagatgcccccccatcctgctcagctgcgtcatgggccccccatgcatacgtacattcctggacaccctcaccacccaacagtgatgatgcatggaggaccgccccaccctggaatgccaatgtcagcatcaagccccacagttcttaatacaggagacccaacaatgagtggacaagtcatggacattcatgctcagtagcttaagggaatatgcattgtctgcaatggtgactgatttcaaatcatgttttttctgcaatgactgtggagttccattcttggcatctactctggaccaaggagcatccctaattcttcatagggacctttaaaaagcaggaaataccaactgaagtcaatttgggggacatgctaaataactatataagacattaagagaacaaagagtgaaatattgtaaatgctattatactgttatccatattacgttgtttcttatagattttttaaaaaaaatgtgaaatttttccacactatgtgtgttgtttccatagctcttcacttcctccagaagcctccttacattaaaaagccttacagttatcctgcaagggacaggaaggtctgatttgcaggatttttagagcattaaaataactatcaggcagaagaatctttcttctcgcctaggatttcagccatgcgcgcgctctctctctttctctctcttttcctctctctccctctttctagcctggggcttgaatttgcatgtctaattcatttactcaccatatttgaattggcctgaacagatgtaaatcgggaaggatgggaaaaactgcagtcatcaacaatgattaatcagctgttgcaggcagtgtcttaaggagactggtaggaggaggcatggaaaccaaaaggccgtgtgtttagaagcctaattgtcacatcaagcatcattgtccccatgcaacaaccaccaccttatacatcacttcctgttttaagcagctctaaaacatagactgaagatttatttttaatatgttgactttatttctgagcaaagcatcggtcatgtgtgtattttttcatagtcccaccttggagcatttatgtagacattgtaaataaattttgtgcaaaaaggactggaaaaatgaactgtattattgcaatttttttttgtaaaagtagcagtttggtatgagttggcatgcatacaagatttactaagtgggataagctaattatactttttgttgtggataaacaaatgcttgttgatagcctttttctatcaagaaaccaaggagctaattattaataacaatcattgcacactgagtcttagcgtttctgatggaaacagtttggattgtataataacgccaagcccagttgtagtcgtttgagtgcagtaatgaaatctgaatctaaaataaaaacaagattatttttgtcaaaaaaaaaaaaaaaaaa

SEQ ID NO: 50 - DNA, 3346 bp, Mus <mouse, genus>
  Mouse Meis1 (NM_010789.3)
agcattctggtcggaatccacctctccgcctgtgcaacacacactttacacacgcacggcgactgcaagcgggcagcatcgatcgtggctcctttaagacaaactcagacagacatttttttaaccctcctctctaatctcccttcagtgcagcagttgcaaagagggagagagaaagagaaagagagcgagagaagagagaaactgattaggaattaggactgattcaaggaaagcgggcgctagggctttgtgcatttgaatattaacatttgaggtgttctgaccagaagaagacagaacggacgatcattcattcaccacgttgacaacctcgcctgtgattgacagctggagtggcagaaagccatgagatttggtagttgggtctgaggggcgctcttttttttttttctttttcttttcttttctttctttttttttaaactgatttttttgggggggagagaagatctgctttttttttcccctcccactgctgtcttggtggaaccagagcgcttttatgctcagcgacgcgggcgccttgcttcaggtccggtagaccgaagatctgggaccagtaattcacactgctggagacgcaaagggatttttttttgttattgttgtgctttatttttttttccgggggagtttgcatatttgtttcttttcacactggccttaaagaggatatattagaagttgaagtaggaagggagccagagaggccgatggcgcaaaggtacgacgacctaccccattatgggggtatggatggagtaggcatcccctccacgatgtatggggacccgcatgcagccaggtccatgcaaccggtccaccacctgaaccacgggcctcctctgcactcgcatcagtacccgcacacagctcacaccaacgccatggcccccagcatgggttcctcggtcaatgacgctttaaagagagataaagatgccatttatggacaccccctcttccctctcttagcactgatttttgagaaatgtgaattagctacttgtaccccccgcgagccgggggtggcgggcggggacgtctgctcgtcagagtcattcaatgaagatatagcggtgttcgccaaacagattcgcgcagaaaaacctctattctcttctaatccagaactggataacttgatgattcaagccatacaagtgttaaggtttcatctgttggaattagagaaggtacacgaattatgtgacaatttctgccaccggtatattagctgtttgaaagggaaaatgcctatcgatttggtgatagatgatagagaaggaggatcaaaatcagacagtgaagatgtaacaagatcagcaaatctaactgaccagccctcttggaatagagaccatgatgacacggcatccactcgttcaggaggaaccccgggcccttccagcggtggccatacttcacacagtggggataacagcagtgagcaaggtgatggcttggacaacagtgtagcttcccccagcacaggtgacgatgatgaccctgataaggacaaaaagcgtcacaaaaagcgtggcatctttcccaaagtagccaccaatatcatgagggcgtggctgttccagcatctaacacacccttacccttctgaagaacagaaaaagcagttggcacaagatacaggacttaccatccttcaagtgaacaattggtttattaatgcccggagaagaatagtgcagcccatgatagaccagtccaaccgagcagtcagccaagggacaccttataaccctgatggacagccaatgggaggttttgtaatggacggtcagcagcacatgggcatcagagcgccagggctgcaaagtatgccaggggagtatgtagcccggggtggcccaatgggtgtgagtatgggacagccgagttatacccaagcccagatgcccccccatcctgctcagctgcgtcatgggccccccatgcatacgtacattcctggacaccctcaccaccccgcagtgatgatgcatggaggacagccccaccctggaatgccaatgtcagcctcaagcccctcggttcttaacacaggagacccgacaatgagtgcacaagtcatggacattcacgctcagtagcttaagggaatatgcgttgtctacaatggtgactgatctcgaatcaggtcttttcctgcaaggactatggagttccattcttgacatctactttggaccaaggagcatccctagttcttcatagggactcttaaaatgcaggagaaccatccgaagtcaactcgggggacatgcaaaaataactatataagacattaaaagaacaaagagtgaaatattgtaaatgctattatactgttatccatattacgttgtttcttatagattttttaaaaaaaatgtgaaatttttccacactatgtgtgttgtttccatagctgttcacttcctccagaagcctccttacattaaaaagccttacagttatcctgcaagggacaggaaggtctgatttgcaggatttttagagcattaaaataactatcaggcagaagaatctttcttcttgcctaggatttcagccatgtgcgtgcgctctctctctctctctctctctctctctctctctctctctctctctctctctctctcttctcctccctctccctctttctagcctggggcttgaatttgcatgtctaattcatttactcaccatatttgaattggcctgaacagatgtaaatcgggaaggatgggaaaaactgcagtcaccaacaatgattaatcagctgttgcaggcagtgtcttaaggagactggtaggaggaggcatggaaacccaaaggccgtgtgtgtttagaagcctaactgtcacatcaagcatcatcgtccccatgcaacaacaaccatcaccttatacatcacttcctgttttatgcagctcaaaaaacatagactgaagatttattttttaatatgttgactttgtttctcagcaaagcattggtcatgtgtgtatttttccatagtcccaccttggagcatttatgtagacattgtaaataaattttgtgcaaaaaggactggaaagatgaactgtattattgcatttattttgtttttttttttgtgaaagtagcagattagtgcaaggtggcatgcatataaggttaactgagtggggtacgctaattatactttttgttgtggataaaaaatgcttgtcaatagcctttttctatcaagaaaacaaggagctaattattaataacagtcatggcacactgtgtcctatcttagcatttaaaagtatgcaaactccaggtccag

SEQ ID NO: 51 - DNA, 4414 bp, Homo sapiens
  Human STAT5A (NM_001288718.1)
agatggccggagtaaaagaaggagggaggtgctgcggtggtgggggtgatcttggcttcactagaatccccagttcttcccctctctacagttttgtctctgaggtcacaaaacctgtggcccccaagacacacatgcgcacacacgcgcgtgcacacacacaccccacacatttattttttaatctaggggctcaaaagatgacacgcgccagagctggaaggcgtcgccaattggtccacttttccctcctccctttttgcggatgagaaaactgaggcccaggtttgggatttccagagcccgggatttcccggcaacgcccgacaaccacattcccccggctattctgacccgccccggttccgggacgctccctgggagccgccgccgagggcctgctgggactcccgggggaccccgccgtcggggcagcccccacgcccggcgccgcccgccgggaacggccgccgctgttgcgcacttgcaggggagccggcgactgagggcgaggcagggagggagcaagcggggctgggagggctgctggcgcgggctcgcgcgctgtgtatggtctatcgcaggcagctgacctttgaggaggaaatcgctgctctccgctccttcctgtagtaacagccgccgctgccgccgccgccaggaaccccggccgggagcgagagccgcggggcgcagagccggcccggctgccggacggtgcggccccaccaggtgaacggccatggcgggctggatccaggcccagcagctgcagggagacgcgctgcgccagatgcaggtgctgtacggccagcacttccccatcgaggtccggcactacttggcccagtggattgagagccagccatgggatgccattgacttggacaatccccaggacagagcccaagccacccagctcctggagggcctggtgcaggagctgcagaagaaggcggagcaccaggtgggggaagatgggtttttactgaagatcaagctggggcactacgccacgcagctccagaaaacatatgaccgctgccccctggagctggtccgctgcatccggcacattctgtacaatgaacagaggctggtccgagaagccaacaattgcagctctccggctgggatcctggttgacgccatgtcccagaagcaccttcagatcaaccagacatttgaggagctgcgactggtcacgcaggacacagagaatgagctgaagaaactgcagcagactcaggagtacttcatcatccagtaccaggagagcctgaggatccaagctcagtttgcccagctggcccagctgagcccccaggagcgtctgagccgggagacggccctccagcagaagcaggtgtctctggaggcctggttgcagcgtgaggcacagacactgcagcagtaccgcgtggagctggccgagaagcaccagaagaccctgcagctgctgcggaagcagcagaccatcatcctggatgacgagctgatccagtggaagcggcggcagcagctggccgggaacggcgggccccccgagggcagcctggacgtgctacagtcctggtgtgagaagttggccgagatcatctggcagaaccggcagcagatccgcagggctgagcacctctgccagcagctgcccatccccggcccagtggaggagatgctggccgaggtcaacgccaccatcacggacattatctcagccctggtgaccagcacattcatcattgagaagcagcctcctcaggtcctgaagacccagaccaagtttgcagccaccgtacgcctgctggtgggcgggaagctgaacgtgcacatgaatcccccccaggtgaaggccaccatcatcagtgagcagcaggccaagtctctgcttaaaaatgagaacacccgcaacgagtgcagtggtgagatcctgaacaactgctgcgtgatggagtaccaccaagccacgggcaccctcagtgcccacttcaggaacatgtcactgaagaggatcaagcgtgctgaccggcggggtgcagagtccgtgacagaggagaagttcacagtcctgtttgagtctcagttcagtgttggcagcaatgagcttgtgttccaggtgaagactctgtccctacctgtggttgtcatcgtccacggcagccaggaccacaatgccacggctactgtgctgtgggacaatgcctttgctgagccgggcagggtgccatttgccgtgcctgacaaagtgctgtggccgcagctgtgtgaggcgctcaacatgaaattcaaggccgaagtgcagagcaaccggggcctgaccaaggagaacctcgtgttcctggcgcagaaactgttcaacaacagcagcagccacctggaggactacagtggcctgtccgtgtcctggtcccagttcaacagggagaacttgccgggctggaactacaccttctggcagtggtttgacggggtgatggaggtgttgaagaagcaccacaagccccactggaatgatggggccatcctaggttttgtgaataagcaacaggcccacgacctgctcatcaacaagcccgacgggaccttcttgttgcgctttagtgactcagaaatcgggggcatcaccatcgcctggaagtttgactccccggaacgcaacctgtggaacctgaaaccattcaccacgcgggatttctccatcaggtccctggctgaccggctgggggacctgagctatctcatctatgtgtttcctgaccgccccaaggatgaggtcttctccaagtactacactcctgtgctggctaaagctgttgatggatatgtgaaaccacagatcaagcaagtggtccctgagtttgtgaatgcatctgcagatgctgggggcagcagcgccacgtacatggaccaggccccctccccagctgtgtgcccccaggctccctataacatgtacccacagaaccctgaccatgtactcgatcaggatggagaattcgacctggatgagaccatggatgtggccaggcacgtggaggaactcttacgccgaccaatggacagtcttgactcccgcctctcgccccctgccggtcttttcacctctgccagaggctccctctcatgaatgtttgaatcccacgcttctctttggaaacaatatgcaatgtgaagcggtcgtgttgtgagtttagtaaggctgtgtacactgacacctttgcaggcatgcatgtgcttgtgtgtgtgtgtgtgtgtgtgtccttgtgcatgagctacgcctgcctcccctgtgcagtcctgggatgtggctgcagcagcggtggcctcttttcagatcatggcatccaagagtgcgccgagtctgtctctgtcatggtagagaccgagcctctgtcactgcaggcactcaatgcagccagacctattcctcctgggcccctcatctgctcagcagctatttgaatgagatgattcagaaggggaggggagacaggtaacgtctgtaagctgaagtttcactccggagtgagaagctttgccctcctaagagagagagacagagagacagagagagagaaagagagagtgtgtgggtctatgtaaatgcatctgtcctcatgtgttgatgtaaccgattcatctctcagaagggaggctggggttcattttcgagtagtattttatactttagtgaacgtggactccagactctctgtgaaccctatgagagcgcgtctgggcccggccatgtccttagcacaggggggccgccggtttgagtgagggtttctgagctgctctgaattagtccttgcttggctgcttggccttgggcttcattcaagtctatgatgctgttgcccacgtttcccgggatatatattctctcccctccgttgggccccagccttctttgcttgcctctctgtttgtaaccttgtcgacaaagaggtagaaaagattgggtctaggatatggtgggtggacaggggccccgggacttggagggttggtcctcttgcctcctggaaaaaacaaaaacaaaaaactgcagtgaaagacaagctgcaaatcagccatgtgctgcgtgcctgtggaatctggagtgaggggtaaaagctgatctggtttgactccgctggaggtggggcctggagcaggccttgcgctgttgcgtaactggctgtgttctggtgaggccttgctcccaaccccacacgctcctccctctgaggctgtaggactcgcagtcaggggcagctgaccatggaagattgagagcccaaggtttaaacttctctgaagggaggtggggatgagaagaggggtttttttgtactttgtacaaagaccacacatttgtgtaaacagtgttttggaataaaatatttttttcataaaaaaaaaaaaaaaa

SEQ ID NO: 52 - DNA, 3628 bp, Mus <mouse, genus>
  Mouse Stat5a (NM_001164062.1)
taacagcctccaccgccgccgccgtcaagagccgtcaggagccgtcagaagccccggcctggagcgacagccgcaggcgctccgcagcaccaggtaaacagccatggcgggctggattcaggcccagcagcttcagggagatgccctgcgccagatgcaagtgttgtatgggcagcatttccccatcgaggtccggcactacctggcccagtggatcgagagccagccgtgggatgctattgacttggataatccccaggaccgaggtcaggccacccaactcctggagggcctggtgcaggagctgcagaagaaggcggagcaccaggtgggggaagatgggtttttgctgaagatcaagctggggcactatgccacacagctccagaacacgtatgaccgctgtcccatggagctggttcgctgtatccgtcacattctgtacaacgaacagaggctggttcgcgaagccaacaattgcagctcccctgctggtgtcctggttgacgccatgtcccagaagcaccttcagatcaaccaaaggtttgaggagctgcgcctgatcacacaggacacggagaacgagctgaagaagctgcagcagacccaagagtacttcatcatccagtaccaggagagcctgcggatccaagctcagtttgcccagctgggccagctgaacccccaggagcgcatgagcagggagacggccctccagcagaagcaagtgtccctggagacctggctgcagcgagaggcacagacactgcagcagtaccgagtggagctggctgagaagcaccagaagaccctgcagctgctgcggaagcagcagaccatcatcctggacgacgagctgatccagtggaagcggagacagcagctggccgggaacgggggtccccccgagggcagcctggacgtgctgcagtcctggtgtgagaagctggccgagatcatctggcagaaccggcagcagatccgcagggctgagcacctgtgccagcagctgcccatcccaggccccgtggaggagatgctggctgaggtcaacgccaccatcacggacatcatctcagctctggtcaccagcacgttcatcatcgagaagcagcctcctcaggtcctgaagacccagaccaagtttgcggccaccgtgcgcctgctggtggggggaaagctgaatgtgcacatgaaccccccgcaggtgaaggcgaccatcatcagcgagcagcaggccaagtccctgctcaagaatgagaacacccgcaatgagtgcagcggcgagatcctgaacaactgttgcgtcatggagtaccaccaggccactggcacgctcagcgcccacttcagaaacatgtcactgaaaagaatcaagcgcgccgacaggcgtggtgcagagtcggtgacggaggagaagttcacagtcctgtttgagtctcagttcagcgttggcagcaacgagctggtgttccaggtgaagaccctgtccctccctgtggtcgttatcgtccatggcagccaggaccacaatgctactgccaccgtgctgtgggacaatgcctttgctgagccgggcagggtgccatttgctgtgcctgacaaggtgctgtggccgcagctgtgtgaagcgctcaacatgaaattcaaggctgaagtacagagcaaccggggcttgaccaaagagaacctcgtgttcctggcacagaaactgttcaacatcagcagcaaccacctcgaggactacaacagcatgtctgtgtcctggtcccagttcaaccgggagaacttgcccggctggaactacaccttctggcagtggttcgacggggtgatggaggtgctgaagaagcaccataagccccattggaatgatggggctatcctgggtttcgtgaacaagcaacaggcccacgacctgctcatcaacaagccggacgggaccttcctgctgcgcttcagtgactcggaaatcgggggcatcaccattgcttggaagtttgactctccggaccgaaacctctggaatctgaagccattcacgacgcgagatttctccattcggtccctggccgaccggctgggggacctgaactaccttatctacgtgttcccagaccgacccaaggacgaggtctttgccaagtattacactcctgtacttggttcgtcaatgcatccacagatgccggagccagcgccacctacatggaccaggctccttccccagtcgtgtgccctcaacctcactacaacatgtacccacccaaccctgaccctgtccttgaccaagatggcgagtttgacctggatgagagcatggatgttgccaggcacgtggaagaacttttacgccggcccatggacagtctcgacgcccgcctctccccacctgctggtctcttcacctccgctagaagctccctgtcctgaacgctggactccatgcttctcttggaaaaccaccttcagtgtgaggagcccacgtcagttgtagtatctctgttcataccaacaatggctttgcacgtttcacagggctaccttgcccacacagttctgggtttgtggctaaagcggtggtgacctttttgttcagacctcaagggcccccagggcctctcgtgtaagagctgaacctatcattgctgacaaacctatttctccggtgtcctttttctgtccaatggccatttcagtgaaattctagaaaaggcagggaggcaggtttaggcaactaagttggagttttactcctaagctagaagcttcgcccagaccggtgtgctcctgtcctcgcacaggtggaagattggggttcatcttagtgaccctttatacctttgtgtatacatacgggctgcagactttgtgattgctcggtgtgcttaagctgttcccttcaacacagcagagggctgccacagccgagtgtcagttcttgcgccagggtggatggacgtgagattcaagtctaacggccttgtccacgttcccaccatcccttttctccattcgatatcctcacccttccagatggattcatccttcttgcttttttttttttttttatgtttttgctttgcttttttgagacaaggtctctccatatatcccagactatccatgaatgatcctcctacctgtttctagagtgctaggattacaggcatgcatgaccacacgtggcctcatcctttcttcctttcctgtttgcaaccttgcttattatatcagaaaggaggggaatactgggggtctgggaggaggaaacctggggcgaaaaacctgtagcacacaaaacctgtacacactgtctgaaggaagggggtggggagcgctcagtctgctccactctgctgggcggcaagacctagaacgggccctgcactgtcccaccatgggttgtggtctcagaaatcgcttcagcagctcttccctggaggctgtgacagagcagccaggaggagccgactaggagtcctggcttccaacctctctgaaggaagcagagggatgctttttatattttgtacatagaactcaacatttatgtaaacagtgtttttgaataaagtttttgttggtttggtttttgcaaatctaaaaaaaaaaaaaaaaaaaaaaa

SEQ ID NO: 53 - DNA, 8044 bp, Homo sapiens
  Human BCL11b (NM_138576.3)
tgcgctttccacctaccagaccctgaaagaaagtgtcaggagccggtgcaaaacccagtttaagttcaagaagacatttgcaagtgcaagaggccaagcagtttgaagaagtgtaagagattttttttccttcgaaagaatatatttttaaagaaaccagccagtccgcggaaagcaacagcagttttttttttttttgcctctttttcttattttagatcgagaggtttttcttgcttttcttcccttttttttctttttgcaaacaaaacaaaaaacagcatagaagaaagagcaaaataaagaagaagaagaggaggaagagagggaaagagaggaagggaaaaaaaacaccaacccgggcagaggaggaggtgcggcggcggcggcggcggcggcagcggcggcagcggcgcggcggcggctcggaccccctcccccggctccccccatcagtgcagctctccgggcgatgccagaatagatgccggggcaatgtcccgccgcaaacagggcaacccgcagcacttgtcccagagggagctcatcaccccagaggctgaccatgtggaggccgccatcctcgaagaagacgagggtctggagatagaggagccaagtggcctggggctgatggtgggtggccccgaccctgacctgctcacctgtggccagtgtcaaatgaacttccccttgggggacatcctggtttttatagagcacaaaaggaagcagtgtggcggcagcttgggtgcctgctatgacaaggccctggacaaggacagcccgccaccctcctcacgctccgagctcaggaaagtgtccgagccggtggagatcgggatccaagtcacccccgacgaagatgaccacctgctctcacccacgaaaggcatctgtcccaagcaggagaacattgcagggccgtgcaggcctgcccagctgccagcggtggcccccatagctgcctcctcccaccctcactcatccgtgatcacttcacctctgcgtgccctgggcgctctcccgccctgcctccccctgccgtgctgcagcgcgcgcccggtctcgggtgacgggactcagggtgagggtcagacggaggctccctttggatgccagtgtcagttgtcaggtaaagatgagccttccagctacatttgcacaacatgcaagcagcccttcaacagcgcgtggttcctgctgcagcacgcgcagaacacgcacggcttccgcatctacctggagcccgggccggccagcagctcgctcacgccgcggctcaccatcccgccgccgctcgggccggaggccgtggcgcagtccccgctcatgaatttcctgggcgacagcaaccccttcaacctgctgcgcatgacgggccccatcctgcgggaccacccgggcttcggcgagggccgcctgccgggcacgccgcctctcttcagtcccccgccgcgccaccacctggacccgcaccgcctcagtgccgaggagatggggctcgtcgcccagcaccccagtgccttcgaccgagtcatgcgcctgaaccccatggccatcgactcgcccgccatggacttctcgcggcggctccgcgagctggcgggcaacagctccacgccgccgcccgtgtccccgggccgcggcaaccctatgcaccggctcctgaaccccttccagcccagccccaagtccccgttcctgagcacgccgccgctgccgcccatgccccctggcggcacgccgcccccgcagccgccagccaagagcaagtcgtgcgagttctgcggcaagaccttcaagttccagagcaatctcatcgtgcaccggcgcagtcacacgggcgagaagccctacaagtgccagctgtgcgaccacgcgtgctcgcaggccagcaagctcaagcgccacatgaagacgcacatgcacaaggccggctcgctggccggccgctccgacgacgggctctcggccgccagctcccccgagcccggcaccagcgagctggcgggcgagggcctcaaggcggccgacggtgacttccgccaccacgagagcgacccgtcgctgggccacgagccggaggaggaggacgaggaggaggaggaggaggaggaggagctgctactggagaacgagagccggcccgagtcgagcttcagcatggactcggagctgagccgcaaccgcgagaacggcggtggtggggtgcccggggtcccgggcgcggggggcggcgcggccaaggcgctggctgacgagaaggcgctggtgctgggcaaggtcatggagaacgtgggcctaggcgcactgccgcagtacggcgagctcctggccgacaagcagaagcgcggcgccttcctgaagcgtgcggcgggcggcggggacgcgggcgacgacgacgacgcgggcggctgcggggacgcgggcgcgggcggcgcggtcaacgggcgcgggggcggcttcgcgccaggcaccgagcccttccccgggctcttcccgcgcaagcccgcgccgctgcccagccccgggctcaacagcgccgccaagcgcatcaaggtggagaaggacctggagctgccgcccgccgcgctcatcccgtccgagaacgtgtactcgcagtggctggtgggctacgcggcgtcgcggcacttcatgaaggaccccttcctgggcttcacggacgcacgacagtcgcccttcgccacgtcgtccgagcactcgtccgagaacggcagcctgcgcttctccacgccgcccggggacctgctggacggcggcctctcgggccgcagcggcacggccagcggaggcagcaccccgcacctgggcggcccgggccccgggcggcccagctccaaggagggccgccgcagcgacacgtgcgagtactgcggcaaggtgttcaagaactgcagcaacttgacggtgcaccggcggagccacaccggcgagcggccttacaagtgcgagctgtgcaactacgcgtgcgcgcagagcagcaagctcacgcgccacatgaagacgcacgggcagatcggcaaggaggtgtaccgctgcgacatctgccagatgcccttcagcgtctacagcaccctggagaaacacatgaaaaagtggcacggcgagcacttgctgactaacgacgtcaaaatcgagcaggccgagaggagctaagcgcgcgggccccggcgccccgcacctgtacagtggaaccgttgccaaccgagagaatgctgacctgacttgcctccgtgtcaccgccaccccgcaccccgcgtgtccccggggcccaggggaggcggcactccaacctaacctgtgtctgcgaagtcctatggaaacccgagggttgattaaggcagtacaaattgtggagccttttaactgtgcaataatttctgtatttattgggttttgtaatttttttggcatgtgcaggtactttttattattattttttctgtttgaattcctttaagagattttgttgggtatccatcccttctttgttttttttttaacccggtagtagcctgagcaatgactcgcaagcaatgttagaggggaagcatatcttttaaattataatttggggggaggggtggtgctgcttttttgaaatttaagctaagcatgtgtaatttcttgtgaagaagccaacactcaaatgacttttaaagttgtttactttttcattccttccttttttttgtcctgaaataaaaagtggcatgcagttttttttttaattattttttaattttttttttggtttttgtttttggggtggggggtgtggatgtacagcggataacaatctttcaagtcgtagcactttgtttcagaactggaatggagatgtagcactcatgtcgtcccgagtcaagcggccttttctgtgttgatttcggctttcatattacataagggaaaccttgagtggtggtgctgggggaggcaccccacagactcagcgccgccagagatagggtttttggagggctcctctgggaaatggcccgacagcattctgaggttgtgcatgaccagcagatactatcctgttggtgtgccctggggtgccatggctgctattcgctgtagattaggctacataaaatgggctgagggtacctttttggggagatggggtggcctgcagtgacacagaaaggaagaaactagcggtgttcttttaggcgttttctggcttgacggcttctctctttttttaaatcacccccaccacataaatctcaaatcctatgttgctacaaggggtcatccatcatttcccaagcagacgaatgccctaattaattgaagttagtgttctctcatttaatgcacactgatgatattgtagggatgggtggggtggggatcttgcaaatttctattctcttttactgaaaaagcaggggatgagttccatcagaaggtgcccagcgctacttcccaggtttttattttttttttcctatctcattaggttggaaggtactaaatattgaactgttaagattagacatttgaattctgttgacccgcactttaaagcttttgtttgcatttaaattaaatggcttctaaacaagaaattgcagcatattcttctctttggcccagaggtgggttaaactgtaagggacagctgagattgagtgtcagtattgctaagcgtggcattcacaatactggcactataaagaacaaaataaaataataatttataggacagtttttctactgccattcaatttgatgtgagtgccttgaaaactgatcttcctatttgagtctcttgagacaaatgcaaaactttttttttgaaatgaaaagactttttaaaaaagtaaaacaagaaaagtacattctttagaaactaacaaagccacatttactttaagtaaaaaaaaaaaaaattctggttgaagatagaggatatgaaatgccataagacccaatcaaatgaagaaataaacccagcacaaccttggacatccattagctgaattatcctcagccccttttgtttttgggacaacgctgcttagatatggagtggaggtgatttactgctgaattaaaactcaagtgacacaagttacaagttgatatcgttgaatgaaaagcaaaacaaaaacaattcaggaacaacggctaattttttctaaagttaaatttagtgcactctgtcttaaaaatacgtttacagtattgggtacatacaagggtaaaaaaaaaattgtgtgtatgtgtgttggagcgatctttttttttcaaagtttgcttaataggttatacaaaaatgccacagtggccgcgtgtatattgttttcttttggtgacggggttttagtatatattatatatattaaaatttcttgattactgtaaaagtggaccagtatttgtaataatcgagaatgcctgggcattttacaaaacaagaaaaaaaatacccttttcttttccttgaaaatgttgcagtaaaatttaaatggtgggtctataaatttgttcttgttacagtaactgtaaagtcggagttttagtaaatttttttctgccttgggtgttgaatttttatttcaaaaaaaatgtatagaaacttgtatttggggattcaaaggggattgctacaccatgtagaaaaagtatgtagaaaaaaagtgcttaatattgttattgctttgcagaaaaaaaaaaaatcacatttctgacctgtacttatttttctcttcccgcctccctctggaatggatatattggttggttcatatgatgtaggcacttgctgtatttttactggagctcgtaattttttaactgtaagcttgtccttttaaagggatttaatgtacctttttgttagtgaatttggaaataaaaagaaaaaaaaaacaaaaacaaacaggctgccataatatatttttttaatttggcaggataaaatattgcaaaaaaaacacatttgtatgttaagtcctattgtacaggagaaaaagggttgtttgacaacctttgagaaaaagaaacaaaaggaagtagttaaatgctttggttcacaaatcatttagttgtatatattttttgtcggaattggcctacacagagaaccgttcgtgttgggcttctctctgaacgccccgaaccttgcatcaaggctccttggtgtggccacagcagaccagatgggaaattatttgtgttgagtggaaaaaaatcagtttttgtaaagatgtcagtaacattccacatcgtcctccctttctctaagaggccatctctaagatgtcagatgtagaggagagagagcgagagaacatcttccttctctaccatcactcctgtggcggtcaccaccaccacctctcccgcccttaccagcagaaagcaatgcaaactgagctgctttagtccttgagaaattgtgaaacaaacacaaatatcataaaaggagctggtgattcagctgggtccaggtgaagtgacctgctgttgagaccggtacaaattggatttcaggaaggagactccatcacagccaggacctttcgtgccatggagagtgttggcctcttgtctttcttccctgctttgctgctttgctctctgaaacctacattccgtcagtttccgaatgcgagggcctgggatgaatttggtgcctttccatatctcgttctctctccttcccctgcgtttcctctccatccttcatcctccattggtcctttttttttctttcattttttatttaatttcttttcttcctgtctgttcctcccctaatcctctattttatttttattttttgtaaagccaagtagctttaagataaagtggtggtcttttggatgagggaataatgcatttttaaataaaataccaatatcaggaagccattttttatttcaggaaatgtaagaaaccattatttcaggttatgaaagtataaccaagcatccttttgggcaattccttaccaaatgcagaagcttttctgttcgatgcactctttcctccttgccacttacctttgcaaagttaaaaaaaaggggggagggaatgggagagaaagctgagatttcagtttcctactgcagtttcctacctgcagatccaggggctgctgttgcctttggatgccccactgaggtcctagagtgcctccagggtggtcttcctgtagtcataacagctagccagtgctcaccagcttaccagattgccaggactaagccatcccaaagcacaagcattgtgtgtctctgtgactgcagagaagagagaattttgcttctgttttgtgtttaaaaaaccaacacggaagcagatgatcccgagagagaggcctctagcatgggtgacccagccgacctcaggccggtttccgcactgccacaactttgttcaaagttgcccccaattggaacctgccacttggcattagagggtctttcatggggagagaaggagactgaattactctaagcaaaatgtgaaaagtaaggaaatcagcctttcatcccggtcctaagtaaccgtcagccgaaggtctcgtggaacacaggcaaacccgtgattttggtgctccttgtaactcagccctgcaaagcaaagtcccattgatttaagttgtttgcatttgtactggcaaggcaaaatatttttattaccttttctattacttattgtatgagcttttgttgtttacttggaggttttgtcttttactacaagtttggaactatttattattgcttggtatttgtgctctgtttaagaaacaggcacttttttttattatggataaaatgttgagatgacaggaggtcatttcaatatggcttagtaaaatatttattgttcctttattctctgtacaagattttgggcctctttttttccttaatgtcacaatgttgagttcagcatgtgtctgccatttcatttgtacgcttgttcaaaaccaagtttgttctggtttcaagttataaaaataaattggacatttaacttgatctccaaa

SEQ ID NO: 54 - DNA, 7922 bp, Mus <mouse, genus>
  Mouse Bcl11b (NM_001079883.1)
aatttattttagccttttctctattttagagcaagccatcttcctggctttttcttctttctttttgcaaaaacaaaaacaaaaacacagcccagaagaaagagcaaaataaagacgaagaagaagaagaggaggaggaagaggaagagaggaagggcagaggcaccaacccgggcggaggaggaggcgcggcggcggcggcggctcagaccccctccccggcccgcatctgtgcagctttccgggcgatgccagaatagatgccggggcaatgtcccgccgcaaacagggcaacccgcagcacttgtcccagagggaactcatcacgccagaggctgaccatgtggaggctaccatcctcgaggaagacgagggtctggagatagaggagcctagcagcctggggctgatggtgggaggccccgaccctgatctactcacctgtggccagtgtcagatgaacttcccgctgggggacatcctggtttttatagagcacaagaagaaacagtgtggaggcctgggcccctgctacgacaaggtcctggacaagagcagtccacctccctcctctcgctctgagctcaggagagtatctgagccagtggagatcgggatccaggtcacccctgatgaagatgaccacctactgtcacccacgaaaggcatctgtcccaagcaggagaacattgcagggccgtgcaggcctgcccagctgccatcgatggcccccatagctgcctcctcttcccaccctcccacctccgtgattacttcacctctgcgtgccctgggcgttctcccaccctgtttcccgctgccttgctgtggtgcacgccccatctcgggcgacgggactcagggtgagggtcagatggaggctccctttggatgccagtgtgagttgtcaggtaaagatgagccttccagctacatttgcacaacatgcaagcagcccttcaacagcgcctggttcctgctgcagcacgcacagaacacacatggcttccgaatctacctggagcctgggccggccagcacctcgctcacgcccaggctcaccatcccgccaccgctcgggccggagaccgtggcgcagtccccactcatgaatttcctgggggacagcaatcctttcaacctgctgcgcatgacgggccccatcctgcgggaccaccctggcttcggtgagggccgcttgccaggtacgccaccgctcttcagcccaccgccacgccatcacttggacccacaccgcctcagtgcagaggagatggggctcgtggcccagcaccccagtgccttcgaccgagtcatgcgcctgaaccccatggccatagactctcctgccatggacttctcccggcggctgcgagaactggccggcaacagctccacgccgccgcccgtgtccccaggccgtggcaaccctatgcaccggctgctgaaccctttccagcccagtcccaagtccccgttcctcagcacgccaccgctgccacccatgcctgcgggcacaccgccaccgcagccgcctgccaagagcaagtcctgtgagttctgcggcaagaccttcaagttccagagcaatctcatcgtgcaccggcgcagccacacgggcgagaagccctacaagtgccagctgtgcgaccatgcgtgctcgcaggcgagcaagctcaagcgccacatgaagacgcacatgcacaaggcgggctctctggctggccgctcagacgacgggctctcagctgccagctcccctgagccgggcaccagcgagctgccaggtgacctgaaagcggccgatggcgacttccgccaccatgagagcgacccatctctgggccccgagcctgaggacgacgaggacgaggaggaggaagaagaggagctgctgctggagaacgagagccggcctgagtcgagcttcagcatggactcggagctgggccgtggccgcgagaacggaggtggcgtgccaccgggggtggcgggcgcaggggctgcagctgcggctctggcggatgagaaggctctggccctgggcaaggtgatggaggacgcagggctgggcgcactgccgcagtatggggagaagcggggcgccttcctgaagcgtgcaggcgacacgggtgatgccggagctgttggctgtggggacgcgggtgcaccgggtgcagtgaacgggcgcggcggggccttcgcgccaggcgcagagccctttccagctctcttcccacgcaagccagcaccgctgcccagccctgggctcggtggtcccgcgctgcacgcggccaagcgcatcaaggtggagaaagacctggagctgccacctgccgccctcatcccatctgagaacgtgtactcgcagtggctcgtgggctacgcagcatcgcgccacttcatgaaggacccattcctgggcttcacggatgcgcgccagtcgcctttcgccacatcgtcggaacattcctctgagaacggcagcctgcgcttctcaacgccacccggggacctgctggacggcgggctgtccgggcgcagtggcacggcgagcgggggcagcacacctcacctgggtggtccgggtcctgggaggccgagctccaaggagggccgccgcagcgacacatgtgagtactgcggcaaggtcttcaagaactgtagcaacctgacggtgcaccggaggagccacaccggcgagcggccttacaagtgcgagctgtgcaactacgcgtgcgcgcagagcagcaagctcacgcgccacatgaagacgcacgggcagatcggcaaggaggtgtaccgctgcgacatctgccagatgcccttcagcgtctacagcaccctggagaaacacatgaaaaagtggcacggtgaacacttgctgactaatgatgtcaaaatcgagcaggctgagaggagctaagcgcatacgtgggggacactgcgtgcgtgcgtctgtacagcgtgaccatcgccaaccttcgccaacgggaccggtgaccggactggcctctgcatccccggggcccagggaggcggcagtccagcctaacctgtgtctgcgaagtcctatggaaacctgagggttgattaaggcagtaaaaaattaaaaaaaaaaaaacaaaaaaacaaaaaaatttgtggagccttttaactgtgcaataatttctgtatttattgggttttgtaatttttttggcatgtacgtgcaggtacctattattattattatttctgtttaaattcctttaaaagattttgttgagtatccatcccttcatttttttttttaataacccagtagtagtctgagcaatgactcgcaagtgacgtagagggaagctatcttttaaattataattttgtgtgtgtgtgtgggggggtgctgcttttttgaaatttaagctaagcatgtgtaatttcttgtcaagaagccaacacttaaatgacttttaaagttgtttgcgttttcatcatttactttgtcctgaaatgaaaagtggcatgtgggatttttttccgggggggaggggtggctttcaaaaccattttttttttccgggaggtggatgtacagcggattacaatctttaaaattgtagcactttgtcttagcatcgcattggagagttagcactgatgtcctcctgagccacagaggcgtctctgtgtggaattcaactttcatgctatggaaggaaaatgttgaggggggcgtggcaaacgagcctctcccccacttgggaccccgagaatcttttccagggtgactctaggaacagcccccacatcctgcaattgtgtgttaccaggagatatgataatgtccttttctgggggagcttggcgtattgggaagccgcctctgccctttgctgtagatttggctgcataaaatgggccgaggatacccactgggtagacagctgtggcctgtagtggcgggaaagaagagactaacaatgttctctcaggcttctcctggcaagatggcttctcttttcagcccccagcctacagataaatcccaggtgtccattgctacagtggtaacttgactgtgtcccaagcagacaactggccctgatggtgaactggagaagttagctgcggggtcgctcatctcacgctgatgggcactgtagggcaaaggaatctcacccgttctctcttcccggaggagctggtaagagttctgtccaaggtgccccacgctgcttccgtttctgtgttttgtcttttccttcctccaattaagttgggacatactatacattggacttgttgggatttgatgtttgaattctgttgacccgcactttaaagcttttgtttgcatttaaattaaatggcttctaaacaagaaattgcagcatattcttgtctttggcccagaggtgggttaaactgtaagggacagctgagattgagtgtcagtgttgctaagcgtggcattcacaatactggcactataaagaacaaaattaaataatttattggacagtttctctactgccattcaatttgatgtgcgtgccttgaaaaccgatcttcctatttgagtctcttgagacaaatgcaaaactctcttttttttttgagatgaaaaaaaaaaaagactttttaaaaagcaaacaagagaagtacattctttagaaacaaagccacatttactttaaattaaaaaaaaaaatcctggttgaagagagaggacgggaaaatgccataagaccagtcaaatgaagaaataaacccagcacagccctggacatctattagcagaatcgttttcagacccccctcccccttttttggggcaacgctgctagatatggagtggaggtgacttactgctgaattaaaactcacgtgacacaagccgatattgttgaatgaaaaaacaaacaacaacaacaacaacaaaaaacaattcaggaacaatggctgattttttttttcctcctaaatttaaatttagtgcactctgtcttaaaaatacgtttacagtattggatacatacaagggtaaaataaatcgtgtgtatgtgtgttggagcgatctttttattttattttattttcaaagtctgcttaataggttatacagaatgccacaatggctaggtgtatattgttttcttttggtgatggggttttagtatacattatatatattgaaatttcttgattactgtcaaagtggaccagtatttgtaataattgagactgcctgggcattttacaaaatgagaagaaaaaaaagtcctttttcttttccttgaaaccgttacagtaagttttaaatggtgggtctataaaatctgctctgtcacagcaacctgtaaagtcggagttttagtaaatttttttctgccttgggtgttgaatttttattttgaaaacaaaatgtatagaaacttgtatttggggtttaaagggggattgctgcaatgtgtagaaaaagtatgtagagaaagtgcttaatattgttactgctttgcagaagaagaaaaaaaaaatcacacttctgacctgtgcgtatttttctctcccacctccctctggaatggatctattggtcggttcatatgatgtaggctctcgctgtatttttaactggagcttgtaattttttaactgtaagcttgtccttttaaagggatttaaatgtacctttttgttagtgaatttggaaataaaaagagaaaaaaaaaacaaaaacaaacaggctgccataatatatttttttaatttggcaggataaaatattacaaaaaaaaaatcccccacaaaacaacaaacaaacaaaaatcccacccacatttgtatgttaagtcctcttgtatggggtggggggagggttgtttgacaaccttcaagagaaaaagacacagaaagagacatgctttgattcacaagtcattttagttgtatatagtctgtcagaattggcctactcaaaaagaactgttggctttgggctttcattcgaatgccccaactttgcatctggcctccttggtgaggccacagccgacttgatggcaagtccttacttgtgttgagtggagaaaagaaagcccttcctccaagaggcagtctataagatggtagcgcggtgagagagcaagggaggttaccttctccgctgtggctactgcggccaccccctccaccccctggccacgctcaggagcagagagaatcgacagctgcttttgtccttgagcaaacctggatggagcagcgaagcttctgagaggagcagctgggcccaggggagcctctgccactgagactggtgcaggcgggacagaggagagccttgcacgcaggtcctgttcccttggaatgtctgctccattttccccctctgtctctctgcttttctctgcaattccatccgtttcagaccagtgaggcctggaatgaaggaattctgtgccttcccatctatgttccctccgtcctccccaggctctgcctactctttgtggactcctctttaattttcttcctcctttgccccctctccccaaaccctcttttctcttcctttcttctctccttcttttcttcctcctcctcctcttttctcctcctcctcctcctcctcctcctcctcctcctcctcctcttcttcttcttcttcttcttcttcttctttttcttcttctcctcctccttcttcttcttttttttttttttgtaaagccaagtagctttaagataataaaatggttgtttattggatgagggaataatgatacactccacaaatacctatatcaggaagccatttttttttaatttcaggaaatgtaagaaaccatcatttcaggttatgaaagcgtgattgtgcatctttccaggcagatctttactaaatgcagagtctgtctcactgtttcccatttgacacagttaaaagatgggggcctagtgggaggccaggcctaagtctcagtgtcctgcatgcctgccctacggcccagggttaccctgcccttttgacaccctgcctctctgctacctgggagcctctgtgtggttctcctgtgctcataaaagctagccagtgctcaccagctcacctatcaccagaatgccaggactaagccatcctaaagcacaaggacttgtgtgtctctgtcaactgcagagagaagaggatttttgcttctcttatcaaagagaaaaatcaaccaaccaacctacccgaagcaggtgacccagcctaagggctctaccgcgggtgacccagccgacctcaggtcgggttccacactgccacaactttacccaaagttgctccctattggaacctgccacttgccattggagggtcatgggggggtggggggagaggagactggattactcgaagcaaaatgtgaaccctgaagcgaacacagccttccacctggccctccccgtccgaggtttgattccgtgattttggtgctttctgtgtctgccctgcatagccaaggcacattgatctctgcggtttgcttttgtactggcaaggcggaatatttttattaccttttctattacgtatcgtatgagcttttgttgtttgcctagagggtttgtctcttacagcaagtttggagctatttattattgcttggtatttgtgctctgcttttaagaatgggcacttggttttatttttgtttgtttgtttttttgttgttttttaattatggataaaatgttgagatgacaaaaggtcatttcaatatggcttagtaaaaatatttattgtttcttctctgtacaagattttgggcctcttttttcccccttaatgtcacaatgttgagttcagcatgtgtctgccatttcatttgttcaaaaccaagtttgttctggtttcaagttatgaaaataaattgggacatttaacttga

SEQ ID NO: 55 - DNA, 7530 bp, Homo sapiens
  Human NFATC2 (or NFAT1) (NM_012340.4)
agcaggaagctcgcgccgccgtcgccgccgccgctcagcttccccgggcgcgtccaggacccgctgcgccaggcgcgccgtccccggacccggcgtgcgtccctacgaggaaagggaccccgccgctcgagccgcctccgccagccccactgcgaggggtcccagagccagccgcgcccgccctcgcccccggccccgcagccttcccgccctgcgcgccatgaacgcccccgagcggcagccccaacccgacggcggggacgccccaggccacgagcctgggggcagcccccaagacgagcttgacttctccatcctcttcgactatgagtatttgaatccgaacgaagaagagccgaatgcacataaggtcgccagcccaccctccggacccgcataccccgatgatgtcctggactatggcctcaagccatacagcccccttgctagtctctctggcgagccccccggccgattcggagagccggatagggtagggccgcagaagtttctgagcgcggccaagccagcaggggcctcgggcctgagccctcggatcgagatcactccgtcccacgaactgatccaggcagtggggcccctccgcatgagagacgcgggcctcctggtggagcagccgcccctggccggggtggccgccagcccgaggttcaccctgcccgtgcccggcttcgagggctaccgcgagccgctttgcttgagccccgctagcagcggctcctctgccagcttcatttctgacaccttctccccctacacctcgccctgcgtctcgcccaataacggcgggcccgacgacctgtgtccgcagtttcaaaacatccctgctcattattcccccagaacctcgccaataatgtcacctcgaaccagcctcgccgaggacagctgcctgggccgccactcgcccgtgccccgtccggcctcccgctcctcatcgcctggtgccaagcggaggcattcgtgcgccgaggccttggttgccctgccgcccggagcctcaccccagcgctcccggagcccctcgccgcagccctcatctcacgtggcaccccaggaccacggctccccggctgggtacccccctgtggctggctctgccgtgatcatggatgccctgaacagcctcgccacggactcgccttgtgggatcccccccaagatgtggaagaccagccctgacccctcgccggtgtctgccgccccatccaaggccggcctgcctcgccacatctacccggccgtggagttcctggggccctgcgagcagggcgagaggagaaactcggctccagaatccatcctgctggttccgcccacttggcccaagccgctggtgcctgccattcccatctgcagcatcccagtgactgcatccctccctccacttgagtggccgctgtccagtcagtcaggctcttacgagctgcggatcgaggtgcagcccaagccacatcaccgggcccactatgagacagaaggcagccgaggggctgtcaaagctccaactggaggccaccctgtggttcagctccatggctacatggaaaacaagcctctgggacttcagatcttcattgggacagctgatgagcggatccttaagccgcacgccttctaccaggtgcaccgaatcacggggaaaactgtcaccaccaccagctatgagaagatagtgggcaacaccaaagtcctggagatacccttggagcccaaaaacaacatgagggcaaccatcgactgtgcggggatcttgaagcttagaaacgccgacattgagctgcggaaaggcgagacggacattggaagaaagaacacgcgggtgagactggttttccgagttcacatcccagagtccagtggcagaatcgtctctttacagactgcatctaaccccatcgagtgctcccagcgatctgctcacgagctgcccatggttgaaagacaagacacagacagctgcctggtctatggcggccagcaaatgatcctcacggggcagaactttacatccgagtccaaagttgtgtttactgagaagaccacagatggacagcaaatttgggagatggaagccacggtggataaggacaagagccagcccaacatgctttttgttgagatccctgaatatcggaacaagcatatccgcacacctgtaaaagtgaacttctacgtcatcaatgggaagagaaaacgaagtcagcctcagcactttacctaccacccagtcccagccatcaagacggagcccacggatgaatatgaccccactctgatctgcagccccacccatggaggcctggggagccagccttactacccccagcacccgatggtggccgagtccccctcctgcctcgtggccaccatggctccctgccagcagttccgcacggggctctcatcccctgacgcccgctaccagcaacagaacccagcggccgtactctaccagcggagcaagagcctgagccccagcctgctgggctatcagcagccggccctcatggccgccccgctgtcccttgcggacgctcaccgctctgtgctggtgcacgccggctcccagggccagagctcagccctgctccacccctctccgaccaaccagcaggcctcgcctgtgatccactactcacccaccaaccagcagctgcgctgcggaagccaccaggagttccagcacatcatgtactgcgagaatttcgcaccaggcaccaccagacctggcccgcccccggtcagtcaaggtcagaggctgagcccgggttcctaccccacagtcattcagcagcagaatgccacgagccaaagagccgccaaaaacggacccccggtcagtgaccaaaaggaagtattacctgcgggggtgaccattaaacaggagcagaacttggaccagacctacttggatgatgagctgatagacacacaccttagctggatacaaaacatattatgaaacagaatgactgtgatctttgatccgagaaatcaaagttaaagttaatgaaattatcaggaaggagttttcaggacctcctgccagaaatcagacgtaaaagaagccattatagcaagacaccttctgtatctgacccctcggagccctccacagcccctcaccttctgtctcctttcatgttcatctcccagcccggagtccacacgcggatcaatgtatgggcactaagcggactctcacttaaggagctcgccacctccctctaaacaccagagagaactcttcttttcggtttatgttttaaatcccagagagcatcctggttgatcttaatggtgttccgtccaaatagtaagcacctgctgaccaaaagcacattctacatgagacaggacactggaactctcctgagaacagagtgactggagcttggggggatggacgggggacagaagatgtgggcactgtgattaaaccccagcccttgcgttcgtttttccaggtcacagatacagctcctgtaccttttgaaggcaaggagttctcagagcaaccaaaggaacgtgacccaagagcccagcttacaggctgaagaaacccaaaaccctcgatagagacagaaactgaactgtcagtccttagagctcgcccagtccatgccacaactgggccacagctaaagctttatttttgaattctcattccaaaaccaaactgtcttgcccagacaagatcacctgttaagacttcttggcgttaagttatgacatgtatacgcgtttgttattattattttttctgctttaaaaggctgaccagggcacctagccctggagctgtcttggcgagctgttctttaacccctgcagcacgcagtcctgctaacacaatttccatagacttggggggctgacccaggctgcagagagcaagcacctgtctgctgcagctgtacaacctggatgctttgcaaggttccggcttgctttcttcctagcagccagagtgcttttccgtaaagcggtggagaatctcaagcatgtgcatttaattgaggaatagcagaagggctaaagcaaccaagaaaagaagtgtgggtatttttgttaagtaaaacagcccaagtgcttctggaggtgggtttctaccaagatagaggaaaagggctgaattccctctaagtgggacagccgagctcaggatgtgcttcccagcttcactggttaatttgacctgaacctatttaaagatcccttctgcccctgaagacctatccgcactcaaattctaacatgaagaaatctactcgaatgcatcctttactttgaatgagctctattcggttgcatgttatatgtgatttccttcctcccaactgtttccactgagcgcacccagtctcccctagtcttcctctgtgggtgtgatttttgtgatttttacaaacaaaacccttgaagttcttggcagatgtgtttgtttctgtttgcatgtactgcagataccccaggacaagcgggggattcatttttcagccattcagttgtttcctcaataatccgcagcaaagtgaaaatattcttagcactcagactgtacttagagtgttttctcagtccagtctgtacagtctgtaggcagaaggcctcagaagaaagtcatggccactcagtgcccactgtgggctttgtaagtcctggctctcccgtcaaggttacccagaggtaaaagcttcctgggagtggggccaggtgtgtttggcactccagatagaaggcaaaatgctcagattcgggcctgtgcacttgtatgcaacctgtcggtcgatacctagcatttatttttccctgacaatgaacgacctttccctcacccaccctaagctcaaagagtttagcaaaattctcttttaaataaacagaatgccagtaagaggttgacccctaccatggaacttctgggatgctaaatacttcctcatgaacaaaataagttccttattataagttccttatactagcagcttcacctaaagaattttctctccagcaatattgacttcactggggaaaagccaagagtgtgtggtgagtgatttgttctcactcgacctggctaggactggctaggagctgttttttgtacatgagggaatttgggctttcctcagttatctgaatgttttacccaagtgccttcctgctattgtagcaaagtagctcagcttccttgtccacagggtgaaaaaggactaatgcattttccatcagttttctaactatgttagcaaaaacggcctcctggtagctcaacctcctgtacgcgtgtgtgtgtgtaatacacacacaaataaacccctctgtttttctaagacatcttagctggatattataggaagcactttcataaacaactgtaacaaatcgcaaaggaaagagaaacaaaagcattagatttgagacataaacaggcaagagaaagtgtattaggaactgacagctatcaaggaagttttgtcagttacaaatgctaggaggaaattttgccaagaaggatggctcatgaaatatttccagtacgggaagaggcaataagatcctctaagagaatgagaaagtaggggtgtctaaatggtaaagatgggtgtgttgcacgtgtgttagaaggatctcagttgagtgaaggtttgcactgctacatctaagttaatgtaaatatgtagcactctgacaggtctaccgtgttgctgaatgtagtatatttccaaagtttgcaagtcttcctgtattgtacaaagatgctgctgcttgataatatgtatagcaatccagattagtatgttattaaattttattttcttacctgtatttttatgctttttacctgtcctcaaaatattacacccctgttggaattagatttatatttataaatggtcagaaatctttttaagtgtctctttttacacataggttgatttttttttcttaagagaaatgatgtattcttgaaacatttgttactcattccaggaaacaaaaacccatataataaaacccccactcagagcctgttagtcacctctctagaagatggcatctcaggagaaggaatggctttgtggaagaaggaatcacctttttcttgctcaagaattatgctgacttcagccctgagcctggatctggtcactgagaatcatcaagtgtctagatcctccccccaaaataactaatttagtaggtgattttgattttaaaaaattgacaccaaaaccctgcctgcattgtaatggaattcgaaaagaattcatgttcacagaactcaacgttcaggctaatatttacagaagggaccaaatctaaatcctggtagataactcctgtatgctttatccaaaggacacccacagttttccagcatagatataaccaaggatgaattgattccttcaaagaactgggaggcacggatattgcattttttgtttacatccagtagccaagacgcctcagtgagccagtcttgggcagaggctgtcacatttaggcagattggaagttggtatgttctaattctcactctggactacagtgaggctgaatttatcatgtcaaaaaaaaaaaaaaaaaaagacctttccaagtgctttctattgctcagaattgaaagaatgttttcatttcaagtttacaagaggcatggatggagttgtgacgttcttgacaagctgggctaacctttcccgaacttgtttcccggaggcaaggtgctcggtgacccagcgcatcttaaccttgggtctcctaggctcgaggctagggcattacgtttcgtggaaccaaagcagccaattgcatagcaagtattttcctgcattccaattaaatgcttaagaaaaagcagcatcctataaaattgtgatcataaacatccatttccctcagcttttgtgagtgccttgacttacagccaacatcactgtttaactcagtctgtttaaaaacaaacttttctggtggttgataacagagagttgctccctgagccatcagggtcctgggagctggaagtgaaagggttattaacattctacctttatgcagctgttggctgaccagaataaactccctgctgagttcaagctttgaatggaatggatgcaaatgatgttgtttccattagagcaggtgctcacagcattctgattggcctgagcagaccgaggctatggctgttgggacaagcttagcatcctggacatcttgtcaaagaacctcactcacccctctggcctctacagccctcagaggagagaaaaccaattctccaacaaacaggtctctccaacatggtggtgctggcaggcttaggtttagaaaatcctgactgttaaaggcgtttgaatacatcacattcctatgcaaatgtttttaatctccagtttaatgtagtttatttttcctatatgtaaagtatttttatacggcttgtatcatgatagtttagcaataaaacagttggaagcaacatctaaaaaa

SEQ ID NO: 56 - DNA, 6759 bp, Mus <mouse, genus>
  Mouse Nfatc2 (or Nfat1) (NM_010899.3)
aggctgcaacaggtgccttgagcaggaagctcgcgccgccacccgctccccggacgcgtccaggacccactgcgccgtgagccatcctcggcctcaccgtgcgccacagatacggtgacccctgctctgcgccccgcgactctatacgaacccgcatcccgaacgccccgagccatggacgtcccggagccgcagcccgaccccgatggcggggacggccccggccacgagcccgggggcagtccccaagacgagctggacttttccatcctcttcgattatgactatctgaaccctatcgaagaagaaccgatcgcacataaggccatcagctcaccctccggactcgcatacccggatgatgtcctggactatggcctcaagccatgcaacccccttgccagtctctctggcgagccccctggccggttcggagagccggatagtatagggttccagaactttctgagcccggtcaagccagcaggggcttcgggcccgagccctcggatcgagatcactccatcccacgaactgatgcaggcagggggggccctccgtgggagagacgccggcctgtcccccgagcagccggccctggccctggccggcgtggccgccagcccgaggttcacactgcccgtgcccggctacgagggctaccgcgagccgctttgcttgagccccgctagcagcggctcctctgccagcttcatttctgacaccttctccccctacacctcgccctgcgtctcacccaataacgccgggcccgacgacctgtgtccccagtttcaaaacatccctgctcattattcccccagaacctctccaataatgtcacctcgaaccagcctcgccgaggacagctgcctgggccgacactcgcccgtgccccgtccggcatcccgctcctcctcacccggtgccaagcggaggcattcgtgcgcagaggctttggttgctcctctgcccgcagcctcaccccagcgctcccggagcccctcgccacagccctcgcctcacgtggcactgcaggacgacagcatccccgctgggtacccccccacggccggctctgctgttctcatggatgccctcaacaccctggccaccgactcgccctgcgggatcccctccaagatatggaagaccagtcctgacccgacgcctgtgtccaccgctccgtccaaggctggcctggcccgccacatctaccctactgtggagttcctggggccatgtgagcaggaggagaggaggaattccgctccagagtccatcctgctggtaccacctacttggcccaagcagttggtgccggccattcccatctgcagcatccctgtgactgcatccctcccaccactcgagtggccactctccaatcagtcgggctcctatgagctacggattgaggtccaacccaagccccatcaccgggcccactatgagacggagggcagccgtggcgctgtcaaagccccaacaggaggacaccctgtggtgcagctccacggctacatggagaacaagcctctggggcttcagatcttcattgggacagcagatgagaggatccttaagccgcacgccttctaccaagtacacaggatcactgggaaaacggtcaccaccacgagctatgagaagatcgtaggcaacaccaaggtcctggagatccccctggagccaaagaacaacatgagagccaccatcgactgtgcaggcatcctgaagctccgaaacgctgacatcgagctgcggaagggcgagacggacatcggcaggaagaacacgcgtgtgcgcctggtgttccgcgtgcacgtcccagagcccagtgggcgcatcgtctccctgcaggctgcgtccaaccccatcgagtgctctcagcgctctgcccacgagctgcccatggtggagagacaagacatggacagctgcctggtctacgggggccagcagatgatcctcacgggccagaacttcacagcggagtccaaggttgtgttcatggagaagactacagatgggcagcagatttgggagatggaagctacggtggataaagacaagagccagcctaacatgctttttgttgagatccccgagtatcggaacaagcacatccgcgtgcccgtgaaagtcaacttctacgtcatcaacggaaagaggaaacgaagtcagccacagcactttacctaccacccagtccctgccatcaagacagagcccagcgatgagtatgaaccatctttgatctgcagccccgcccatggaggcctggggagccagccatattacccacagcacccaatgctggccgagtccccctcctgccttgtggctaccatggccccctgccaacagttccgctcggggctctcatcccccgatgctcgctaccaacagcagagccccgcagctgccctctaccagagaagcaagagcctgagtcccggcctgctgggctaccagcagccgtccctcctggcagcacccttgggtctggctgatgcccaccgctctgtgctggtgcatgctggttctcaggggcaggggcagggctccaccctgccacacacatcctcggccagccagcaggcctcacccgtgatccactactcacccaccaaccagcagcttcgcggtgggggtcaccaggagttccagcatatcatgtactgtgaaaacttcggccccagctctgccaggcctggcccgcctcccatcaaccaaggtcagaggctgagcccgggcgcctaccccacagtcatccaacaacagactgccccgagccaaagagctgccaaaaacggacccagtgaccagaaggaagctctgcccacgggagtgaccgtcaaacaggaacagaacctggaccagacctacctggatgacgttaatgaaatcatcaggaaggagttttcaggacctccctcccgaaatcagacctagaaacaaacataatctcgcgacgccttctactctggaccgcttctgtctcctcctgccgtctgtgactggaacactgcgcatgcgcacagtgcacgcagatggtgtcagagcctgggagcctgctgccgcgcaaacagcatcttagccgttgtccatggtgactggacacgaaaagcaactgcctgctgaccaaagcctcattctcaactcaccaggatgctgaacctgagacgccaggctgcgctggcaggagaactggagaaactgcgatagcccacagacatggcttcattttttttgaattttctctttccaaagccaaacagccttgccctgacaggaccacctgtcccaacttctcagccttaagttataacacacgtacgtgtctgccagcttctgggcctttgctgtgttttcctctgcttcaaagagccaaccaaggaggccgtgggctgagagccctctcggccagctattccctaacctgctgcctacaccagactggctggtggcatccagtcccggctgcctgttgggaaccctgcttctgaaggttcccctctccaccccctccacccagaggtcgggagaaccttctggatccttgcattgactgttaaggagctaaaaccaccaaacccagtcaaaacctacacgtgtttgtcatgaccgccaccaaacagaacaaaggggccgaaatctccctttgctctgaactcaaagcaggaaagtgctggcttcaccctagtttgttttttgttttttgtttttaacctgaattcaggtaaagcctccatagactcctgaacgctgctgtatgagctgtgactcaggcggatccaccccagcatatgccttagtgtgatcaagccctgcctggcccggttgtgtgtcctgtgggattctccacacacactgcctgctacaggcggtcctccatggtcttcctcctggttcagttttcttcttccaacagcgtttcccccaatcatgtacgcaagaccgtcctctccccttgccttcatcccagatgtctctattgggcatcttcttaaagtgactttctcggctttgtgtgctaggcagaggacccgagaagcaagctacagtggctaagtacccgtggttggtttcttacgtcctggctttcttgtcaaagtcatctgaaaggaaatggctggagccgggccagctgtcgctggttctccttacagagaccccatgcccagggttcagcttgaacatgcaaatatgactttgtggtcaggacctagagtgtctcccccttgctgcagccctgggctttccctccactgaccccatgcgtagacctgggcagaattctcgtgtgaacccagaatgtctgtaagaagttgagcactaagccgctatgagtctaagtacttcctgctaagcaagaaacgttctgctggccctttacggccaggagcttctgactggagcaatgccgacttctctggggaagggtgatgagggttcggtgagtgacagttcacacttgccctggctgagagccacgttttgcacatgagggagtcaggcccttcctcagatatctccaagttttacccaagtgccttcctgcaattgtagtcattgtaattgtagctcagctgcactgtccacagggagacaaagggctaactcacttcccattagttttcatgtcagcgaaggggttcctggtagctcagactcctatactttcctctgtgtgtatgtgtgcatgtgtgtgtgtgtgtgtgtgtgtgtatatacgtgtacacaattctcttccctttatactatcttagccagatagtctcagaaacttgctgataaatatcccaaacagccaaggagagaaagcagcatctgttaccagacaaacaggccatagaaggtgtatgagcggcagagagctatggagaaggtttggtcagttacagactccaggggaaacgtggccgggagtgactgcttatcaaccatttccaggatggggagatgcagtctgatcttagcgaatgagaaaagatgcccgagcagtgacgacgagtgtaccgcacgtgggttagaggggcggaagcggaaatgtgtccttgctaaatctgtggtgtcgttccggtgacagttccatattgctaaatgtggcactttctcttccaagtccacacatctccctgactgtacaaaggcaccgctgatggggagtatatctatctacccagatcagtatggtattaaattttattttcttatttgtattttgatgctttttatctgcctttaaaatatctcacccctgttggagttagaacatatttataaatgaccagatgtctttttttaagggtctatttctttttttaaaaaaaatctatatcttcattttctgtaagagaaatggtatactcctgagttttgttttattttgttttgttttgttttgctttttgtttctcattctgggaaacaaatccaaagactcacctcgggtcctatcaagacctcaggatgggagagaaagggactttgtaggagagaacaccttttttagcttgagaaagagggcctgctccttcagctccatgtcagggctgtccctgagaaccgtacgtgaaaggtttggttggtggtctcaatctaaagccacagaactctgcctttccatggacaagctccttcaggcaggctgacagttgacagagccaaccacgtggagtcctcagaggtgacactgaggtgcagcatccaaagaacagccaccttctccccagcgcagcgtagccacggaccaagtgacctgggataacactgttcacatgcagcagcctggtcatccattatccagcaccaccagccgtggccagccgccggcagcactgtcacacagggaggccagaagccagtgtgttttaattagcactcagaacctataggaggctgagttggtttatcttcacaccacagtgctcagcatcaggagaaacgggggctacgtaacaactgtgttcatttgccgcgcttccgaaaagacagaggtggccaggctagggcgagtattcctggactctttgccgtcagggaaggctggaggaacccgacacatcctcaccactggcatctcccaagtttggacaccaaccttcatggacccaaaccaggcagctgcagagcgggaggtttccctgcagcccagcagttgcttaaatgaggcaacatcaccttcacctacgaccagcttacccgtgccttgacagacatacggccaccatcgttgtcttaatccagtttgtttacagctaactctaaatggtgggccaggagtggtgcttccctgagcaggacccctctgagatcacaatgaagtcctgggaactggagtcaaaagtgttaatgctttcagatgggaataaacgtccctgccctgcctggccctgcctggctctgccctctcaggctttagatggactgggtgcagacagtgctgttgctatgtgagtaggaaccccagcattctgtgagagcatcccagacatcagacatccccgtccccctgtcatttctcagccctcatgggagcctgctcatcgggctctgaaggccggggtttgggaaaatctccaccccactacctgaggagtcgggatatatcacattcctatgcaaaacgattttaatctccggtttcctgcagtttatttttgctatatgtaaagtatttttatacggcttatatgatgacagcttagcaataaacagttgagagcaactctaaaaaaaaaaaaaaaaaaa

SEQ ID NO: 57 - DNA, 2042 bp, Homo sapiens
  Human HOXB4 (NM_024015.4)
ggaaaacgagtcaggggtcggaataaattttagtatattttgtgggcaattcccagaaattaatggctatgagttcttttttgatcaactcaaactatgtcgaccccaagttccctccatgcgaggaatattcacagagcgattacctacccagcgaccactcgcccgggtactacgccggcggccagaggcgagagagcagcttccagccggaggcgggcttcgggcggcgcgcggcgtgcaccgtgcagcgctacgcggcctgccgggaccctgggcccccgccgcctccgccaccacccccgccgcccccgccaccgcccggtctgtcccctcgggctcctgcgccgccacccgccggggccctcctcccggagcccggccagcgctgcgaggcggtcagcagcagccccccgccgcctccctgcgcccagaaccccctgcaccccagcccgtcccactccgcgtgcaaagagcccgtcgtctacccctggatgcgcaaagttcacgtgagcacggtaaaccccaattacgccggcggggagcccaagcgctctcggaccgcctacacgcgccagcaggtcttggagctggagaaggaatttcactacaaccgctacctgacacggcgccggagggtggagatcgcccacgcgctctgcctctccgagcgccagatcaagatctggttccagaaccggcgcatgaagtggaaaaaagaccacaagttgcccaacaccaagatccgctcgggtggtgcggcaggctcagccggagggccccctggccggcccaatggaggcccccgcgcgctctagtgcccccgcacgcgggagccacgaacctcggggtgggggtgggcagtgagtgcaggggatggggtggggggacaggagggggccctggggcctgggccccggaaaaatctatctgccctcccccacactttatatacgaataaacgcagaagagggggaggggaagctttatttatagaaatgacaatagagggccacggggaggcccccccagaagcaagattcaaatctcttgctttctttcttaaaaaaaagaaaaagaaaaagcaagaagaaggaagaaagaaaaagacagaaagagaaataggaggaggctgcagctcctcgttttcagctttggcgaagatggatccacgtttcatctttaatcacgccaggtccaggcccatctgtcttgtttcctctgccgaggagaagacgggcctcggtggcgaccattacctcgacacccgctaacaaatgaggcccggctcggccgcctccgcctctgctactgccgctgctggaagacagcctggatttcctttctttgtcccccactcccgatacccagcgaaagcaccctctgactgccagatagtgcagtgttttggtcacggtaacacacacacactctccctcatctttcgtgcccattcactgagggccagaatgactgctcacccacttccaccgtggggttgggggtgggcaacagaggaggggagcaagtagggaagggggtggccttgacaactcaggagtgagcaggaaaattgagtccaaggaaaaagagagactcagagacccgggagggccttcctctgaaaggccaagccaagccatgcttggcagggtgaggggccagttgagttctgggagctgggcactactctgccagtccagagttgtacagcagaagcctctctcctagactgaaaatgaatgtgaaactaggaaataaaatgtgcccctcccagtctgggaggaggatgttgcagagccctctcccatagtttattatgttgcatcgtttattattattattgataatattattattactatttttttgtgtcatgtgagtcctctctccttttctctttctgacattccaaaaccaggccccttcctacctctggggctgcttgagtctagaacccttcgtatgtgtgaatatctgtgtgctgtacagagtgacaatagaaataaatgtttggtttcttgtgaccagcaaaaaaaaaa

SEQ ID NO: 58 - DNA, 2566 bp, Mus <mouse, genus>
  Mouse Hoxb4 (NM_010459.7)
agctccctcttatcctggggaggagatggggccctatgggagtcagagaaaggttggtggagattaggtagggcaggggtgggggctacacccgcagccccaacttctgagggatgcagggtttgtgctctgcccagccccctcacccccaaacaggccctccaattaacctgctcactctttcttagttcatcacccctctctgttgtggagaaagccaggcgaggagggggtctccccgcgggagccctatgtaaatcctggtgttgggtgggtggggaggggtagagaaggggaaataaacctctttggctggagtagggtccgggtgagcagatttccttatccgggaatcgcaggccgggtggccattggctcggaggatcacgtgggcctctaactttgttcacttgacagtaagtaggagggctttcggaaacaggaaaacgagtcaggggtcggaataaattttagtatattttgtgggcaattcccagaaattaatggctatgagttcctttttgatcaactcaaactatgtcgaccccaagttccctccgtgcgaggagtattcacagagcgattacctacccagcgaccactcgcccgggtactacgccggcggccagaggcgagagagcggcttccagccggaggcggcctttgggcgccgggcgccgtgcactgtgcagcgctacgcggcctgccgagaccccgggcccccgccacctccgccgcccccgccgcccccgccaccgcccgggctgtcccctcgggctccagtgcagccaacagccggggccctcctcccggagcccgggcagcgcagcgaggcggtcagcagcagccccccgccgcctccctgcgcccagaaccccctgcatcccagcccgtcccactccgcgtgcaaagagcccgtcgtctacccctggatgcgcaaagttcacgtgagcacggtaaaccccaattacgccggcggggagcccaagcgctctcggaccgcctacactcgccagcaggtcctggagttggagaaggagtttcactacaatcgctacctgacgcgccgccggagggtggagatcgcccacgcgctctgcctgtccgagcgccagatcaagatctggttccagaatcggcgcatgaagtggaaaaaagaccacaagttgcccaacaccaagatccgctcgggtggcaccgcgggcgcagccggaggcccccctggccggcccaacggaggcccccctgcgctctagtgccccccaagcaggagttcgaacatgggggggtggggggaacagcgagcaccgaagggggtgcggggtatgggagggtccccgggcttgagcccagaaaaaatctatctaccctaccctcactttatctataaggaataaacacagagaaggggggtagggaagccttatttatagaaaggacaataagggagccgggtaaagtccttcggagacaagattcgagtctcttgctttcttcctttaaaaaaaaaaaagaaagaaagaaagaaggaaagaaagagagagagagaaaagaaaaagaagaaaggaaggaagcaagaaaaggaggaagaaaggaaaagacagaagagaaatggaggagtctgctgcgcctggttttcagctttggtgaagatggatccaggcttcatctttaatcacgccaggcccgggcccatctgtcttgtttactctgccgaggagaagacgggcgagcgagcttcggtggcgaccattacctcgacacttggctaacaaatgaggccaggctcggccgctgccgccgcctctgctgctgtcgctgctggatcacagcctggatttttctttctttgtcccctactcctgacacccagcgaatgcaccctcagactgccagatagcacagtgttttggccacggtaacaaacacacacacatataactttcctccctgtctgtacccactttggggtgggggtgggtgggaagactgctcactcccttccaccatagacttagaagggggaacagaagggaattgaagggcagtctgcacaacgtgggttcccaaatccgagcccaagaaataaatgaaaatgaaaaaagaaaggtagcaattgggacacccaagaaggccttctgctagaaggtccagctaggcctggcagggtgaggggcagttgagttctgggagctgggaatgtcttctgggcagttcacagtagtagagtcaaggccttctcttaggttacaaatgaatgtgaaattaggaaataaaatactgtggccctcctactctggaaggacaatgttgcagaaccctctcccgttgttatcattgttgcatcgtttattattattattattattattattattattattattattattattattattttatgtcatgtgtgtcctctctcctgttctctttctgacattccaaaaccaggccccttcctacctctggggctgcctgagcctagaaccttttgttggtgtgaaaatttgtgtcctgtacagagtgacaacagaaataaatgtttggtttcttgtgaccatca

SEQ ID NO: 59 - DNA, 3014 bp, Homo sapiens
  Human KLF4 (NM_001314052.1)
gcagaggcggtggcgggcggcggcggcaccgggagccgccgagtgaccctcccccgcccctctggccccccaccctcccacccgcccgtggcccgcgcccatggccgcgcgcgctccacacaactcaccggagtccgcgccttgcgccgccgaccagttcgcagctccgcgccacggcagccagtctcacctggcggcaccgcccgcccaccgccccggccacagcccctgcgcccacggcagcactcgaggcgaccgcgacagtggtgggggacgctgctgagtggaagagagcgcagcccggccaccggacctacttactcgccttgctgattgtctatttttgcgtttacaacttttctaagaacttttgtatacaaaggaactttttaaaaaagacgcttccaagttatatttaatccaaagaagaaggatctcggccaatttggggttttgggttttggcttcgtttcttctcttcgttgactttggggttcaggtgccccagctgcttcgggctgccgaggaccttctgggcccccacattaatgaggcagccacctggcgagtctgacatggctgtcagcgacgcgctgctcccatctttctccacgttcgcgtctggcccggcgggaagggagaagacactgcgtcaagcaggtgccccgaataaccgctggcgggaggagctctcccacatgaagcgacttcccccagtgcttcccggccgcccctatgacctggcggcggcgaccgtggccacagacctggagagcggcggagccggtgcggcttgcggcggtagcaacctggcgcccctacctcggagagagaccgaggagttcaacgatctcctggacctggactttattctctccaattcgctgacccatcctccggagtcagtggccgccaccgtgtcctcgtcagcgtcagcctcctcttcgtcgtcgccgtcgagcagcggccctgccagcgcgccctccacctgcagcttcacctatccgatccgggccgggaacgacccgggcgtggcgccgggcggcacgggcggaggcctcctctatggcagggagtccgctccccctccgacggctcccttcaacctggcggacatcaacgacgtgagcccctcgggcggcttcgtggccgagctcctgcggccagaattggacccggtgtacattccgccgcagcagccgcagccgccaggtggcgggctgatgggcaagttcgtgctgaaggcgtcgctgagcgcccctggcagcgagtacggcagcccgtcggtcatcagcgtcagcaaaggcagccctgacggcagccacccggtggtggtggcgccctacaacggcgggccgccgcgcacgtgccccaagatcaagcaggaggcggtctcttcgtgcacccacttgggcgctggaccccctctcagcaatggccaccggccggctgcacacgacttccccctggggcggcagctccccagcaggactaccccgaccctgggtcttgaggaagtgctgagcagcagggactgtcaccctgccctgccgcttcctcccggcttccatccccacccggggcccaattacccatccttcctgcccgatcagatgcagccgcaagtcccgccgctccattaccaaggtcagtcccggggatttgtagctcgggctggggagccctgtgtgtgctggccccacttcgggacacacgggatgatgctcaccccaccttcttcacccctagagctcatgccacccggttcctgcatgccagaggagcccaagccaaagaggggaagacgatcgtggccccggaaaaggaccgccacccacacttgtgattacgcgggctgcggcaaaacctacacaaagagttcccatctcaaggcacacctgcgaacccacacaggtgagaaaccttaccactgtgactgggacggctgtggatggaaattcgcccgctcagatgaactgaccaggcactaccgtaaacacacggggcaccgcccgttccagtgccaaaaatgcgaccgagcattttccaggtcggaccacctcgccttacacatgaagaggcatttttaaatcccagacagtggatatgacccacactgccagaagagaattcagtattttttacttttcacactgtcttcccgatgagggaaggagcccagccagaaagcactacaatcatggtcaagttcccaactgagtcatcttgtgagtggataatcaggaaaaatgaggaatccaaaagacaaaaatcaaagaacagatggggtctgtgactggatcttctatcattccaattctaaatccgacttgaatattcctggacttacaaaatgccaagggggtgactggaagttgtggatatcagggtataaattatatccgtgagttgggggagggaagaccagaattcccttgaattgtgtattgatgcaatataagcataaaagatcaccttgtattctctttaccttctaaaagccattattatgatgttagaagaagaggaagaaattcaggtacagaaaacatgtttaaatagcctaaatgatggtgcttggtgagtcttggttctaaaggtaccaaacaaggaagccaaagttttcaaactgctgcatactttgacaaggaaaatctatatttgtcttccgatcaacatttatgacctaagtcaggtaatatacctggtttacttctttagcatttttatgcagacagtctgttatgcactgtggtttcagatgtgcaataatttgtacaatggtttattcccaagtatgccttaagcagaacaaatgtgtttttctatatagttccttgccttaataaatatgtaatataaatttaagcaaacgtctattttgtatatttgtaaactacaaagtaaaatgaacattttgtggagtttgtattttgcatactcaaggtgagaattaagttttaaataaacctataatattttataaaaaaaaaaaaaaaaaaaaaaaaaaaaaa

SEQ ID NO: 60 - DNA, 3057 bp, Mus <mouse, genus>
  Mouse Klf4 (NM_010637.3)
agttccccggccaagagagcgagcgcggctccgggcgcgcggggagcagaggcggtggcgggcggcggcggcacccggagccgccgagtgcccctccccgcccctccagccccccacccagcaacccgcccgtgacccgcgcccatggccgcgcgcacccggcacagtccccaggactccgcaccccgcgccaccgcccagctcgcagttccgcgccaccgcggccattctcacctggcggcgccgcccgcccaccgcccggaccacagcccccgcgccgccgacagccacagtggccgcgacaacggtgggggacactgctgagtccaagagcgtgcagcctggccatcggacctacttatctgccttgctgattgtctatttttataagagtttacaacttttctaagaatttttgtatacaaaggaacttttttaaagacatcgccggtttatattgaatccaaagaagaaggatctcgggcaatctgggggttttggtttgaggttttgtttctaaagtttttaatcttcgttgactttggggctcaggtacccctctctcttcttcggactccggaggaccttctgggcccccacattaatgaggcagccacctggcgagtctgacatggctgtcagcgacgctctgctcccgtccttctccacgttcgcgtccggcccggcgggaagggagaagacactgcgtccagcaggtgccccgactaaccgttggcgtgaggaactctctcacatgaagcgacttcccccacttcccggccgcccctacgacctggcggcgacggtggccacagacctggagagtggcggagctggtgcagcttgcagcagtaacaacccggccctcctagcccggagggagaccgaggagttcaacgacctcctggacctagactttatcctttccaactcgctaacccaccaggaatcggtggccgccaccgtgaccacctcggcgtcagcttcatcctcgtcttccccggcgagcagcggccctgccagcgcgccctccacctgcagcttcagctatccgatccgggccgggggtgacccgggcgtggctgccagcaacacaggtggagggctcctctacagccgagaatctgcgccacctcccacggcccccttcaacctggcggacatcaatgacgtgagcccctcgggcggcttcgtggctgagctcctgcggccggagttggacccagtatacattccgccacagcagcctcagccgccaggtggcgggctgatgggcaagtttgtgctgaaggcgtctctgaccacccctggcagcgagtacagcagcccttcggtcatcagtgttagcaaaggaagcccagacggcagccaccccgtggtagtggcgccctacagcggtggcccgccgcgcatgtgccccaagattaagcaagaggcggtcccgtcctgcacggtcagccggtccctagaggcccatttgagcgctggaccccagctcagcaacggccaccggcccaacacacacgacttccccctggggcggcagctccccaccaggactacccctacactgagtcccgaggaactgctgaacagcagggactgtcaccctggcctgcctcttcccccaggattccatccccatccggggcccaactaccctcctttcctgccagaccagatgcagtcacaagtcccctctctccattatcaagagctcatgccaccgggttcctgcctgccagaggagcccaagccaaagaggggaagaaggtcgtggccccggaaaagaacagccacccacacttgtgactatgcaggctgtggcaaaacctataccaagagttctcatctcaaggcacacctgcgaactcacacaggcgagaaaccttaccactgtgactgggacggctgtgggtggaaattcgcccgctccgatgaactgaccaggcactaccgcaaacacacagggcaccggccctttcagtgccagaagtgtgacagggccttttccaggtcggaccaccttgccttacacatgaagaggcacttttaaatcccacgtagtggatgtgacccacactgccaggagagagagttcagtatttttttttctaacctttcacactgtcttcccacgaggggaggagcccagctggcaagcgctacaatcatggtcaagttcccagcaagtcagcttgtgaatggataatcaggagaaaggaagagttcaagagacaaaacagaaatactaaaaacaaacaaacaaaaaaacaaacaaaaaaaacaagaaaaaaaaatcacagaacagatggggtctgatactggatggatcttctatcattccaataccaaatccaacttgaacatgcccggacttacaaaatgccaaggggtgactggaagtttgtggatatcagggtatacactaaatcagtgagcttggggggagggaagaccaggattcccttgaattgtgtttcgatgatgcaatacacacgtaaagatcaccttgtatgctctttgccttcttaaaaaaaaaaaaagccattattgtgtcggaggaagaggaagcgattcaggtacagaacatgttctaacagcctaaatgatggtgcttggtgagtcgtggttctaaaggtaccaaacgggggagccaaagttctccaactgctgcatacttttgacaaggaaaatctagttttgtcttccgatctacattgatgacctaagccaggtaaataagcctggtttatttctgtaacatttttatgcagacagtctgttatgcactgtggtttcagatgtgcaataatttgtacaatggtttattcccaagtatgcctttaagcagaacaaatgtgtttttctatatagttccttgccttaataaatatgtaatataaatttaagcaaacttctattttgtatatttgtaaactacaaagtaaaaaaaaatgaacattttgtggagtttgtattttgcatactcaaggtgagaaataagttttaaataaacctataatattttatctgaacgacaaaaaaaaaaaaaaa

SEQ ID NO: 61 - DNA, 3681 bp, Homo sapiens
  Human MYB (NM_001130173.1)
aatatcaacctgtttcctcctcctccttctcctcctcctccgtgacctcctcctcctctttctcctgagaaacttcgccccagcggtgcggagcgccgctgcgcagccggggagggacgcaggcaggcggcgggcagcgggaggcggcagcccggtgcggtccccgcggctctcggcggagccccgcgcccgccgcgccatggcccgaagaccccggcacagcatatatagcagtgacgaggatgatgaggactttgagatgtgtgaccatgactatgatgggctgcttcccaagtctggaaagcgtcacttggggaaaacaaggtggacccgggaagaggatgaaaaactgaagaagctggtggaacagaatggaacagatgactggaaagttattgccaattatctcccgaatcgaacagatgtgcagtgccagcaccgatggcagaaagtactaaaccctgagctcatcaagggtccttggaccaaagaagaagatcagagagtgatagagcttgtacagaaatacggtccgaaacgttggtctgttattgccaagcacttaaaggggagaattggaaaacaatgtagggagaggtggcataaccacttgaatccagaagttaagaaaacctcctggacagaagaggaagacagaattatttaccaggcacacaagagactggggaacagatgggcagaaatcgcaaagctactgcctggacgaactgataatgctatcaagaaccactggaattctacaatgcgtcggaaggtcgaacaggaaggttatctgcaggagtcttcaaaagccagccagccagcagtggccacaagcttccagaagaacagtcatttgatgggttttgctcaggctccgcctacagctcaactccctgccactggccagcccactgttaacaacgactattcctattaccacatttctgaagcacaaaatgtctccagtcatgttccataccctgtagcgttacatgtaaatatagtcaatgtccctcagccagctgccgcagccattcagagacactataatgatgaagaccctgagaaggaaaagcgaataaaggaattagaattgctcctaatgtcaaccgagaatgagctaaaaggacagcaggtgctaccaacacagaaccacacatgcagctaccccgggtggcacagcaccaccattgccgaccacaccagacctcatggagacagtgcacctgtttcctgtttgggagaacaccactccactccatctctgccagcggatcctggctccctacctgaagaaagcgcctcgccagcaaggtgcatgatcgtccaccagggcaccattctggataatgttaagaacctcttagaatttgcagaaacactccaatttatagattctgattcttcatcatggtgtgatctcagcagttttgaattctttgaagaagcagatttttcacctagccaacatcacacaggcaaagccctacagcttcagcaaagagagggcaatgggactaaacctgcaggagaacctagcccaagggtgaacaaacgtatgttgagtgagagttcacttgacccacccaaggtcttacctcctgcaaggcacagcacaattccactggtcatccttcgaaaaaaacggggccaggccagccccttagccactggagactgtagctccttcatatttgctgacgtcagcagttcaactcccaagcgttcccctgtcaaaagcctacccttctctccctcgcagttcttaaacacttccagtaaccatgaaaactcagacttggaaatgccttctttaacttccacccccctcattggtcacaaattgactgttacaacaccatttcatagagaccagactgtgaaaactcaaaaggaaaatactgtttttagaaccccagctatcaaaaggtcaatcttagaaagctctccaagaactcctacaccattcaaacatgcacttgcagctcaagaaattaaatacggtcccctgaagatgctacctcagacaccctctcatctagtagaagatctgcaggatgtgatcaaacaggaatctgatgaatctggaattgttgctgagtttcaagaaaatggaccacccttactgaagaaaatcaaacaagaggtggaatctccaactgataaatcaggaaacttcttctgctcacaccactgggaaggggacagtctgaatacccaactgttcacgcagacctcgcctgtggcagatgcaccgaatattcttacaagctccgttttaatggcaccagcatcagaagatgaagacaatgttctcaaagcatttacagtacctaaaaacaggtccctggcgagccccttgcagccttgtagcagtacctgggaacctgcatcctgtggaaagatggaggagcagatgacatcttccagtcaagctcgtaaatacgtgaatgcattctcagcccggacgctggtcatgtgagacatttccagaaaagcattatggttttcagaacacttcaagttgacttgggatatatcattcctcaacatgaaacttttcatgaatgggagaagaacctatttttgttgtggtacaacagttgagagcagcaccaagtgcatttagttgaatgaagtcttcttggatttcacccaactaaaaggatttttaaaaataaataacagtcttacctaaattattaggtaatgaattgtagccagttgttaatatcttaatgcagatttttttaaaaaaaacataaaatgatttatctgtattttaaaggatccaacagatcagtattttttcctgtgatgggttttttgaaatttgacacattaaaaggtactccagtatttcacttttctcgatcactaaacatatgcatatatttttaaaaatcagtaaaagcattactctaagtgtagacttaataccatgtgacatttaatccagattgtaaatgctcatttatggttaatgacattgaaggtacatttattgtaccaaaccattttatgagttttctgttagcttgctttaaaaattattactgtaagaaatagttttataaaaaattatatttttattcagtaatttaattttgtaaatgccaaatgaaaaacgttttttgctgctatggtcttagcctgtagacatgctgctagtatcagaggggcagtagagcttggacagaaagaaaagaaacttggtgttaggtaattgactatgcactagtatttcagactttttaattttatatatatatacattttttttccttctgcaatacatttgaaaacttgtttgggagactctgcattttttattgtggtttttttgttattgttggtttatacaagcatgcgttgcacttcttttttgggagatgtgtgttgttgatgttctatgttttgttttgagtgtagcctgactgttttataatttgggagttctgcatttgatccgcatcccctgtggtttctaagtgtatggtctcagaactgttgcatggatcctgtgtttgcaactggggagacagaaactgtggttgatagccagtcactgccttaagaacatttgatgcaagatggccagcactgaacttttgagatatgacggtgtacttactgccttgtagcaaaataaagatgtgcccttattttacctacaaa

SEQ ID NO: 62 - DNA, 3777 bp, Mus <mouse, genus>
  Mouse Myb (NM_001198914.1)
gggagtgtccaaacctctttgtttgatggcatctgtttacagagttacactttaatatcaacctgtttcctcctcctccttctcctccttctcctcctcctcctcggtgacctccttctcctcccctttctccggagaaacttcgccccggcggtgcggagcgccgctgcgcagccgggggaggacgcaggcaaggcggagggcagcgggaggcggcaaccggtgcggtccccggggctcttggcggagccccggcccgcctcgccatggcccggagaccccgacacagcatctacagtagcgatgaagatgatgaagacattgagatgtgtgaccatgactacgatgggctgctgcccaaatctggaaagcgtcacttggggaaaactaggtggacaagggaagaggatgagaagctgaagaagctggtggaacagaacggaacagacgactggaaagtcattgccaattatctgcccaaccggacagatgtgcagtgccaacaccggtggcagaaagtgctgaaccctgaactcatcaaaggtccctggaccaaagaagaagatcagagagtcatagagcttgtccagaaatatggtccgaagcgttggtctgttattgccaagcacttaaaagggagaattggaaagcagtgtcgggagaggtggcacaaccatttgaatccagaagttaagaaaacctcctggacagaagaggaggacagaatcatttaccaggcacacaagcgtctggggaacagatgggcagagatcgcaaagctgctgcccggacggactgataatgctatcaagaaccactggaattccaccatgcgtcgcaaggtggaacaggaaggctacctgcaggagccttccaaagccagccagacgccagtggccacgagcttccagaagaacaatcatttgatggggtttgggcatgcctcacctccatctcagctctctccaagtggccagtcctccgtcaacagcgaatatccctattaccacatcgccgaagcacaaaacatctccagtcacgttccctatcctgtcgcattgcatgttaatatagtcaacgtccctcagccggctgcggcagccatccagagacactataacgacgaagaccctgagaaggaaaagcgaataaaggagctggagttgctcctgatgtcaacagagaacgagctgaagggacagcaggcattaccaacacagaaccacacttgcagctaccccgggtggcacagcacctccattgtggaccagaccagacctcatggggatagtgcacctgtttcctgtttgggagaacaccatgccaccccatctctgcctgcagatcccggctccctacctgaagaaagtgcctcaccagcaaggtgcatgatcgtccaccagggcaccattctggacaatgttaagaacctcttagaatttgcagaaacactccagtttatagattctgattcttcgtggtgtgatctcagcagttttgaattctctgaagaagcggcagctttttcacctagccagcagcccacaggcaaagccttccagcttcagcaaagagagggccatgggactagatctgcaggagagcctagcctgagggtgaccaggcgagtgctgagcgaggcatccctcggcccagactcaccccaagcgaggcacagcaaggttccgctggtcgtcctacgaaaaaggcggggccaggccagccccctagccgctggagagcctagcccctccctctttgctgacgtcatcagctcaactctcaagcgttcccctgtcaaaagcctacccttctctccctcgcagttcttgaacacttccagcaaccatgaaagctcgggcttagatgcacctaccttaccctccactcctctcattggtcacaaactgacaccatgtcgagaccagactgtgaaaacccagaaggaaaattccatctttagaactccagctatcaaaaggtcaatcctcgaaagctctcctcgaactcccacaccattcaaacatgcccttgcagctcaagaaattaaatacggtcccctgaagatgctacctcagaccccctcccatgcagtggaggacctacaagatgtgattaagcaggaatcggatgaatctggaattgtggctgagtttcaagagagtggaccaccgttactgaaaaaaatcaagcaggaggtggagtcgccaactgagaaatcgggaaacttcttctgctcaaaccactgggcagagaacagcctgagcacccagctgttctcgcaggcgtctcctgtggcagatgccccaaatattcttacaagctctgttttaatgacacctgtatcagaagatgaagacaatgtcctcaaagcctttaccgtacctaagaacaggcccctggtgggtcccttgcagccatgcagtggtgcctgggagccagcatcctgtgggaagacagaggaccagatgacggcctccggtccggctcggaaatacgtgaacgcgttctcagctcgaactctggtcatgtgagacatttccagaaaagcattatggttttcagaacacttaaaagttgactttcgacacatggctcctcagcgtggagcgctccatggctgagagaagagcctgattttgttgtggtacaacagttgagagcagcaccaagtgcatttttagttgcttgagatctcacttgatttcacacaactaaaaaggatttttttttttaaaaataataataatgaataacagtcttacctaaattattaggtaatgaattgtgaccatttgttaatatcataatcagattttttaaaaaaaataaaatgatttatttgtattttagaggatacaacagatcagtatttttgactgtggtgaatttaaaaaaaaaatttacacaaagaaatatcccagtattccatgtatctcagtcactaaacatacacagagagatttttaaaaaccaggagaagcattattttgaatgttagctaaatcccaagtaatacttaatgcaaccctctaggagctcatttgtggctaataatcttggaaatatctttattatactaaaccatttcatgaggagaattttgttgtcagcttgcttgaaaagttattactgtatgaaatagttttattgaaaaaattatatttttattcagtaatttaattttgtaaatgccaaatggagaaatgtgttcgctgctatggttttagcctgtagtcatgctgctagctagtgtcagggggcaatagagcttagatggaaaaaagagaaagagactcggtgttagataacggactatgcactagtattccagacttttttatttttatatatatgtaccttttccttttgtaattggaaaacttatttgggagaattttgcatttgttgtacatttttgttttttaggattttttttttttgttgttattgtcgatttataaaagcattgcacttctttttctttttttgggagatttgtgttgtttatgtcatatgttttgttttgagttcagcctgaatgttcatccgtttgggcgtttttctgacttggaagaacattctctgtaggtttctaagtgtacagagccggaactgcctcgtggttcctgggcttcagggaagacaaatatggaagtcaacagccagtttctgccttgagagcatttgcaagaatgctggccttgaattctgaaatgacagtgtatctactgccttgtagcaaaataaagctatcctcttattttacatacttcc

SEQ ID NO: 63 - DNA, 1696 bp, Homo sapiens
  Human NFE2 (NM_006163.2)
tgttcttggggatcctcaagcatatactgtcatcatcttggaaagaaaaggctgagaacgtaaaactgaggacagaggaggaaagcagggtgacccctgatgttgccctagaaaatggaaaacaaaacacagcaaaacagaaaaacagaagatctgactctgcctttagccaggaaaacagtttgggggagtaaaaagtattagggaaaagagtgggcattttgcctggaaaaaaggtttctagagccatctgggctttccgggaacctggaccagactctggcccagtaggatgtccccgtgtcctccccagcagagcaggaacagggtgatacagctgtccacttcagagctaggagagatggaactgacttggcaggagatcatgtccatcaccgagctgcagggtctgaatgctccaagtgagccatcatttgagccccaagccccagctccataccttggacctccaccacccacaacttactgcccctgctcaatccacccagattctggcttcccacttcctccaccaccttatgagctcccagcatccacatcccatgtcccagatcccccatactcctatggcaacatggccataccagtctccaagccactgagcctctcaggcctgctcagtgagccgctccaagaccccttagccctcctggacattgggctgccagcagggccacctaagccccaagaagacccagaatccgactcaggattatccctcaactatagcgatgctgaatctcttgagctggaggggacagaggctggtcggcggcgcagcgaatatgtagagatgtacccagtggagtacccctactcactcatgcccaactccttggcccactccaactataccttgccagctgctgagacccccttggccttagagccctcctcaggccctgtgcgggctaagcccactgcacggggggaggcagggagtcgggatgaacgtcgggccttggccatgaagattccttttcctacggacaagattgtcaacttgccggtagatgactttaatgagctattggcaaggtacccgctgacagagagccagctagcgctagtccgggacatccgacgacggggcaaaaacaaggtggcagcccagaactgccgcaagaggaagctggaaaccattgtgcagctggagcgggagctggagcggctgaccaatgaacgggagcggcttctcagggcccgcggggaggcagaccggaccctggaggtcatgcgccaacagctgacagagctgtaccgtgacattttccagcaccttcgggatgaatcaggcaacagctactctcctgaagagtacgcgctgcaacaggctgccgatgggaccatcttccttgtgccccgggggaccaagatggaggccacagactgagctggcccagaggggtggaactgctgatgggatttccttcattcccttctgataaaggtactccccaaccctgagtcccagaaggagctgagttctctagaccagaagaggatgacaatggcaacaagtgtttggaagttccaaggtgtgttcaaagaggcttgccttgaggagggctggaatctgtcttccctgactcggctcctcaggtctttagcctccaccttgtctaagctttggtctataaagtgcgctacagaaatggcaaaaaaaaaaaaaaaa

SEQ ID NO: 64 - DNA, 1896 bp, Mus <mouse, genus>
  Mouse Nfe2 (NM_001302338.1)
gatctctaagcactcacttcttgggaagaaagggctgaaatactaggtgtggtggtacatgcctttaattccagcacttgggaggcagaggcagtcggatctctgtgagctagaagccagcctggtctacatagcaagttctaggacacagccagggacacatagcgagaccttgttttaaaaaacaacaatgaaagggttagaccctacgctgaggacacaagaagaaggcaagggtgactcttgatgttttcttccagaatggaaaatgaaatttcaatccccaaacctgagaaagactggattttgtctctggacaggaataccatttttagggagtaagagaaggcaacttgctgagaaaaagtaaggatacctactctgtgtccagaggactgactatggtcagatcaggtgaggtagagagtactccactgaagaaaagaacattacagttcatagggtggttgatggcacctgttgcaggaatcctttgtgcttgtggagacctggggccatcagctggcacagtaggatgcccccgtgtcctcctcagcagaacaggaacaggttatcacagctgcctgttggggagcttggagagatggaactgacttggcaagagatcatgtccattactgagctgcagggtctaaatgttccaagtgagacatcttttgagcctcaagcacccaccccataccctgggccactgccacctccaacatattgcccctgttcaattcatccagatgcaggcttctcccttcccccaccatcttatgagctcccagcatctactccccatgtcccagaactaccatactcctatggtaatgtagccataccagtgtcaaagccacttaccctttcaggcctgctcaatgagcccctcccagaccacttagctctcctggacattgggctgccagtggggcaacccaagccccaagaagacccagaatctgactcaggattatccctcaactacagtgatgcagaatctcttgagctagagggtatggaggctggcaggcggaggagcgagtacgcggacatgtacccagtggagtatccttactcacttatgcccaattctttggcccatcccaactatactcttccacccactgagacacccttggccttagagtcatcctccggtccagttcgggctaagcctgctgtccgtggggaggcagggagtcgggacgagcggcgagccctggccatgaagattcctttccctacggacaagatagttaacttgccggtagatgactttaatgagttgttggcacagtatccgctaacggagagccagctggctctagttcgggacatccgtcgacggggcaagaacaaggtggcagcccaaaactgtcgcaagagaaaactggaaaccattgtgcagctggagcgagagctggagcggctgagcagtgaaagggagcggcttctcagagcccgaggggaggctgaccgcactctggaggtcatgcgccaacagctggcagagctgtaccatgatattttccagcatcttcgggatgaatctggcaacagttactcaccagaggaatatgtactgcaacaggctgctgatggtgccatctttctggtaccccgtggaaccaaaatggaggctacagattgagctggtctagagagtggacactggtgctagagactccctcattcccttctgatgaaggcacttcttaatcccacaagactcagagtcctccagaccaaaaggcagatgtaaccatatcacctgggagtatttggtgaggtttgcctggaggccaggtgttggcttctcaggtcctcaaccccacctcttgtccaagctttggttcataaagagctgtgtggaaatagctaaaaaaaaaa

SEQ ID NO: 65 - DNA, 4093 bp, Homo sapiens
  Human NF-KB (NM_003998.3)
gtgagagagtgagcgagacagaaagagagagaagtgcaccagcgagccggggcaggaagaggaggtttcgccaccggagcggcccggcgacgcgctgacagcttcccctgcccttcccgtcggtcgggccgccagccgccgcagccctcggcctgcacgcagccaccggccccgctcccggagcccagcgccgccgaggccgcagccgcccggccagtaaggcggcgccgccgcccggccaccgcgcgccctgcgcttccctccgcccgcgctgcggccatggcgcggcgctgactggcctggcccggccccgccgcgctcccgctcgccccgacccgcactcgggcccgcccgggctccggcctgccgccgcctcttccttctccagccggcaggcccgcgccgcttaggagggagagcccacccgcgccaggaggccgaacgcggactcgccacccggcttcagaatggcagaagatgatccatatttgggaaggcctgaacaaatgtttcatttggatccttctttgactcatacaatatttaatccagaagtatttcaaccacagatggcactgccaacagcagatggcccataccttcaaatattagagcaacctaaacagagaggatttcgtttccgttatgtatgtgaaggcccatcccatggtggactacctggtgcctctagtgaaaagaacaagaagtcttaccctcaggtcaaaatctgcaactatgtgggaccagcaaaggttattgttcagttggtcacaaatggaaaaaatatccacctgcatgcccacagcctggtgggaaaacactgtgaggatgggatctgcactgtaactgctggacccaaggacatggtggtcggcttcgcaaacctgggtatacttcatgtgacaaagaaaaaagtatttgaaacactggaagcacgaatgacagaggcgtgtataaggggctataatcctggactcttggtgcaccctgaccttgcctatttgcaagcagaaggtggaggggaccggcagctgggagatcgggaaaaagagctaatccgccaagcagctctgcagcagaccaaggagatggacctcagcgtggtgcggctcatgtttacagcttttcttccggatagcactggcagcttcacaaggcgcctggaacccgtggtatcagacgccatctatgacagtaaagcccccaatgcatccaacttgaaaattgtaagaatggacaggacagctggatgtgtgactggaggggaggaaatttatcttctttgtgacaaagttcagaaagatgacatccagattcgattttatgaagaggaagaaaatggtggagtctgggaaggatttggagatttttcccccacagatgttcatagacaatttgccattgtcttcaaaactccaaagtataaagatattaatattacaaaaccagcctctgtgtttgtccagcttcggaggaaatctgacttggaaactagtgaaccaaaacctttcctctactatcctgaaatcaaagataaagaagaagtgcagaggaaacgtcagaagctcatgcccaatttttcggatagtttcggcggtggtagtggtgctggagctggaggcggaggcatgtttggtagtggcggtggaggagggggcactggaagtacaggtccagggtatagcttcccacactatggatttcctacttatggtgggattactttccatcctggaactactaaatctaatgctgggatgaagcatggaaccatggacactgaatctaaaaaggaccctgaaggttgtgacaaaagtgatgacaaaaacactgtaaacctctttgggaaagttattgaaaccacagagcaagatcaggagcccagcgaggccaccgttgggaatggtgaggtcactctaacgtatgcaacaggaacaaaagaagagagtgctggagttcaggataacctctttctagagaaggctatgcagcttgcaaagaggcatgccaatgcccttttcgactacgcggtgacaggagacgtgaagatgctgctggccgtccagcgccatctcactgctgtgcaggatgagaatggggacagtgtcttacacttagcaatcatccaccttcattctcaacttgtgagggatctactagaagtcacatctggtttgatttctgatgacattatcaacatgagaaatgatctgtaccagacgcccttgcacttggcagtgatcactaagcaggaagatgtggtggaggatttgctgagggctggggccgacctgagccttctggaccgcttgggtaactctgttttgcacctagctgccaaagaaggacatgataaagttctcagtatcttactcaagcacaaaaaggcagcactacttcttgaccaccccaacggggacggtctgaatgccattcatctagccatgatgagcaatagcctgccatgtttgctgctgctggtggccgctggggctgacgtcaatgctcaggagcagaagtccgggcgcacagcactgcacctggctgtggagcacgacaacatctcattggcaggctgcctgctcctggagggtgatgcccatgtggacagtactacctacgatggaaccacacccctgcatatagcagctgggagagggtccaccaggctggcagctcttctcaaagcagcaggagcagatcccctggtggagaactttgagcctctctatgacctggatgactcttgggaaaatgcaggagaggatgaaggagttgtgcctggaaccacgcctctagatatggccaccagctggcaggtatttgacatattaaatgggaaaccatatgagccagagtttacatctgatgatttactagcacaaggagacatgaaacagctggctgaagatgtgaagctgcagctgtataagttactagaaattcctgatccagacaaaaactgggctactctggcgcagaaattaggtctggggatacttaataatgccttccggctgagtcctgctccttccaaaacacttatggacaactatgaggtctctgggggtacagtcagagagctggtggaggccctgagacaaatgggctacaccgaagcaattgaagtgatccaggcagcctccagcccagtgaagaccacctctcaggcccactcgctgcctctctcgcctgcctccacaaggcagcaaatagacgagctccgagacagtgacagtgtctgcgacagcggcgtggagacatccttccgcaaactcagctttaccgagtctctgaccagtggtgcctcactgctaactctcaacaaaatgccccatgattatgggcaggaaggacctctagaaggcaaaatttagcctgctgacaatttcccacaccgtgtaaaccaaagccctaaaattccactgcgttgtccacaagacagaagctgaagtgcatccaaaggtgctcagagagccggcccgcctgaatcattctcgatttaactcgagaccttttcaacttggcttcctttcttggttcataaatgaattttagtttggttcacttacagatagtatctagcaatcacaacactggctgagcggatgcatctggggatgaggttgcttactaagctttgccagctgctgctggatcacagctgctttctgttgtcattgctgttgtccctctgctacgttcctattgtcattaaaggtatcacggtcgccacctggcattccttctgaccacagcatcattttgcattcaaattaagggttaagaaaagagatattttaaaatgagagtcacttgatgtgccattttaaaaaaaaaggcatattgctttttctaatgtggttatttctctgatttgcaaaaaaaaaaaaaaaaaaaatacttgtcaatatttaaacatggttacaatcattgctgaaaatggtattttcccccttttctgcattttgctattgtaaatatgttttttagatcaaatactttaaaggaaaaaatgttggatttataaatgctattttttattttacttttataataaaaggaaaagcaaattgatgacctcaaaaaaaaa

SEQ ID NO: 66 - DNA, 4128 bp, Mus <mouse, genus>
  Mouse Nf-kb (NM_008689.2)
gtccgtctgtctgctctctctcgacgtcagtgggaatttccagccaggaagtgagagagtgagcgagagaggacgagagagaagtaccgaggcgagccgggcaggaagaggaggtttcgccacccgagcagcccggctgcgcgctgacggcttcccgtgccctgcgcgcccccggcctgccgccgccgccgccgccgccgccgccctcggcctgctcgcgggccggctctagcagcgcaggccggagctcagggccccgccgcgcccggcccgccccgcgcttctccgcccgcgccgcagccatggcgcgccgctgagccgcccgcccgcccgcccgcgccccgacccggctcgggctcccgccggtccgcgccgctccgcagcgggagcccgcaggcgaggagaggccgcgccgcatctccagggtaccctcagaggccagaagagggtgtcagagcccttgtaactggagtttgacggtcgtgagctgcgcatcttcaccatggcagacgatgatccctacggaactgggcaaatgtttcatttgaacactgctttgactcactcaatatttaatgcagaattatattcaccagaaataccactgtcaacagatggcccataccttcaaatattagagcaaccaaaacagaggggatttcgattccgctatgtgtgtgaaggcccatcacacggagggcttccgggagcctctagtgagaagaacaagaaatcctacccacaggtcaaaatttgcaactatgtggggcctgcaaaggttatcgttcagttggtcacaaatggaaaaaacatccacctgcacgcccacagcctggtgggcaagcactgtgaggacggggtatgcaccgtaacagcaggacccaaggacatggtggttggctttgcaaacctgggaatacttcatgtgactaagaaaaaggtatttgaaacactggaagcacggatgacagaggcgtgtattaggggctataatcctggacttctggtgcattctgaccttgcctatctacaagcagaaggcggaggagaccggcaactcacagacagagagaaggagatcatccgccaggcagccgtgcagcagaccaaggagatggacctgagcgtggtgcgcctcatgttcacagccttcctccctgacagcactggcagcttcactcggagactggagcctgtggtgtcagacgccatctatgatagcaaagccccgaatgcatccaacctgaaaatcgtgagaatggacagaacagcaggatgtgtgacgggaggggaggagatttaccttctctgtgacaaggttcagaaagatgacatccagattcggttttatgaagaggaagaaaatggcggagtttgggaaggatttggggacttttcccccacagatgttcatagacagtttgccattgtcttcaaaacgccaaagtataaggatgtcaacattacaaagccagcttccgtgtttgttcagcttcggaggaaatcagacctggaaactagtgaaccgaaaccctttctctactaccctgaaatcaaagacaaagaggaagtgcaaaggaaacgccagaagcttatgccgaacttctcggacagcttcggtggcggcagtggagcgggagccggtggtggaggcatgttcggtagtggcggtggcggagggagtaccggaagccctggcccagggtatggctactcgaactacggatttcctccctacggtgggattacattccatcccggagtcacgaaatccaacgcaggggtcacccatggcaccataaacaccaaatttaaaaatggccctaaagattgtgccaagagtgatgacgaggagagtctgactctccctgagaaggaaactgaaggtgaagggcccagcctgcccatggcctgcaccaagacggaacccatcgccttggcatccaccatggaagacaaggagcaggacatgggatttcaggataacctctttcttgagaaggctctgcagctcgccaggcgacacgccaacgcccttttcgactacgcagtgacgggggatgtgaagatgttgctggccgtgcaacgccatctcaccgccgtgcaggatgagaatggggacagtgtcttacacttagccatcatccacctccacgctcagcttgtgagggatctgctggaagtcacatctggtttgatctctgatgacatcatcaacatgagaaatgacctgtatcagacacctctgcacttggccgtgatcaccaagcaggaagatgtagtagaggatttgctgagggttggggctgacctgagccttctggaccgctggggcaactctgtcctgcacctagctgccaaagaaggacacgacagaatcctcagcatcctgctcaagagcagaaaagcagcgccccttatcgaccaccccaatggggaaggtctaaatgccatccacatagctgtgatgagcaatagcctgccatgtctgctgctgctggtggctgccggggcagaagtcaatgctcaggagcagaagtctgggcgcacagcgctgcacctggccgtggagtacgacaacatctccttggctggctgcctgcttctggagggtgatgcccacgtggacagtaccacctatgatgggactacacctctgcatatagcggccggaagagggtccaccagactggcagctcttctcaaagcagcaggagcagaccccctggtggagaactttgagcctctctatgacctggacgactcttgggagaaggctggagaagatgagggagtggtgccaggtaccacacccctggacatggctgccaactggcaggtatttgacatactaaatgggaaaccgtatgagcctgtgttcacatctgatgatatactaccacaaggggacatgaagcagctgacagaagacacgaggctacaactctgcaaactgctggaaattcctgatccagacaaaaactgggccactctggcacagaagttgggtctggggatactgaacaatgccttccggctgagtcctgctccttctaaaactctcatggacaactatgaggtctctgggggtaccatcaaagagctgatggaggccctgcaacagatgggctacacagaggccattgaagtgatccaggcagccttccgcaccccggcaaccacagcctccagccccgtgaccactgctcaggtccactgtctgcctctctcgtcttcctccacgaggcagcacatagatgaactccgggatagtgacagcgtctgtgacagtggtgtggagacatccttccgcaaactcagctttacagagtctcttactggagacagcccactgctatctctgaacaaaatgccccacggttatgggcaggaaggacctattgaaggcaaaatttagcctgctggccgttcccccacactgtgtaaaccaaagccctgacagtccattgcatcgtcccaaaggaggaaggcaaagcgaatccaaaggtgctggagaatcgccggcctgcagggtcactcgatttcattcaaggccttccgaatttggcgtcctttcttggttctgaaatgaaatgtagttgccacgcacagacggtgtctagcaatcatggcgctcgctcgctcagctgcactctatggctcaggtgcagtgtcttgagctttctctgctgctactggatcacatttgctttgtgttgttactgctgtccctccgctgggttcctgctgtcattaaaaggtgtcgctgtccccacccggtgtcctttctagccatctactgtaagttgtgcattcaaattaagattaaggaaaaacatatttttaaatgagtaccttgatgcgcaataaaaaaaagacatttctttttttaatgtggtttatctgtgatttaaaaataaaaaacacatgaacttacaatatttaaaacatgctacaatcagtgctgaaaatagtattttccccgttttatgcattttactattgtaaatatgttttctaaatcaaatactttaaaagaagaaatgttgaatttataaatgctatttacttttttattttacttttataataaaagtacaagcacattgttgacctaaaaaaaaaaaa